European Patent Specification EP 3 551 194 B1, published October 18, 2023. Title: GLYCAN POLYMERS AND RELATED METHODS THEREOF. Applicant: KALEIDO BIOSCIENCES, INC. The sequence listing filed with the application follows.

SEQUENCE LISTING (124 sequences)

SEQ ID NO: 1 - DNA, 2217 bp, Lactobacillus sp.
  source: /note="GH36.0-1"
atggcagtaacgttgcagcaaactttaattgacattgatgaagaacaacttgtctttcacctgcataacgatcaaatctcgtatattctaggtgtggagacaggcaacgtgttggcccacttgtactttggcccacgggttcggggttatcatggcgagcgtcagtatccccggattgatcgggggttctcaggaaatttaccgaatacgactgatcgaagctattccaaggatgatttgccacaggaatacggtggcaataataccggtgattatcggcaacccgccgcgattattcgcgcggccaatggtgctcgaacagttgattttcgttatcaagactgccggatggaagccggtaagccggaacttaagggcttgccacaaacttatgtcgaagatgaggatgaagcccaaactttgattgtgacgttgcgagatgccacattaggcgtgacactcgaattagcctacacgatttatcgggatcggccagttatcacgcgtagcgcccggttgattaatcacagtgagcaagctgtcgacttagaaaaagtggcttcgatgcagatggacctgccaacccaaccattagatgccatttcgttacctggaagctatgcgcgtgagcgccagcttagtcgtgaacggctccatcgaggtgtaactcagtttgaaagtcgccggggtgctagttctcatcatatgaatccttttgtggcgctagctgatccgaatactaatgaatttcaaggcaatgtccttggtgcattgctaatttattcaggtaaccaccagattagtttagaacgggacccaattggtcagacacgcttgactatgggaatcaatgaatataacttcgactggcgattggcggccggtgatagtttccaaacgcccgaggttgcaatggtatactcgacgacggggcttaatggtatgtcgcaaacctaccatgatttattgcgtgatcgcgtggcgcgcagtcgttacaagcacgatctccggccgatcttgatcaacaattgggaagccacttactttgactttgatgcggacaagattcaatcaatcttggatgctgcagcaccactgggtatcgaaatgtttgtgctggatgacggttggttcggtcatcgaaatgatgataatagttcgctaggtgactggtttgttaatcggaacaagttaccaggaggcttagcggatattagcaaacggacccatgataaagggatgcggttcggactttggttcgagccagaaaatatttcagccgattccgatctttatcgggcccatcctgattgggtgttaggcgtaccagatcgtggccgaacgttatcgcggaacgaatacgtgcttgatttcagccagccggatgttgtcgacaatatttttgaacaaatgaccgcagttcttgataaggtgcccattgattatatcaagtgggatatgaaccgcaatttaacggaagtctattcgccacatagcgattcaactcatgaaggtgagactagccaccgctttatcttaggtgtatatgacttgatggagcgtttaacaaaacgctatccacagatcttatttgaaggctgctctggcggtggtggccgctttgatgctggtttaatgtattatatgccacagagttggccatcagataataatgacccgattgaacggctcaaaattcaatatgggacttcactcgtttatccaatttctgcaattaccgcccatgttgggacgagcccggatgaattgttaggacggtcgacgtcgatgaagatgcgtggtgctgtggcaatgagtggtaccttgggctatgaactggacgcggcccaactaagtgatgcggacaagcaggccgttaaaagacaggttgccttctataagcagcaccgtgagttagttcaatacgggaccttttatcgattagagagcccgtttgaatctaatacggtggcgtggatgtttgttagtccggatcagaaagaagccttgctgctcaccttcgttattttaggtgcagttcaaccagaaccgcatattacgaagttagcgggattagaccctcagcagacctacgttgagaccgacacaaacaaaatgtacggtggcgatgaattgatgcaactaggactctacacgactcccgttcaaactagtgactttacggcgcaggtacattacttcaaggctaaggactaa

SEQ ID NO: 2 - DNA, 1911 bp, Lactobacillus sp.
  source: /note="GH2.0"
atggtaacgaacttaaggagggttatttttatggaagcagagctgaaatggttggacgacccagaagtttttcgggtcaatcaactgccggcccacagcgatcatcgcttttaccgggaccaagaagaagccgctttggaaaagagtagctacgttcagaatttaaatgggcgttggggctttaagttctccaagaacccaatggagcgccccgtcgacttttacaagcttgattttgatcgtaacgactttggtgagattgaagtgccaagtgaaatcgagctgagtaactttgcccagatcaactacaccaacatcacgatgccttggactgggaaaatttaccgccggcctgcctacaccctgggggataacaaggaagagggttcctttagccaggggcaagacaatacggtggggtcttacgtgcgccacttcaccctagcagagggtctcaaaaaccacgacgttcacgtggtctttgaaggggttgaacgggcgatgtacgtgtggttaaacggccactttatcggttacgccgaggattcctttaccccgtccgaatttgatttaacgccgtacttagtagatggcgataacctcttagccgttgaggtttacaagcacgctacctcttcttggattgaagaccaagacatgttccgcttctccgggatcttccgcgacgtcaacttggtggcccaaccaagcatccacgtccaagacttaaagatcgacgcccgggtggccgatgacatgaagaccgggagcctagggctggtgttgaagatggttggccaaccggggagcgttcaggttgaagtcgccgatcaaaccggggccgccgtgctcaaccgccagttaaacgccgatggcaactggacaatggcaccagtccaactggtggggattcacctgtgggataaccaccatccgtacctttaccaattaaccctgacggttcgtgacgctacgggccgggtcgtcgaagtaatcccatatcagtttggcttccgccgggttgaaatcgaccaagacaaggtgctgcgtttaaacggtaagcgcctcatcatcaacggggtcaaccgccacgagtggaattgccaccggggccgggcggtgaccatagaagacatgcacaccgatttgggcatcttcaaggaaaataacatcaacgccgtgcggaccagccactacccagaccaaatttcgtggtattacctgtgtgaccgggaaggcatctacatgatggcggaaaacaacttggaaagccacgctacttggcaaaaatttggccaagacgagccgtcatataacgtgccagggtcgcttccccagtggaaagaggccgttgtcgaccgggcccgcagtaactacgaaacctttaagaaccacaccgccatcctcttctggtcggtggggaacgaatcctatgccggtgaagacattttagccatgaataactactacaaagaagttgatgatacccggccagttcactacgaaggggtcgtgcacaccaaggaataccgtgaccaaatttccgactttgaaagctggatgtacctaccgccaaaggaagttgaagcctacctgaaaaagaacccggacaaaccatttatcgagtgtgagtacatgcactcgatggggaactccgttgggggaatgggttcatacatcaaactcttggataagtacccgcagtactgtgggggctttatttgggacttcgttgaccaagccattgaagtggtcgacccagtaaccgggcaaaagtcgatgcgctacgggggcgactttgatgaccaccacgctgacaatgaattctcaggtgacgggatttgctttgctgaccggaccccgaagccggccatgcaggaggtgaaatactactatggattacacaaataa

SEQ ID NO: 3 - DNA, 2232 bp, Ruminococcus sp.
  source: /note="GH36.0"
atgagcatttgttatcacgaaggatcccgggaatttcatctttccaacagggatatcagttatattatcacagtcttaaaaaacggacagttaggacagctgtattttgggaaaaaactgcatgacagggagagttttgcccatctgctggagctgcgtcaccgcccaatggctgtatgtacttacgaaggagattccacattctcgatggaacatatcaagcaggaatatccgtcctatggagcaggggatatgcggtatccggcggtggagattctgcaggaaaacggaagccggatcacggattttgtgtatcagacacatcggatttatgacgggaagcccgcgcttgcaggactgccggctacctataccgaagattccaaagaggcacagacactggaaatcgaactgaaagatgagctgattcacaccacactgatcttgtactatacgatttttgaagagcttccggcgattacaagaagtgcaaaggtgatttaccacggaacagagaagatcgtgctggaacgtgcaatgagctgcagtgtggatctgccggatcacgactatcaaatgatcgagctgacgggagcctggggaagagagcgtgcggtgactgagcgaaagctgcagtatggaattcagggaatttatagtatgcgcggatgcagcagcagtaactttaatccgtttctggcactgcgtcgggagaataccacggaagcgtgcggggaagtgtatggcttcagtcttgtttacagcgggaattttctggcgcaggcagaggtggatacatacgatgtcacaagagtgacgctgggaattcatccggaccggttttcctgggaaatgaaaaacggagatgagtttcagacaccggaggcggtgatggtctattccaatcgcggactgaacgggatgagtcaggcattccacagtctgtatcgtgcacgcctggcaagaggatactggagagaccgaccgagaccgattctcatcaataactgggaagcgacttattttgatttcaatgaggaaaagattctggagatcgtgcgcacggcaaaacagcttggaatcgaattgtttgtactggatgacggatggttcggaaaacgggaggatgatcattcttctctgggagactggtatccgaatctggaaaagctgccggatggcattgcaggaatcgcgaagaaggtagcggcggaaggcatgaaattcggtctctggtttgagccggaaatggtcaacaaggacagcaatctctatagagagcatccggactggattttgtctactccgggacgtcatatttcccatggaagaaatcagtatattctggatttttccagagccgaagtggtggatgccatttatggacaaatggaaaaaatcctggaggatgcgccgatttcttatatcaaatgggatatgaaccgctgtatgtcagaagtatactctcatacagccagtgccgcagatcagggtaaggtcatgcatcagtatattctaggtgtttatcggttatatgagaagctgacgggcagatttcctgaaattttatttgaatcctgtgcaagcggcggttcccgttttgatccgggattgctgtattatgcgccgcaggcatggacatcggatgatacggatgcagtggaacgttgtaagatccagtatggaacgtcccttgtctatccagtgagcagtatgggatctcacgtatcagcagtgccgaatcatcaggtgcttcgcaacacatctttgaaaatgcgtgcggatgtagcgtatttcggaacattcggatatgagctgaacccgaacagtctgacagaggcagagcgggaggtaatcaaaaagcagacggcatttatgaaagaacacagaagcctgatccagtatggaacattctatcgacttcagagcccgtttgcaggaaatgaaatggcatggatggttgtgtctgaggacaaaaaagaagcgattgtgggctggtatcgcttcctggagccgatcaatatcggatatcggagcgtcagactgcagggactggatccgaagcttccgtatcagatttcggatatggaaatggcattgtacggagatgagctgatgcaggccggactgatcgtatcagacgtggcgtccggacaaaatccggagcagtataatggagagaacggagatttccagtctcttctttatctgctgaaagcaaaggaagaataa

SEQ ID NO: 4 - DNA, 1992 bp, Ruminococcus sp.
  source: /note="GH31.0"
atgattagaaaatacagatatggagctccgtttgatacggaggcactgaccgaaaaaattgaaacagctgaggaagcttttccatatggggaaatcagccagaaagaaggatttgcttttacctatatcatggacgaagatgacatcgtttatggtctgggcgaatccaaccgtggaatcaataagagaggttactgctatatcagcaactgcacagatgatccaattcatacagaggacaagcgttctctgtatggagcccacaattttattatagtaagcggaaagactacatttggcctgttttttgactatccgtcaaaactgacctttgatatcggatataccagaatggacaccctcaaagtgtcctgcgagaatgcagatctggatatctatgtgatcgaaggtgagaatgcttacgatatcgtaaaacagttccgtcgtgtgatcggccgcagctacattccgccgaagttcgcttttggttttggacagagccgctggggctatacaacaaaagaagacttccgcgcagttgcaaaaggatatcgtgaaaatcatatcccgatcgacatgatctacatggatattgactatatgcaggattttaaggacttcacagtcaatgagaaaaactttcctgatttccctgaatttgtaaaggaaatgaaagaccaggagcttcgcctgatcccgatcattgatgccggcgtcaaggtggaaaaaggctacgaggtttacgaggaaggtgtaaaaaataactacttctgtaaaagagaagacggaagtgattttgttgcagctgtatggcctggagatacccattttccggatatgctgaatccggaagcccggaaatggttcggagataaataccgtttcctgatcgaccagggaatcgagggattctggaacgatatgaatgaaccggcaatcttttattcttctgagggacttgcagaggcaaaagaattcgccggagaatttgcaaaagacaccgaaggcaagatccatccgtgggcaatgcaggcaaagatgaaagatattgttaacagtccggaggattacaaaagattctatcacaatgtaaatggtaagaaaatccgccacgacaaagtgcataatctttttggttataacatgacaagagcagccggagaagcattcgaacgcattgatccggaaaaacgtttcctgatgttttccagatcttcttatattggaatgcatcgttacggaggaatctggatgggagacaataaatcctggtggtcacacattcttttaaatctgaagatgcttccatctctgaatatgtgtggatttatgtacacaggcgcagaccttggcggatttggtgacgacacgaccagagatcttctgctccgtttccttgcactcggtgtgtttacacctctgatgcgtgatcatgcggcagaaggaacaagagaacaggaatgttaccagttcgaaaacatcgaagatttccgcagcgtcattaacgccagatatcgtcttgtgccgtatctttacagtgaatacatgaaagctgcgttgaatgacgatatgtactttaaaccgcttggcttcgtttatccggatgataagatggcaatccgcgtcgaagaccagctgatgcttggcaacgagatcatgatcgcaccggtatacgagcagaacgcaagaggccgttacgtttacctgccagaagaaatgaaattcatcaagtttatgccggatggaagcatttctgaagaagtcctcgaaaagggagttcattatgtggatgttgctctcaatgaagtgcctcttttcattcgaagcggcaaatgcatcccggttgcagaagcagcagagtgcgtgaaggatattgatacagaaaatatgcagcttatcggatatgaaggcagcagctatactctgtatgaagatgatggaatccataaagattatgataagaaagaaaattatcgggttctgacgaaataa

SEQ ID NO: 5 - DNA, 1866 bp, Lactobacillus sp.
  source: /note="GH42.0"
ttgcttgaaccaagagaaggaaaatataatttctcaaaattagataaagttgtacaacaattatctgatgctaactttgatattgtgatgggaacagccacagcagcgatgccagcttggatgtttaaaaaatatcccgatattgccagagtagattatcaagacagacgtcatgtatttggtcagcggcataacttctgtcctaatagctcaaattatcaaagattagctggtgaattagtaaagcagttagttgaacgctacaaggataataagcatatcgtagtttggcacataaacaatgaatatggtggcaactgttattgtgagaattgtcaaaacgcttttagaaaatggttgaagaataaatataagaccgttgaaggtcttaacaaggcatggaatatgaatgtatggagccatacgatttatgactgggatgaaattgttgttcctaatgagttaggggatgtatggggaatagaaggtagtgaaactattgtagctggtctttcaattgattatctgcgttttcaatctgaaagtatgcaaaatcttttcaagatggaaaagaagattattaaaaaatatgatccggaaactcctgtaacgactaatttccatggtttgcctaacaagatggttgattatcaaaagtgggcaaaaggtcaagatattatttcatatgatagttatccaacttatgatgctcctgcatataaagcggcattcttgtatgacttaatgcgaagcttgaaacatcagccatttatgttaatggaatctgcgccttcacaagttaactggcaaccatatagtccgcttaagcggcctggacaaatggaagcaactgaatttcaagctgtagcccatggtgctgatacggtacaattcttccaattaaaacaagcagttggtggctccgaaaaattccacagtgcagttattgctcattcgcaaagaaccgatactagagtatttaaagaactagctgatttagggaagaaattaaagaatgctggaccaacgattttagggtcaaagactaaggcaaaggtcgcaattgtctttgattggagtaacttctggtcgtatgagtatgtggacggaattactcaagatttgaactatgtagattctattcttgattactaccgtcagttctatgaacgcaatattccaactgacatcattggtgtagacgatgactttagcaactatgatttggttgtagcgcctgtgctttatatggttaaacatggtcttgataagaagatcaacgactatgttgaaaacggtggtaactttgtcactacttatatgtcaggcatggtgaactcatcagataatgtatatcttggtggctatcctggtccattgaaggaagttacaggcatttgggttgaagaaagtgatgcagtagtcccaggacaaaagattaaggtcttaatgaatggtaaggattatgatactggtctgatctgtaacttgattcatccaaatgacgctaagattttggcaacttatgcgagtgaattttatgcaggtacgccagctgttaccgaaaatcaatatggcaaaggtagggcttggtatattggtacaaggcttgaacatcaagggttaactcaattattcaatcatattatttttgaaacgggtgttgaatcactggtttgcgatagtcataaactagaaataactaagcgtgttactgaagatggtaaggaactttactttgtgcttaatatgagtaatgaagaaagaacgttaccaagcaagttcacaggttatgaagatattttaactggtgaaaaagctcataaagatatgaaaggttgggatgttcaagtattgagaaattag

SEQ ID NO: 6 - DNA, 2199 bp, Lactobacillus sp.
  source: /note="GH36.0-2"
atgaccagtaacttaattaaatttgatgatcaaaataaagtatttcatttacataacaagcaaatatcatatttgctttctattgaagatggtggcacattaagtcatttatactttggtggagctgttaaaaattacaataatcaattaaagtatcctagattagaccgcggattttcaggaaatttgcctgaatcgcttgatcgtacattttcacgtgattcacttccaaaagaatatagtagtgctggtgaaatggactttcatactcctgctacaatagtacgtaatccagatggctcaaatgctttgtttttagcttataagtcatacaaaatcgaagatggtaagccagatttaaagggattaccacactcttggacaaaagaagatgacgaagcgcaaacgttaatagttactcttgaagataaggtaagcaagctagaatatgacttattatatacaatttatcgagatcgtcctgtaattgtacgttcagttcaagttcataatcatggtgaagaagcagtatatctcgaaaaagttgcttctatgcaaatggattatgtagataaggattttgaagtcattactttaccgggtgctcatgcaaatgagaggcgtgtgcaaagagaaaatattggtcaaggaattaaagtgttttctagttatcgtggcacatcaagtcaccaaatgaatcctttcatggcattagtagatcatgataccaatgaatttatgggtgaagcttatggttttgcactagcatattccggtaatcataaatttgaagttgaacgtgatcaatttggtcaaatccacgtgaataccggaattaatgattacaattttaaatggaaattgaatccaaatgaagaatttcaaactccagaagttttgatggtttattctgatcaaggattaaataaaatgagtcaggcatttcatagcttgatccatgaacgtattatgcgtagtaaatttaaggatcaaattagacctgttctggttaacaactgggaagcaacttattttgatttcaatgaagataaattaaaaactattgtcgataaggctaagaaattaggcctagaaatgtttgtcttagatgatggttggtttggtcatcgtgacgatgacaacagttctttaggagattggaaagtttataagaagaagtttcctaatggattaggacattttgcagattatgttcatgaacaaggattaaagtttggactatggtttgaaccagaaatgatctcatatgaatcaaatctatataaagaacatccagattatttaatgcatgtacctggtagaaagccgtgtccgtcaagaaatcaatatgtcctagaacttggtcgtaaagaagttcgtgataatatctttgagcagatggtaaaaatcctagatagtaaaaagattgattatattaaatgggatatgaaccgtagtttgtctgatatttatgaatcggatttacctgctgatcaacaaggagaagcatatcatcgttatgtattaggttattacgatttattaaataaattggtaactagatatcctgatattttatttgaaggatgctctggtggtggcggtagatttgatgtcggacaagcttattacacaccacaaatttgggctagtgacaatactgatgctattgaaagattaaagattcaatacggtactagccttgtttatccgcaatcaatgatgacatcacatgtttcagtatcacctaatgaacagaatggaagaattactccatttaatacacgtggggctgtagcaatgtggggcgacttaggctatgaacttgatttaaccaagatgagtgatgaagaaagtgatcaagttgttaaacaagtcacagaatataagaaaattagagaagttacccagtttggtacgctttatcgtttaaaggcttcagcaagcaatcaatgtgcatggatgatggttgattctaataagaatgaagcagttgtaactgtcgtcaatgtaatggctcacgctcaaccatattgtacgaagacaaaattagctggtcttgatccagataaacgatacaagaatttagaaactgatgaagtttttggtggcgacgagctaatgcaccttggcttttatgatcctattgaacgtggtgattttaaagccaaaatgtatcattttaaggctatcaattag

SEQ ID NO: 7 - DNA, 1263 bp, Bifidobacterium sp.
  source: /note="GH51.0-1"
atgggcatcgacgacttctaccgctggagccagaaagccggcaccgaaatcatgcttgccgtcaacatgggcacccggggtctgaaggccgcgctcgacgagctcgagtatgtcaacggcgcgcccggcaccgcttgggcggatcagcgcgtggccaacggcatcgaggagccgatggatatcaagatgtggtgcatcggcaacgaaatggacggcccgtggcaggtgggccacatgagtccggaagaatatgccagcgcggtggataaggtggcccacgccatgaagctcgccgagtccggtctcgaactcgtggcctgcggttcctcgggtgcctatatgccgaccttcggcacgtgggagaagaccgtgctcaccaaggcttacgagaatctcgacttcgtctcctgccatgcctactacttcgaccgcggccataaaacccggaccgccgcctccatgcaggacttcctggcctcttccgaagacatgaccaagttcatcgccaccgtctcggacgcggccgatcaggcgcgagaagccaacaacggcaccaaagacatcgccctgtccttcgacgaatggggcgtatggtattcggacaagtggaacgagcaggaagaccagtggaaggcggaggccgcgcagggtttgcaccacgagccatggcctaagtctccgcatttgctggaagacatctacaccgcggccgacgcggtggtcgaaggttccctgatgatcaccctgctcaagcactgcgatcgcgtgcgttccgcctcgcgcgcccagctggtcaacgtcatcgcccccatcatggccgaggaacacggcccggcatggcggcagaccacgttctacccgttcgccgaagccgcccttcacgcgcgcggccaggcctacgctccggccatcagctcccccaccatccataccgaggcatatggcgacgtgccggccatcgacgcggtagtcacgtgggatgaacaggcccgcaccggtctgctgcttgccgtcaaccgcgacgccaacaccccgcacacgctcaccatcgacctttccgggctgcccggcctgcccggtctcggcacgctcgcgctcggcaaggcgcaactgttgcatgaggacgatccgtaccgcaccaacaccgccgaagcgcccgaagccgtcacgccgcaaccgctcgacattgcgatgaacgccaccggcacctgcacggcaacgcttcccgccatctcctggatcagcgtggaattccacggctaa

SEQ ID NO: 8 - DNA, 3072 bp, Bifidobacterium sp.
  source: /note="GH2.0-5"
atgacagacgtcacacatgtcgatcgcgcatcgcaggcttggctgaccgacccgacggtgttcgaggtgaaccggactccggcccattccagccacaagtggtacgcccgcgacccccagagcggacaatggtccgatctcaagcagagccttgacggcgagtggcgggtcgaggtcgttcaggccgccgacatcaacctcgaagaggaacccgcgacggccgagtcgttcgacgactcctcgttcgagcgtatccaggttccgggccacctgcagacggccggtctgatgaaccacaagtacgtgaacgtccagtatccgtgggacggccacgagaacccgttggaaccgaacatcccggagaacaatcacgtcgcgctctaccgcaggaagttcaccgtctccgcccccgtggcaaacgccaagcaggccggcggatcggtgtcgatcgtgttccacggcatggccacggcgatctacgtgtgggtcaacggcgcgttcgtcggctatggcgaggacggcttcacgcccaatgagttcgacatcaccgaactgctgcacgacggggagaacgtcgtggccgtcgcctgctacgaatactccagcgcctcctggcttgaggatcaggacttctggcgtctgcacggcctgttccgctccgtcgaactcgccgcccgcccgcatgtgcacatcgagaacacgcagatcgaagccgattgggatcccgaggccggcaccgcctccctcgatgccgcgctgaccgtgctcaacgcggccgacgcggccacggtccgcgcgaccctgaaggacgccgacggcaacacggtgtggcagacgacgggcgacgcggaggcgcagaccgcgatctccagcgggccgctgcagggcatcgccccttggagcgccgaaagcccgacgctgtacgagcttgacgtcgacgtcatcgaccaggcgggcgacgtcatcgaatgcacgtcccagaaggtcggtttccgccgcttccgcatcgaggacggcatcctgaccatcaacggcaagcgcatcgtgttcaagggcgccgaccgccacgagttcgacgccgaacggggccgcgccatcaccgagcaggacatgatcgatgacgtggtcttctgcaagcgccacaacatcaactccatccgcacctcgcactacccgaaccaggaacgctggtacgaactgtgcgacgagtacggcatctacctgatcgacgaagccaacctcgaagcccacggcagctggtccctgcccggagacgtcctcaccgaggacaccatcgtgccgggtagcaagcgcgaatgggaaggcgcctgcgtcgaccgcgtcaacagcatgatgcgtcgcgactacaaccacccgagcgtgctgatctggtcactgggcaacgaatcctacgtgggcgacgtgttccgcgccatgtacaagcacgtgcacgacatcgacccgaaccgtccggtgcactacgagggcgtgacccacaaccgtgactacgatgacgtcaccgacatcgagacccgtatgtactcgcatgccgacgagatcgagaagtacctgaaggacgacccgaagaagccgtacctctcctgcgaatacatgcacgccatgggcaactccgtgggcaacatggacgaatacacggcgctcgaacgctacccgaagtatcagggcggcttcatctgggacttcatcgaccaggccatctacgccacccagcccgacggcaccaggagcctgcgctacggcggagacttcggcgaccgtccgtccgactacgagttctccggcgacggcctgctgttcgccgaccgcaagccttcccccaaggcccaggaagtcaagcagctgtactcgaacgtccacatcgacgtgacgaaggactcggtgtccgtcaagaacgacaacctgttcaccgccaccggcgactacgtgttcgtcctgagcgttctcgccgacggcaagccggtctggcagtccacccggcgtttcgacgtgcccgccggcgagacccgcacgttcgatgtcgcatggccggtggcggcgtaccgcgccgacgcccgcgaactggtgctgcaggtttcgcagcgtctcgccaaggcgaccgattgggccgaaagcggctacgagctcgccttcggacagaccgtggtgcccgcggacgccaccgcgacgcccgacacgaagccggccgatgggaccatcaccgtgggccgttggaacgccggcgtgcgaggcgccggacgcgaggtcctgctgtcgcgcacccagggcggcatggtctcctataccttcgccggcaacgagttcgtgctgcgccgtcccgcaatcaccaccttccgtccgctgaccgacaacgatcgcggcgccggtcacggtttcgagcgcgtccagtggctgggcgccggccgctacgcccgctgcgtggacaacgtgctcgagcagatcgacgacagcacgctcaagggcacgtacacgtatgagctcgccaccgcgcagcgcaccaaggtgaccgtctcctacacggcccacaccgatggccgcgtgaacctgcacgtcgaataccctggagagcagggtgacctgcccaccatcccggcgttcggcatcgaatggacgctgcctgtgcagtacacgaacctgaggttcttcggcaccggcccggcggagacgtacctggaccgcaaacacgccaagctcggcgtgtggagcaccaacgctttcgcggatcatgcgccgtacctcatgccgcaggagacgggcaaccatgaggatgtgcgttgggccgagattaccgacgatcacggccacggcatgcgcgtcagccgcgccgatggtgccgcgccgttcgcggtaagcctgttgccgtactccagcttcatgcttgaggaggctcagcaccaggacgagctgccgaagccgaagcacatgttcctgcgcgtccttgccgcacagatgggcgttggcggcgatgattcctggatgtcgccggtgcacccccagtaccatatcccggcggacaagccgatcagcctcgatgtcgacctcgagctgatctga

SEQ ID NO: 9 - DNA, 1548 bp, Bifidobacterium sp.
  source: /note="GH51.0-10"
atgccccagcaggaccatctgaccgcacgtctcgtcgtcgatgacgattttgaggtcgctccggtcaacaatcgtctgttcggttcgttcgtcgagcaccttggccgttgcgtgtacaccggcatctacgagcccgaccacccgaccgccgacgagcacggcttccgcaaggacgtcatcgacctggtcaaggaactcggcgccaccaccatccgctacccgggcggcaacttcgtgtccggctaccgctgggaggacggcatcggccccaagcaggaacgtccccgtcgactcgatctggcctggcattccaccgaaaccaacgaattcggcctgcacgagatggccgaatggcttgaggccaccggcggcaacgagctgatggaggccgtcaacctgggcacgcgcggcctgcaggaggccctggacctgctggagtacgcgaacgtgcccggcggcaccgagctgtcggaacgtcgccgcgccaacggcgccgacaagccgttcgatatccgcatgtggtgcctgggcaacgagatggacggcccgtggcagctcggccacaagtccgccgaggactacggcatgctcgccgcctccgtggccgccggcatgcgccagatcgatccggatgtggaactggtggtgtgcggctcctccgcccatggcatgccgaccttcggcaagtgggagcagaccgttcttgagaagacctacgagaacgtgaacttcgtctcctgccacgcctactaccagccgttcttcaaggaggacggcacgcgcgacatggccagcttcctggcctccggcgtggatatggacggcttcatcaaggacgtggccgccaccatcgacgccaccaaggcccatctgaagagcgcgcacgacgtgtacatctcgttcgatgaatggaatgtctggtaccagggtgaggagccgagcaagacccccgagggcatcggcaactggccggtggccccgcgtctgctggaggacatctacaccgccgccgacgccgtggtgttcggcgatctgatgatcacgctgctcaagaacgccgaccgcgtgcgcgccgccagcctggcgcagctggtcaatgtcatcgccccgatcatgacggagccgggcggcccggcctggcgccagaccacgttccacccgttctccgtgaccgcgcgcctggccaagggcggcaccgtgctggagccgaagctgtccgccggcaccgtggatacgccgcgctatggcgaggtcgacggcgtgaacgccgtggccgtgcgctgcgccgacggctcgctcgccgtgtttgcggtgaaccgttcgctcgaggcgaccgccgagttcgagatcaggctgcaggacggcgcgcagccggcatccgtcgaggcgcagacgctgcacgacgacgatctgttcgccgcgaatacgctctacgaccagaaccgtgtgaccccgcacgccaacgggtcggccatgtacgatgccgagtccggcgtggtccgcgtctccctgccgccggtgagttggaccgccctgcacatcaagtga

SEQ ID NO: 10 - DNA, 1131 bp, Bacteroides sp.
  source: /note="GH76.0-4"
atgttattttgccttacctccgcagtgggaaagacaccgggaaatacccgttatctttctattgccgactcgattctatctaatgtattgaatctctatcagacgaatgacggactactaacagaaacgtatcctgtcaatcccgaccaaaaaattacttatctggcgggcggaacgcagcagaacggaacgctgaaggcttcttttctatggccgtattccgggatgatgtcgggttgtgtggctttatacaaagcgaccggaaacaagaagtacaaaaagattctcgagaaaagaattctaccgggaatggagcagtattgggataacagtcgcttgccggcctgttatcagtcataccccaccaagtacgggcagcacggacgttattatgacgataacatctggattgcactggattactgcgattattaccaactgactcacaagcctgcatctttggaaaaagccgttgcattgtatcaatatatctacagtggatggagcgatgagataggcggtggcatcttttggtgtgaacagcagaaggaagcgaagcatacttgttccaatgcaccgtctactgtgctcggtgtcaagttgtaccggctgacgaaggatgccaaatacctcgaaaaagcaaaagagacgtatgcctggacgaaaaagcatctgtgcgaccctaccgaccatctttactgggataacatcaacctgaaagggaaagtttccaaagagaagtacgcctacaacagtggacagatgattcaggcgggtgtattgctctatgaggaaacgggagatgagcagtatttgcacgatgcacagcaaacagccgcaggaacagatgcctttttccgcacaaaagccgacaagaaagacccgactgtcaaagtgcataaagacatggcctggtttaacgtgatcttattcagaggactgaaagctctgtataagattgacaagaatccggcgtatgtcaatgcgatggtggaaaatgcgcttcacgcctgggaaaactaccgggatgaaaacggattattaggcagggattggtcgggacacaacaaggaacagtataaatggctgctcgacaatgcctgtcttattgaattctttgcagagatttaa

SEQ ID NO: 11 - DNA, 2556 bp, Bacteroides sp.
  source: /note="GH2.0-1"
atgatgattggtaaactaaaatatttgatgctggggggctgccttatactggggagctgcctggcattgggaggctgtctgatgttattaggagcatgtagcagttcttcccttgtatctccgcgggagcgatccgactttaatgcagactggcgttttcatttgggagacgggctgcaagcggcacaacctggttttgccgacaatgactggcgtgtactggatttgccccacgactgggcgattgaaggagacttcagtcaggaaaatccttccggtacaggaggaggggcacttccgggaggagtcggttggtatcgcaaaacttttagtgtagacaaagcggatgcaggaaagatatttcgcattgagtttgacggagtatatatgaactcggaggtatttatcaatggtgtttcattgggagtacgtccttatggatatattagtttcagctatgacctgactccttatctgaaatgggatgaaccgaatgtgctggctgtacgtgtggataatgcggagcaacctaattcacggtggtattcaggttgtggcatttaccggaatgtgtggctaagcaagaccggcccaatacatgtgggtggatggggaacgtatgtaacaacctcgtcagttgacgaaaaacaggctgtactgaatctcgctactacccttgtgaatgaaagtgatacgaacgaaaatgttactgtctgttcttccttgcaggatgctgaaggcagagaagttgctgaaacccggtcgagtggggaagcggaagccggtaaggaagttgtttttacccagcaactgactgtaaagcaacctcaactgtgggatattgatactccttatctgtatacactggttaccaaagtgatgcgaaacgaagaatgtatggataggtatactactcctgtcggtattcgcacatttagtttggatgcccggaaaggattcacgttgaatggcaggcagacaaaaattaatggtgtgtgtatgcatcatgacctgggctgtttgggagcggcagtcaacacacgtgccattgaacggcacttgcaaattctgaaagaaatggggtgtaacggcatacgttgttcccataatcctcccgcacccgaactgcttgatctttgtgaccgtatgggatttatcgtgatggatgaggcttttgatatgtggcggaagaaaaaaacggcacatgattatgcccgttacttcaatgaatggcacgagcgcgatttgaatgactttattttgcgtgaccgtaatcatccttctgtctttatgtggagtatcggtaatgaagtcctcgaacaatggagtgatgccaaagcggatacgttgagtctggaagaggccaatctgatcttaaatttcggacattcttctgaaatgttagccaaagaaggagaggagagtgtcaactctttgctgacgaaaaaattggtaagctttgtaaaagggcttgatcctacccgtcctgtcactgccggatgcaatgaaccgaattccggcaatcatttattccgttccggcgtactggatgtgattggctataattatcataacaaggatattcccaatgttccggctaatttcccggacaagccgtttatcattactgaaagcaattcagcgttgatgactcgcggatattaccgtatgcccagcgaccggatgtttatctggcccaagcgttgggacaaatcctttgccgattccacatttgcctgttcatcttatgaaaactgtcatgtgccttggggaaacactcatgaggaaagcttgaaattagtcagggacaacgactttatcagcgggcaatatgtatggacgggatttgattatatcggggaaccgactccttacggatggcctgcgcgtagttcgtactttggtattgtagatctggctggtttcccgaaagatgtctactatttgtatcagtcggaatggacggataagcaggtgttgcaccttttcccgcactggaactggactccgggacaggagattgatatgtggtgctactataatcaggctgatgaagtggaactgtttgtgaatggaaagtcgcaaggagtgaagcgtaaagaccttgataatctgcatgtagcttggcgtgtgaagtttgaaccgggaacggtgaaggtcattgcacgagagagtggtaaggtagtggcggaaaaggaaatctgcacagccggaaaacccgcagagattcgtctgactcctgatcgttctattctgactgctgatggaaaagatttgtgttttgtcactgtggaggtgttggatgagaaaggaaatctttgccctgatgctgacaatctagtgaatttcacagtacaaggtaatggctttatcgcaggggtagacaacggaaacccggtatcgatggaacgctttaaggatgaaaagaggaaagcattttatggaaaatgccttgttgtcattcagaacgatggaaaaccgggaaaagcaaagctgacggctacttcagagggacttcggcaagctgtactaaagatttcggcagaggaattgtaa

SEQ ID NO: 12 - DNA, 2361 bp, Bacteroides sp.
  source: /note="GH3.0-1"
atgaaaaacattaagaaaatggtattagtatcagcctttgccggtacttgtcttacgcctcatgcacagactgcctctcctgtcatcccgaccgatccggctattgaaactcatatccgggaatggcttcagaaaatgactctcgaacaaaaaatcggtcagatgtgtgaaatcacgattgatgtggtatccgatcttgaaaccagtcgtaagaaaggattctgccttagcgaggcaatgctcgacacggttatcggtaaatataaagtaggttcactgttgaatgttcctttaggggtagcacagaaaaaggagaagtgggcggaagccatcaaacagatacaggagaaatcgatgaaggagatcggtattccctgcatctatggggtagatcagattcatggaacgacttacacattggacggaacgatgtttccgcaaggcatcaacatgggagccaccttcaaccgcgagctaacgagaagaggtgccaaaatctccgcttatgaaacgaaagcaggctgcatcccctggacgttcgccccggtagtcgacttaggccgcgacccgcgctgggcacgtatgtgggagaactatggtgaagattgttatgtaaacgcagaaatgggtgtatcggccgtgaaaggttttcagggagaagacccgaaccgtatcggagaatacaatgtagctgcgtgcatgaagcattatatgggttacggtgtacctgtttccggtaaagaccgtactccatcttccatctcacgcagtgatatgcgtgaaaaacatttcgctcctttccttgccgctgtacgtcagggtgcattgagcgtaatggtaaactccggcgttgacaacggactgccttttcacgccaaccgtgagttgctgaccgaatggctgaaagaagacttgaactgggacggactgattgttacagactgggcggacattaacaatctctgtacccgggatcacatcgctgccaccaagaaagaggctgtcaagattgtcatcaatgctggtatcgacatgtcgatggttccttatgaagtgagtttctgcgattatctgaaagagttggttgaagaaggagaggtatctatggagcgtatcgatgatgcagtagcccgtgtgttgcgtctgaaatatcgtctgggattatttgaccatccatattgggacattaagaagtatgacaagttcggttctaaggaatttgcagctgttgccctgcaggctgccgaggaatcggaagtgttgctaaagaatgacggaaatatcctgccgatagcgaaaggcaaaaagattctgctgaccggtccgaacgcaaactcgatgcgttgtctgaacggcggatggtcgtatagctggcagggacacgttgctgatgagtatgcgcaggcatatcataccatctacgaggctttgtgtgagaaatacggaaaagagaatattatctatgaaccgggagtgacctatgcttcttacaaaaacgataattggtgggaagaaaacaaaccggaaactgaaaaacctgtggcagcggcagcacaagcggatattatcatcacctgcatcggtgaaaactcttattgcgaaactccgggcaacctgacggatcttaccttatcagaaaaccagcgcaatctggtaaaagctctggccgctacgggcaaacctattgtcctggttctgaatcagggacgtccacgtattatcaacgatatagtgcctttagctaaagcggttgtcaacatcatgttgccaagcaattacggtggtgatgcacttgctaacttattggccggtgatgccaacttcagtggaaaaatgccgttcacctatccccgacttatcaacgctttggcaacttatgactacaagccttgcgaaaacatggggcaaatgggaggtaactacaattatgattcggtgatggatattcaatggccgttcggtttcggattaagctatacgaattataagtacagcaatttaaaagtaaataaaccgacttttaatgctgacgacgaactgatattcacggttgacgtaaccaacacgggcaaagttgccggaaaagagagtgtgttattgttctctaaggacttagtggcaagcagcacaccggacaatatccgtttacgaaacttcgaaaaggtttctctggaaccgggagaaacaaagacggttacgctgaaactgaaaggaagcgacttggcatttgtgggatatgacggtaagtggagactggaaaaaggagatttcaagattaaatgcggtgaccaatggatggatattgtatgcgatcagacaaaagtatggaatactccgaataagaatacgctccacaaataa

SEQ ID NO: 13 - DNA, 2445 bp, Bacteroides sp.
  source: /note="GH31.0-7"
atgaaaatacatcatctattttggggtatatgtttatgcttcagcacaaatatcttattcgcacagaactatcagaaaacatcgtccggtatcaaaaccactgtaaatgcagtggatatagaagtacaattctttgcgcctgctgtggcgagagtaataaagtcaccggaaggtgttgcctatgaaaaacagagtctttctgtaattgccaaacctgaaaaggtgagtttcaaagctgatatacaagataataagattgtattgaataccagtgaactaagtgtcagtgtggacaccgggacgggaattgtttcttatttctcaaaggatggcaaatcattattggcagagaaatccggtatgcagtttatcgatttcgatgatgccgggacaaaaacttatcaggtttatcaaccttttatattagataaggaggaagctatttatggtttgggacaattgcaaaatggaaagatgattcagcggaacatgaccaaaaatctgatacagggaaatgttgaagatgtgtcgccattcttccagtccaccaaaggatatggtgtgttttgggataactattcgccgactctttttacggacaacgaagttgaaacatcttttcgttctgaagtaggtgattgtgtagactattatttcatgtatgggaaggatgccgatggtgtaatagcacaagtacgcagcttgaccgggcaagcaccgatgtttcctttatggacttatggttactggcaaagtaaagaaagatataaaagccaggaggaagtggtagacgttgttcgtaaatatcgtgaattgggtattcctttggatggcattattcaggattggcaatattgggggcataactatttgtggaatgcgatggattttcagaatccgactttcaataatcctcaaaagatgatggaggatgtccatgcgatgaacgcacacatggctatatctatctggtcgtcattcggaccgatgaccaaaccttatagagaattggacaaaaaaggtatgttgtttaatttcactacctggccgcaatcggggttggagtcatggccccccaatatggaatatccttccggtgtaagagtgtatgatgcttacaatcccgaagcgcgtgacatttattggaaatatctgaatgatggaatttttaagttgggaatggatgcctggtggatggattctaccgaacccgatcatttggattggaagccggaggatatggataccaaaacctatctgggctcgttccgtagggtgcgcaatgcttatccgttgatgactgtcggaggggtttacgaccatcagcgtgcagtgacttcggacaaacgggtgtttattttaacccgttcgggattcttggggcagcaacgttatggtgcaaatgtatggagtggtgatgtcgcttccacatgggagagttttagaaatcagattcctgccggattaaacttttctttgtgtggtatgcctcactggaatagtgatattggtggcttttttgcaggacattataataaaagctggaatgatgatagtgcttcaaaaaatccattgtatcaggagctttatgtgcgttggttgcagtttgggacgttcaatccgatgatgcgttcgcacgggacggatgtttatagggaaatctataagttcggaaagaagggcgaacctgtatatgatgctatcgagaagatgataggtttacgttactctctgttgccttatatttattctacttcttgggaggtgagcaatcgtcaatcgagttttatgcgcgctttgatgatggattttgtagatgacagaaaggtgtgggatatcaatgacgaatatatgtttggaaaatcgatccttgtggctccgattgctcatgcacaatatacaccggaagctgtggtaaaagtctccgaagaagaaggatggaacagagatggagcgaaaaaaacaaaaactgacgctgctgtggatttcatggaaacgaaatctactaacatatacttaccggcaggaacgctatggtatgacttctggacgaacgagaaacatgaaggcggaaaggaaattaccaaagagactacactggatgttattccattgtatgtaaaagcgggtagtattattcctgtcggtccacaagttcagtatgcaactgaaaaaccgtgggatcatcttgaattgaaggtgtatgcgggtgcgaatggaaacttcattttatatgaagatgaatttgataattacaattatgaaaaaggagcttatacggaaattccaatctcttggaataatgcatctcgtaaattgacgataggggcaagaaaaggtgcgtatgagggaatgttgaagaaccgtaagtttactgtaactcttcaggatgggactcaaaaaaacatcgattataatgggaaagcgatttctgtaaagttttga

SEQ ID NO: 14 - DNA, 2865 bp, Bacteroides sp.
  source: /note="GH31.0-1"
atgattatgaatatgaaaaacattttctattgcctgttgccgggacttcttttgggagcatgttccaataaggtctacgagaagacaggtgatagtgtgatagtcaaagtacaacacaaagaaacaggaggtccccgtttggttcgccttcaggtgatgggagataagttaattcacgtttctgccactgccgacagcaagtttgccgatccgcaaagtctgattgttgttccgcagaaaaaacaaacatcttttgccgtcgtgcagaatggcgatacgattacagtgtctactgaagaagtgaaagcatctgtattggctagtaccggagaggtgtggtttacggataaaaacggagagttaatcctgcaggagaataagggaggaggaaagacatttactccgatagaagtggaaggaacgaaaggatatacggtctgtcaggtttttgaatctcccgaagatgaagcgttttacggattaggccagcatcaggcggatgaatttaattataagggtaagaacgaagaactgttccagtataatacgaaagtttctgttccgtttgttgtttcgaataaaaactatggtatactgctggatagttattccttctgtcgtttcggtaatccgaatgattactcccagttgaatcgtatctttaaactttatgataagacaggccaggaaggggcgctaaccggtacttatgtgccgaaaaaaggagaaactctggtccgccgggaagactccatctatttcgagaatctgaaaacgattgagaatcttccgaagaaactgccgttaatgggggctaaagtcacttatgaaggagagatagaacctgctcaaacgggagagttcaagtttattctttattatgcgggatatgttaaggtctatttgaacaatgagccggtagtgccggaacgttggcggactgcatggaatcctaatagttataagtttgcagctcatttggaagcaggaaagcgtgtgccgttgaaaatcgagtggcagcctgatggcggacagtcttattgcggactgcgtgcattgacacctgttaatccggaagaacaggggaagcagtcgtggtggagtgaaatgaccaagcagctcgattattattttatggctggtgagaatatggacgacgtgattagcggttatcgttcgctgaccggaaagtctcccgttatgccgaaatgggcaatgggtttctggcaaagtcgtgagaagtataatacacaggaggaaatgttgggagcactgaaaggtttccgtgatcgtaaaatcccattggataatatcgtactggattggaatcattggccggagaatgcctggggaagtcatgagtttgataaagctcgttttccggacccgaaagcaatggttgattccatccatgctatgcatgcccgtatgatgatctcggtatggcctaagttttatgttactaccgaacatttcaaggagttcgacgagaatgggtggatgtatcagcagtctgttaaagatagtttgaaagattgggtaggtcccggttaccattatggtttttatgatgcgtatgatcccgatgcacggaaactgttctggaaacagatgtatgagcactattatccgttgggtatcgatgcttggtggatggatgccagcgaaccgaatgtacgtgactgtaccgacttggaatatcggaaagctttgtgcggacctacagcgttgggttcctctacggaatttttcaatgcgtatgcactgatgaatgcagaagccatttatgacggtcagcgcggagtagataataacaaacgggtgttcttattaacccgttcgggatttgccggattacagcgttattccacggctacatggagtggggatatcggtacacgttgggaggacatgaaggcacagatttctgccggattgaattttgccatgagtggaataccttactggacaatggatattggcggtttttgtgtagagaatcgttatgtggccggacagaaacaatggaacgcgacaaagacggaaaatgctgattataaagaatggcgtgagctgaatacccgctggtatcaattcggtgcgtttgttcctttatatcgtgcacacggacaataccctttccgtgaaatatgggagattgcgccggaagggcatcctgcttatcagtcggttgtatattatactaagttacgttataatatgatgccgtatatttattcgctggcaggtatgacttggtttgatgattatacaatcatgcgtcccttggtaatggatttcacagcggatgctgaagtgaatgatattggtgaccagtttatgttcggtccttcgtttatggtatctccggtttatcgctatggtgaccgcagtcgtgaaatttatttccctcaagcagagggctggtatgatttctattccggcaaattccaggctggaggagagagaaaagtaatagaagctccttatgagcgtattccgttgtatgtgcgtgcaggcgctatcattccgttcggagatgatattcagtatacggatgaaaaaccggcggagcacatccgtttgtatatttatcagggagcggatggggagtttacgttatacgaagatgaaggtgtgaattataactatgaacaagggatgtatgccatgataccgatgaagtatgatgaggctaccaagactttagtgattggtgagcgtcagggggagttcccgggtatgctgaaggagcgtactttcacggtagttacggtgaataaggagaaagcccaaccgtttgatttgaacgcgaaaggggtgactgtgaagtataatggcagcgagcagacattgaaactgtaa

SEQ ID NO: 15 - DNA, 1803 bp, Bacteroides sp.
  source: /note="GH43.12-1"
atgaactggcatatctttgcagaaaagatcagtaattcatatttgattataaagaaaataagaagtattatgaagaatacacaggtaatacaattaatgtcaatcgtctggctctccatatttatgttggggataacaatgatatcatgtaactcaaagaaagaacaacaattaccggctattggaaaatctgtggctctctttgattatttttcttataagggaaatgatgatttttatatttccaatcctctgtcaggtgaagactatttctataatcctattttgccgggatggtattctgatcctagtgtttgtacaaatggagaaggtgattatttcctagtaacatctacattcacttatttccccggtattcctatttttcacagcaaagacttggtgaattggaaacagatagggcatgtgttgaaccgtgcttcgcaattagtgaatatggaaggacagaaagtgagtggcggtatttttgctccggctatttcttataatccgtataacaagacatattatatggtaacaaccaatgtcggagccggaaatttctttgttaagacgcaagacccgtttggtgaatggtcggaacccgtcatgttgccggaggtcggaggtattgatccttctttcttttttgatgaagatggtaaggcatatattgttaataatgatgaggctccggataataaacctgaatatagcggacaccgtactatacgcatacaagagtttgatgtgaaaacagataagacgatcggtccccgtaaagttcttgtaaacaaaggagcccaaccggcagacaagccaatttggatagaaggtcctcatttatataagataaatggaaagtacttcttgatgtccgccgaaggtggaacgggaaactggcattcggaagtgattttccgtggtgattctccgatgggtaagtttcttccatggaaaaacaatccgattctgacgcaaagacatttgaattctgaccgtcctaattcggtaacctgtgctggtcatgcagacttgattcaagcaaaagagggagattggtgggctgtttttctggcttgtcgccctattaataatcagtttgagaatttgggacgtgaaacatttatgatgccggtgaaatggagtgaagacggattcccgtacatgacacaaggcgatgatttagtacctatgattgtaaaacgtgaaggtgcgaaacgcgatacgacagttacttatggtaatttcgagttaatagagaactttgattctcctgtacttgatatgccatggatgactttaagagcttctgcttccgatttatattcattgacggaaacacccggatatttgaccttgaagtgtgcagatattagcgctacggaaaagaaaactccggcatttgtctgtcgtcggttacaacatcataaatttgaatgtgctacccgtatgttgttcaatccttctaacgataaggaaacagccggaatgctgttgtttaaaaatgagacgcatcaatatttcttctgcttgaataaagtgggtgagaataaaaatatttctctgaaacaaatcggtgaaaaggagcagacattggcttcagatgaaatagacgcagatacaaatgaggtatatttgaaattagtatctcaaggaattggttacgatttctattattctattgatggtgaaaaaagctggaaactgctttgtaaagatgtagatcctagttatctctctactacaacggctggtggatttaccggtactacaattggattatacgctacttgcaaataa

SEQ ID NO: 16 - DNA, 1728 bp, Bacteroides sp.
  source: /note="GH43.12-8"
atgagaacattaaaattgattttgtcgggctggcaatccgtggggcttgtcgtatttattatgttgttttttaatatggaggtgagtggcaagggtaaaataacgaaaaatgctcctgtctttacgcaatttatttatcagggggaggatgctatttatcaaaacaatcctttaaagccgggtgagttctataatcctattttgcagggttgctatcccgatccgagtataacgcggaaaggtaatgattattatttggtgtgctcatcttttgctatgtttcccggggtacctattttccattctaatgatttggtcaactggaaacaaatcggtcatgtgctggacagaacgtcacaattaaaggttgaagattgcggtattagtgcaggtgtatatgctcctgctataagatataatcccaataatgatacgttttatatgataaccactcaattttccggtggctttggaaatatggtggtaaagacaaagaatccggagaatggctggagtgatccgatcaaacttcaatttgaaggcattgatccttctcttttctttgatgataatggcaaggcatacgtggtacataatgatgctcctgctaaagcaaacgagcgttactcgggacaccgtgtcataaaaatatgggattatgatgtggagaatgataaagtggttccgggaacggaccggatcatcgtaaacggtggcgtcaatatagaagaaaaaccgatatggattgaagctcctcatatctataagaaagatggacgttattatttaatgtgtgcggaaggaggaaccggaggctggcatagcgaagtcatttttgtaagtgatcatccgaaaggaccttatcttccggcaaataataatcctattttaactcaacgttattttcctgcaaaccgggcggataaagtagactgggctggtcatgcagacttagtggagggacccgacggaaaatattatggtgtatttttaggaatacgccccaatgagaagaacagagtgaataccggacgcgaaacttttattcttccggtggactggagcggaacatttcccgttttcgagaatgggcttatccctatgaaacctacattgaagatgccttcgggagtagagaaccaaacaggaaaaaacggttatttgcctagtggcaactttgtctttaaggatgatttctccgataagacattagactttagatggattggtcttagaggtcctcgtgaagaattcgttgatatgaccgataaaggattgcggatcgtcccttttacctcaaatatcaatgaagtgaaacctacttctaccttgttctaccgtcagcagcataatcaatttacagcggcagcaaccatggagtacaaaccgaaaaatgagaaagattttgccggtataacatgttatcagaatgaaagatatcactatgttttcggtatcactaaaaagggaaaagactattacctgatactgcaaagaaccgaaaaaggacaagcgagtgtcctgggtgaggtgaagatagaaacagagaaacctgtgacactgcaagtaacagccaatggagatgattatcgttttaattattcgattgatggcaagggtttcataaatttaggaggaaccgtttccggtgatattctttctactaatgaggctggtggctttacaggagcaatgattgggctgtatgcaacatctgttggttattaa

SEQ ID NO: 17 - DNA, 1545 bp, Bacteroides sp.
  source: /note="GH51.0-1"
atgaaagcaaaactattagtcagcacggcttttctggcagcatctgtatctctttctgcacaaaagagtgctaccataaccgtacatgccgaccaaggcaaagaaatcataccgaaggaaatttacggccagtttgccgaacacttgggttcatgtatctacggcggtctttgggtaggcgaaaactcggatattcctaatatcaagggatatcgcacagacgtattcaatgcactgaaagacttgtccgttcccgttcttcgctggccgggcggatgctttgccgatgaataccactggatggatggcattggtccgaaagagaaccgtccgaagatggtgaacaacaactggggcggtaccattgaagacaacagtttcggaacgcacgagtttttgaatctttgcgaaatgctgggttgcgaaccatacgtgagtggaaatgtaggtagcggcacagtggaagagcttgccaaatgggtggaatatatgacttctgacggagactcgcctatggccaaccttcgccgtaagaatggtcgcgacaaagcatggaaattgaaatatctcggcgtaggaaatgaaagctgggggtgcggtggcagcatgcgtccggaatattacgcagacttatatcgtcgttattctacttattgccgcaattatgacggcaaccgtctgttcaagattgccagtggcgcaagtgactatgattacaaatggacagatgtattgatgaatcgtgtaggacaccggatggacggtctttctctgcactattataccgtaaccggatggagtggcagcaaaggatcagccactcaattcaacaaggatgattattactggacgatgggcaaatgtctggaagtggaagatgtactcaagaaacattgtaccatcatggacaaatatgacaaggacaagaaaatcgctctcttactggacgaatggggaacctggtgggatgaggaaccgggaaccatcaaaggacatctgtatcagcagaacacattgcgtgatgctttcgtggcttctttaagtcttgatgtattccataaatatacagaccgcctgaaaatggcaaatatcgcgcagattgtcaatgtacttcaatcgatgattctgacaaaagacaaagaaatggtgttgacgcctacttattatgtcttcaagatgtataaagtacaccaggatgccacttatcttcctatcgacctgacttgcgaaaagatgagtgtacgtgataaccgcaccgttccgatggtaagcgccacagcttccaaaaataaagatggggtgatccatatttctctttccaatgtagatgctgatgaagcgcaggaaatcaccatcaatctgggtgatacgaaagccaagaaagctatcggagagattctgaccgcttccaaactgaccgattacaattcttttgaaaaacctaatattgtaaaaccggcacctttcaaagaggtaaaaatcaataaaggtacaatgaaggtaaaacttcctgctaagtccattgttactttagagttacagtaa

SEQ ID NO: 18 - DNA, 2328 bp, Bacteroides sp.
  source: /note="GH3.0-5"
atgaagaagaatatcatatccatggcagcagcaatggctgtcttgtcggcttgcggaccgggtgtgccgcagcttggaaagtcctctttggatgaagtgattggtgccatgacgctggaagaaaaggcacatctggtagtaggtactggtatggcaggtttctcgggtgacagtgccgtaatcggtgcgacgaaaaagctggtgccgggcgcggcaggaaccacctacccgatcgagcgtctcggcattcccgccgtggtgctggccgatggtcccgccggactgcgtatcgaccccaagcgtgagggggattcggctacatactattgtactcatttccctatcgggactttgctcgcctctacctgggaccaggaattggtggaaagtgtaggccggtccatcggtaacgaagtgctggaatacggtgcggacgtgctgttggctccggcactgaacattcaccgtaacccgctttgcggacgtaacttcgagtattattctgaagacccgttggtgtcgggtaagattgccgccgcctacgtacgtggtgtgcagagcaacggtgtgggtaccagtatcaagcactttgctgtgaacaaccaggaaaccaaccgtatggctacggatgcgcatgtatctccacgcgccttgcgcgaaatctacttgaaagggttcgagattgccgtgaaggaatccgctccttggaccgtgatgtcctcatacaactacctgaacggtgtctacacttcggaaaacaaggagttgcagacaacgatgttgcgcgacgaatggggcttcaagggcatggtgatgaccgactggtttggcggcaaggatgccgtggcacagatggtggcaggcaacgacatgttgcagcccggtctgcccaagcagtacgaagccatcgtgaagggtgtgcaggacggagcgttggacgaagccatcctcaatcagaatgtgaagcgtattctggagatgattctccagactccccacttcaagggatataaatactccaacaagcctgatttgaaggcgcatgctgccgttactcgccagtcggcaacggaaggcatggtattgctgaagaacgataacggtgctctgccgctggctgccgacgtgaagaacgtggcactcttcggttgcacttcctacgatttcattgcaggcggtacaggttcgggcaacgtgaaccgcgcttataccgtttcgctattggacggcttgaagaatgccggctatgtggtggatgaagcgctgaagaatagctatgaagcttacctgaaaaccgagaaagaacgtctgtccaaagataagaaagagtggttcatgcccgatacccgtccggctgagatggctgtttccgcacaagtcatccgcgagcaggctgccaaggccgatgtggcactggtgacgctgggacgtacctccggtgagtttctcgaccgtatggtagccgacttcaacctcaccaaagaggagcagagcatgttgaaagcagtgtccgatgctttccacgctgccggaaagaaggtagtggtggtacttaatatcggtggtgtgattgaaactgcttcttggaagtctgttcccgatgccatcctttgtgcatggcaggcaggccaggaaggaggaaacagtgtggctgacgtgctgagtggcaaggcttctccttcgggcaagctgacaatgactttcccggtgaagtttgaagatgccgcttcttccgccaacttcccgatagacatgcgtgtgagcaccgacctcgtgaacaagggcgggaagaagaacgacgtgaaggatgtggattataccaattatgaggaggatatctacgtgggttaccgttacttcgataccttcggcaagcaggtttcctatcctttcggttacggtctttcctatactacttttgcttacgacaaggctgctgtcaagtcagacaacggcgtctataccgtatctgtagaggtgaagaacaccggtaaggtagcaggtaaggaagtggttcagctttatgtatccgctcccgatgctgcagacgccaacaaacccgaaaaggaactgaaagcttttgccaagaccaaggaactgaaaccgggtgaagctactgtggtgacgctgaaagtgaatgctgccgacctggcttcctatgatgaggctgcatcggcatgggtggtaactcccggaaactacaagttcctcgttggggcttcctcacgcgacatcaaggctacgctggaggctgaagtagctgccgcaacgcagaagacgaacaacatcttgaaacttcaggaaccgatgagcctcttgaagagatga

SEQ ID NO: 19 - DNA, 336 bp, Streptococcus sp.
  source: /note="GH13.28-1"
atgtattcagcaaaagataataaacttcttggcgcatggcctggaactaagatgactaaaggagcgtcaggtcgttattcaatcacagttcctgcttcatatgctgaagaaggtgtgaaagttatcttcacaaataaccagggctcacaatatccacaaaatgaaggctttgatttcaaagcagaaggcttgtactcaaaagctgtcttgatgcctgatgttccagcaggaaaaactcgtgtaacctttgataaccctggtggttgggatagtgcgaacgctttctactatggaaatcctgttcaataccctctaggtgtatggccaggaacataa

SEQ ID NO: 20 - DNA, 1458 bp, Streptococcus sp.
  source: /note="GH13.5"
atgacaaatgaaactttaatgcagtactttgaatggtatctgccaaacgatggtaaacactggatgcgattagcggctgatgctcccacacttgctcaaaatggtatcacaaaaatttggatgcctccagcttttaaggctacacatgatggcgacgttggttatggcgtttatgatctttttgatctcggtgaatttgaccaaaaagggactatccgaacaaaatatggaacaaaagctgactatctacatgcaatttctgctttaaaagcaaatcatattgcacctttagctgatgttgtcttaaatcacaaagctgctgctgaccatactgaaactttttccgttgtcgaagttgcccccgatgaccgtacaaaaatcatcagtaaaccttttgacattgagggctggacaaacttcacttttgatggtcgacataaagcttacaatgattttgaatggcattggtaccactttactggaacggattatgatgtaaaaactggtaaaaacggtattttccaaattcagggtgacaacaaaggttgggcaaatcaagatttggttgatggcgaaaatggcaattacgattatcttatgtatgctgaccttgattttaaacacccagaagttatcaaaaatatctatgactgggcagagtggttcgtcaaaacaacaggagtttgtggttttcgcttggatgctattaaacacattgattcattctttatgagcaatttcatccgcgatatgaaggaaaaatacggtaaagacttttatgtttttggcgaattctggaacgatgatgaaaaaactaacaacgattatcttgaaacgactgagtaccgctttgacctaatcgacgttcgactccaccaaaatctttttgaagcaagcaaagaaaaagcttattacgacttgcgagaaatttttaatcatactttggtgaaaaatcagcctaattctgctgttactttcgttgacaatcatgatacccaacgagggcaagcacttgaatctacaattgaagaatggttcaaaccagcggcttacgctctcatcttacttcgccaaactggtcttccatgcatcttctacggtgactactacggcatttcaggtgaatttgcacaacaagactttcaagatgacattgataaattacttttcttaagacaagcagctgtttacggcaaagaaatgaactattttgacaatccaaattgtgttggttggacttatcttggaaatgaagagcaccctacttctcttgctgttttaatcaacaacaaacattctacagcaaaacgaatgtttgttggcaaaaaatggacaggaaaaacttttaccgattatctcggaaatcaaactgctactatcactatcgacgaagaaggttacggcagttttccagttggcgcagaatccgtctctgcttatattccacaagatcaataa

SEQ ID NO: 21 - DNA, 249 bp, Streptococcus sp.
  source: /note="GH13.28-2"
ttgcttattttaacagctattggtgctggcggcttagttcaagttaaagttgttaatgcagatgaacaagtgtcaatgaaagatggtaccatacttcatgcgtggtgctggtctttcaataccattaaagataatgtgcaagccattaaagacgctggttacacaagtgttcaaacgtccccaatcaacactgttgtagctggcgaaggtggaaataagagtttaaaaaattggtattatcaatactga

SEQ ID NO: 22 - DNA, 1260 bp, Bacteroides sp.
  source: /note="GH8.0-2"
atgaagaatttattctatctcctcctctgtctcatcgccggagcatcgtgcagtcaggcagacccgacaaagccctgggataaaggtgcctttgagacacagaaataccggaatctctttgccgagatgggttataaacaggcagacattgacgccaaactcaaatccgtcttcgacggtgtgttctacggccctgacaaagtatatttcgaagtaggcgattctatggcatatatcagcgacgtcaaaaatcatgacgtccgcaccgaaggtatgtcctacggattaatgattgccgtccagttcgaccgtcaggatatcttcgaccgtctctggcgatggggcacaaagtacatgcagcaccaggatggtccactgaaaggttactttgcctggagttgtgcaacggacggtacccgtaactcccaaggccccgcctccgacggagagctttactatgtaaccgccctcatcttcgcttccaaccgttggggaaatgacaccggcatcaactaccttgccgaagcccagaatatcctgaactgttccatggagaaagacggcacaaaccgtgtaatgcctttcatcaatgtggagcataagctcatcactttcgttccggacatacatggcggacgttttaccgacccgtcttaccatgtacccgctttttacgaagtatgggcacgctgggccaatgacggcagagctgacttttggcgtgaatgcgccgaacgcagccgcgaatatctgcataaaagtatccaccccgtaaccggactaaaccccgattataacaactatgacggcagtttgctgggcaacaaccgcatcatcggcgatgctttccgctttgactcctggcgcgtacctatgaacatcgccttagattactcctgggcatgtgccgacaaagagtggcaacaggaatacggcaataaaatccagaacttcctttacagccagggtattgatactttcgtagatcagtataacgtagacggcacgcaagtaaaagacaccctccgggccggagagcataaggcattaagacattctttaggtctggttgctacttccgccgccgcctcactgatgtgtacccacgagaaaagccgcgagtttgtagataagttatggaacgcaaaacatgagccgtatgaagacggatatttcgatgcttactatgacggattgctccgcctcttcgctttcatgcatctgagcggaaattatagaatcatattcccggaaaagtaa

SEQ ID NO: 23 - DNA, 1050 bp, Roseburia sp.
  source: /note="GH13.41-1"
atgagaaagttgacgaaaagctttcaaaagaggcaaagcattgcaagcagagtactgtgttttctgctagtgcttgcaatggtagtaacaatggttccggcgcttggcggtggaaacagtacggtgcaggcggcggagaatccaactgtgaggttgtattttgaaaaaccggatgattggaatatcccggcatttaactattggaatgaatccgatgttgaagtagacaatggggatgcagaaaaggtggaagtctggacgagtcaatcaaaacctgctatgttgaaagatgaatcaacaggttattattatattgatatccggacgaacagcatcagtggctttcagattgtaaacggtggaactggtgtaggaaacccggcagaaaagaaatttgaaaactgtgccattattgatgcaattaattcggcaacatcagatacatcattttatcttttaaagaatgataatggaatgtcatggtacttagacaaagataaaaatcaggtgttaccagagaaagaaaaagcagctgcacataaagttataatttattttgaaaaaccagaaaattggaaaacgcctgttatcaatctatggggcggcgattttgtattggacaatcaaggagctggggatgcgtctattgctgcgtggggaaatcaggacaaaccaaagctggctgtttcagaagctgaaaatatttatactgttacattaaccggaacaacaatatcaggttttcagttggtagatgctgacacaggagcagagacacagtttgatggtcagagcgaagaagtgaaagccatcaatgccatcaccacagacacctccatctattatttaagagatggaaagggtggcatgaaatggtacaaagatgctgacaaatccgaaactctgatcgaatacaaagaagcaggatatgtaagcccggaggtaaatggacgcgaggtaactttccgtgttccggttaagaaaaacaggggatgcagcatctgttacggttccgggaggaatgaatggttggaaacaggattcatctga

SEQ ID NO: 24 - DNA, 3945 bp, Roseburia sp.
  source: /note="GH13.41-2"
atgtggtctggaacatttaccattgcacccggaaaatatgaatacaaatttgcattaaataaaacctgggatgtatcgttttcagatccggcaaataacagggtaagtggaacaaacagtgttttgatcgtcccgggcttggctgacggaaaagcagatgccatgaagggaattgagacagcacttccagaaaaactgacattgtggtctgaagacggaacaagcagtgaagctccggttacttacagtttaaaaactgcaaataaagatattacattaaatggaaatagcattataatcggaaaatcttatacaggacagatcgtagaactgacggcaaaagcagagaacggacagacctctgactttgtggtcaatgtgacagaaaaattatatacatataccatttattattatgattttgataagacacatatgtcagaaaatgcatctgacttatggatctgggagaaaaatggtgctggagcgacagagggaacaccttttaccgcaaccgagacactttctgatgggaatgagtggctgcgcgcagaaataaaacttccatatacagaccttcagatcataccaagatcaaaagacgagtggaaatgggagaaggacacgatttcttatagcaacagcgcaggaacagaaaatgtaacactttatattgtatccaatagtaaacaggcatacacagagattccagagctggtagcaccgagatcccgctacgtcatgatcgagtacgacagaccggcgaaggactataccggctggaacatttacacctggaacagtggatttggctctgatgtatctgtagcatttgcagacatcaatggcaaaatggttgcaaaaataccggtaaaagattcaaaagcagatcttaaattgtctttctgtatgaggcacagcacggcagctgatgaatgggagagcaaagacggcggagatcattatgtgacgatcccggcagaccagtcagtggtaaaagcagtgttcacacagggagaaggaatcacaagagtattgccatgcaacacaggttttgagcgggatggagcaaataatgcaatccatttttactacagaaatgatgaactggcagcagagaataaccttgcttctttagaaggaaatgtaagtattgtgatcaacggacagacttatgcaatggcttatgacgcagaaaacgatcgttttgtatacaatcttacagatgtttccacgggtgattactattattactatgtggtaaatggaaaagaggaattagatgcatttaatgatgtaactgcaaacgacagcaatggaaaagaatgcagcgtatgccacttcaaaaaagcaaatgtgagcgtagaggcttctttatcacagtatgcaatggattacaatgacaacaatgtgttatccgtaaaattgacagcaaaagacggagaaggtcttgaaacgtctgaaattgcagcgatcacagccgatctgagtgagctgggattgggaaaagagtttgcgatcgagccggaacttatggaaggaacaatctcctgcctgaatacagttgcagcaggcgtaaaaaatattccggtcacagtgaaagatatttatggaaatgtatacacaacagcgacaaacgttaccgtcacagagcgcaaaaaaagtgccggagatttcgactgggatgaggcagtgatttactttgcagtgacagaccgtttctttgacggagatgcaagcaacaatgatgcttacggagtaggcgattataacgttggtgaaaaaggcggttccagctatcacggtggagattttgccggattaaaccagaaactggattatttaaaagatctgggtgtgaacacaatctggatcactccgatcgtagaaaatatcacagaggatcagcatgataatgagacagataccgctacctatggctatcatggttactgggcaagtgatttcacaaagttaaacaaacatcttggaaaagagcagcagttcaaagcattactggatgccgctcacagcaagggaatgaaaatcatggtggacgtagtattaaaccatgcaggatacggtagagaagattactttaacagcattttaacagatgcagatggaaacagtatttccatgatccgtgactccagcaacacgatcagtggtgatgataaatatgattcattgtcagatctgcctgattttgtgacggaaaacaaagcagtgacagaccagcttgttgcatggcagaccgagtggatgtcaaaatacaatattgactattatcgtgtggatactgtaaaacatgtagagacaacgacatgggcagcatttaaaaattccctgaccaaagtaaatcctgattttaaaatgataggagagtattccggtgcaggatatgccaacaatgcaggagaattaggaaccggaacgatggatgcacttcttgattttgatttcaacgattttgcacagaactttgtgacaggaaatatttccagcgtggaaaattcactgcagaagagaaacaatgcgatcaacaacacctctgtcatgggaagctttttgagcagccatgatgaggacactctgcagtataaacttgtaaatgagagcaaaatcagcgaagaagaagcttacaacctgatgaaagtggcagcaacacttcagattaccgcaaaaggtcagccggtgctctattatggagaggagattggacagggtggagccaacaactggccgctccagacaaaccgccgcgactttgactggacagagctggaaaaacagaaagcagacagcaacagtatttacaaccactacaagacaatgcttgcaatccgcaatgcgtacacagatgtatttgcaagaggaaacagaagcacagttgcagtttccgacgcagatggctatgaagtgatcagcagaagttatggaaacaacaccttatatgtaggaatgaatgtgaaagaggcagagaaagaagtagtgatcccggtagcagagagtgccggaacagttcttaaaaacctttatgatggaaaaacttacactgtttctgctgaccggaacgtttctgttaccattccggcagcaaaagatggtggaacgattgttttgacagcggagacaaaaacagaaccggctccggatgaaaaacaggatgataagaagacagatacagcagagagcaatggaaatgcacagtcttccggaaacaacgcaaaccagagcacttctgcaaataagacaactccaaaacaggaagaacaggctgtagcagaagtaaccgtgcaggaggagagttttgcaaatgtgatcgaggcagtgaataaggcaaaaaccggaagtaaaatccgtgtaaatctgttaaagacaacaaagattccagcaaatgtgttcgagagtatcaaaggaaaagatatgaacgtaaccttcaaggtaagtgatcaggccagctggatcatcaatggaaaagatatcaccggtaatgtgacagcaccgatcgatcttggtctggttgtgggaacaagtgatattccaaaacagaaagtgacagcgctggcagacggaaatgaaaccatccagctttccttaaattatgacggagtatttggctttgagggaatattgagactttccgttggcaaggactacagtggaaaaatagcaaatctttattactataatgagacaaccggtaagtttgagtattatcaggcagtacaggtaaaagaagatggtactgtagactttaagttctcacatgcatccgattatgtcatcgtcttaaatgacacagatatgagccagacaacaggcagtgtgatcgcaagtccgaagacttcggataacacaccgatcgcagcagcagtgatattattactgtttggctgtgcgctgatgggaaccgcatacagaaaaaataaacacttctaa

SEQ ID NO: 25 - DNA, 1590 bp, Bifidobacterium sp.
  source: /note="GH43.10-2"
atgatgattacctcaactaatcctatggtctacacggattttcctgatccagacatcatccgggtcgggggcgtgtattacatggccactacgactatgcatttcacacccgggtgcgatattctgcgcagctatgacctagtgcattgggaattcattgcgcacgcattgaatatcgtggcggatacccctgaagaacgtttggaatgtgaaggtgccaacgcctacggtcgaggcatgtgggcgccgtcactgcgttaccatcggggcacctggtatgtgttgttcgccgccaacgatacgcataccagctatctgctgacggcggacgatccatgcggcccatggcgaaagcgtgagcttgacggcttctattacgacagcggactgttctttgacgacgatgatcgagcctatgtcgtacatgggcagtcgacattgcgcatcacggagttgaatcctgaattaagcgggccgatgccgggtgggctcgaccgggtcatcgtgcaggacgatccgcaggctgaccttggttatgagggcagtcacctgtacaagcatgatggacgctattacgtcttcacctgtcacttcccgcaaggcaagggcaaaacagaagcctgcttgatggccgaatccttggatggcgctttcgaagtgcgtgaaattatcgaagacgacctgtccttccacggttacggagtcgcgcaaggcggtatggtggacactccggacggcgactggtatgcattcatgatgcaggaccgcggcggtgtgggacgcgtgccgatactaatgccgatgcggttcggcgaggacggattccccgtcgtcggcgagaacggcaaagtgccgcagtcggtcagcgtgccggctgcaagctgtgccgaacctgtcacgcccatcaacggcagcgaattcatagcccggtataacgccgaaggcggagtcgatgccaactgtctgcagccatactggcagttcaatcacatctcacataacgaatactggtcactgacggaacgtccgggagcattccgcctgcattccggacgcatcagctcgaatctcaatcatgcatggaacacgctgacgcagcgcacgatggggcctgtgacggtggccgaagtcaccgtcgacgcgtcgacattgcatgatggcgacttcgccggattggcggcgttccaaggatgctattcctacatcgcgcttacgcgaaggaacggccgcacgatgctgaccgtccaatacaagccggcgaatgacgattccatcttctccgataatgattgggacagtccagccgtaacggatgcggaaatcatggcggatgcggattgcatgcgcctgcgcgcggtatatgatttcaccgattgcaaggatgaagtgacgttcttctaccgcgatgcggatacgccggaatccgaatggtgtccattggggacagcgcaccggatggtcttcaaaatggatcatttcacaggttgccgtatcggattgttcctgtattcgacaaaagagaccggtggaatcgccgatttttacgactttgcgtattcgacgccggatacgaaggaaagagagcaatga

SEQ ID NO: 26 - DNA, 1140 bp, Bifidobacterium sp.
  source: /note="GH8.0-3"
atgacaaatgcaaccgataccaacaagacattgggcgagtccatgttcgcacagtgcggatatgcccaggacgccatcgataagcgcgtgtcacaggtctggcatgaaattttcgaaggtccgaacaaattctattgggagaacgacgaaggtcttgcctatgtgatggacaccggcaacaacgatgtacgtaccgagggtatgagctatgcgatgatgatcgccctgcaatacgaccgtaaggacgtattcgacaagctgtggggctgggtaatgcgtcacatgtacatgaaggacggtcatcatgcgcattatttcgcatggtcggtcgcgacggacggtacgccgaactcgaatggtcctgcacctgacggcgaggaatatttcgcgatggacctgttcctcgcctcccgtcgctggggtgatggcgaggatatctacgaatattccgcatggggacgcgagatcttgagatattgcgtccataagggcgaacgctacgacggcgagcccatgtggaatcccgacaacaagctcatcaagttcattccggaaaccgagtggagcgatccgtcctaccatctgccgcacttctatgaagtattcgccgaagaggctgacgaagaagaccgtccattttggcatgaggcagccgccgcaagccgtcgctatctgcaggcggcctgcgacgagcagaccggcatgaacgctgaatacgcggattatgacggaaagccgcatgtcgacgagtccaatcattggcatttctattccgacgcctaccgtaccgcggcgaatatcggactggatgtagcctggaacggtccgcaggaagtgctgtgcgaccgcgtcgccgcgctgcagcgattcttcctgacccacgaccgtactagcgtctacgccatcgacggcaccgccgtggacgaggtcgtgcttcatccggtcggattcctggccgcgaccgcgcaaggcgcacttgcggcggtgcattcggcccagcccgacgcggaacataatgcccgtgaatgggtgcgcatgctgtggaatacgccgatgcgaaccggaacgcgtcgctactatgacaacttcctctatgctttcgccatgctggcgttgagcggaaagtatcggtatgaatga

SEQ ID NO: 27 - DNA, 1557 bp, Bifidobacterium sp.
  source: /note="GH51.0-8"
atggttgtctgcattgacccgaacagtacgattggtcgtatcgatccgaaactgcatggccaattcattgaattccttggcgaatgcattgatgaaggtctatgggtgggagaggattccccgatcgaaaacgagcgtggctaccgcaaggccacattggatgctttgcgtgcattgcagccgccggttattcgctggccgggcggatgctatgcggatacctaccattggcgtgacggtgtgggcccgcaaagcgaacgtaaaaccactttcaacgagaatttcgccacctatgagctggacgatcacagcttcggcaccgacgaattcctgcgtttgtgtgaaatgctcggcgctgaaccgtggatcaatatcaacatgctttccggcacagtcgccgaaatgaaggattggatggagtactgcaatcgtgcgcagcccactgatcttgccaaggaacgtgaggctaacggccataaggcaccttacggggtgaaatattgggggatcggcaacgaagtgtgggctggcggcggtaccatgactccgcggacctacctcaatgaataccgcaggttcgcatccgccatgccgagcttcaccaccgatgtgttcgcgccgaccccaatgtatgctattgcgagtggtcctgacggcaacaagccgcgcgaacgcgtgcagtggacccaggatttcttccgtggtcttgccgaatatcgtcagccgaatatcgacggctatgatctgcacttctacaattggaatgtggacaacgatgccgacactcccacccggttcgatgaagacggctggaatgcggtgattgagggatgcctcgaacttgaagatattctgcgtgatcagtggcgtttgatgaatgacggcctggcgcttattcatgagccggaggtggctatggattccaagctcgcgcatgtcgatctaatcatcggcgaatggggcaattggcacaagaccgcattcttcgcacgccctgcgctcaagcagcaggtgaccatgcgtgacgccatcaccaccgcgcttacgttggatctgctgcagcgtaattgcgacaaggtgaccatggcgtgtaacgcgcagaccatcaatgtgcttaactcactgatcttgactgaaggcgatcggaccatccttacgcctaactacgatgtgttcatgatgtataaggcgcatcgtggcatgaccgcacttgatgtggcgcgtaacgattccgaggattctgccgtgtatacgtttgcgtcacgtaatgaggatggcacgcagctgctgattaatctcaccaatgcgcatatgaacgatggtgccgaagtgcggctgcatttgccgtgcggcgctcaggttgattcgatggaaacgcttgcttccgaagatccgcatgattgcaacacagtggagcattcggatctggtgcgcactcatgccgtggacgtggatagtgccgtgagcgtgcacgaatctgccggcggtgccgagctgacggtaacgttgcccgctgcctcggtgagtgccttgcacgtaacgattcgccagcgataa

SEQ ID NO: 28 - DNA, 4095 bp, Eubacterium sp.
  source: /note="GH13.41"
atgagaaagttaaaagaacgctttcacaggaaacatggcgttgtaagccgtatctttagtatggtacttgcacttgctatgattatgaccatggctccggcaatcggtggtgcaaccactgcatatgctgcgagcccgacaatccggttgtatttggacaaaccaagtacatggaatacaccggttgtcaatgtctgggctgccggtgctacggtagataaccatgacgcaggaaatgccaccatttcacaatggggggatcaggaaaaaccaaagcttgcatatgaggaaagttccggactctattatgtagatgtacagagcagtgagtggacaggctttcagtttgttgatgcaggttctactgagaaagctgcaccggagataaagacagaaggagctgcaattgagcagattaagacttttacttctgatacaagcatttattgtttattggatggcaatggaaaatatcagtggtataaggatgcttcaaagaaggaaacattggttccggagtctgtaccaacagaatgtgatctgactattaattataagagcacattaggcgatgatgttgcagcatatatatataaggagactaataagccagcaggtgaatggccgggaaaaaccatgactgcaacagcaggtcatgaaggctggtatacaatgcatctgacattagataacagtacagattattctcttatcttaaatgatgatggacatggaaaccagttaaaagacgtaacactttctacaaaaggaaaggcagaagcagagtactggtttgatggttctttgtcagagacaaaacctgctgattggaaatatgtaacaaccattcattatcttgcttcaggaatgggaagtactatttacaattatatgtggggagcagatgcctctgcaacaggagcaggtgttggaaaagaatggccgggcggacagatttcggcaaatgctgatcatttgggatggtatgatgtagtatatacacaggatgtaaaacagaatttcagctgtatttttaataataacaacggaacacagacggataatattgatgtttctgtgacatcaactagtactgagctctgggttaccggaacaaaaggtgatacaaccgtatataaaacagcaccggacagctgggaggcaccggttccagaccacacatttactatttattattacaatgaggatttatcaacagacacagacatgggaaaagttgatttgtggatgtggaatgccggattagacggttcctatgtttttgacggaacatattatgatgctgaaaataaagtgacatggtttaaacagaccattacagttgccggcagtaatgtaggaaaaacggtaggattaaaggcacgctatgataatacaaaaggatgggatggcggctctgatactgcagatcgttcttttacaataagcggtgatgagaatgaggtattatattatgtggatggttccgatccggttcatgagaaaccggtaatcgtaccaacggaaaagagataccttgtattggattatgagaatccgggattaaaagaaaaaggtattacaccacagttttatacatggtcatcaggatatgcttcagtattaaccgattttacatatgtaggtggagataaatggacagtaacaatcccagcaaaaccatcctgcacaaaggttgatttttgtattgcattagattcaacaggtgacccatggattaaagatggtggagaccattcagttacattcccttctgatcagaaggttatctatgccagcatgaaagccggcagtgagccggaaattgctatgccatataatgttggctatgaagtagatgcagaaaatcaacaggtatcatactactatcgtgatgatgatgcatttgtagatggcaccttaaaggatatgaaagtatctgttgacgtaaacggaacagagtatccaatgacatacaatgatacaacaaagcgttttgagtatgtaaagaatggtttaacaaatggcaaaacacattatcgttacaaagcaaatggaaattatgttgtagatgcattcaattcaaatagtgaaaaatataatgacgcagattactcatattttgaatactataaattaaatgcaacagttacagcagaagttatgaataagtcatttaactacaatgagaataatgtagttaagtttaaggttaaacaggctgatacagatactcagaaacttgaagttgcaagtgcaagtattgatgtttcttcacttggtggaagtagtgagatgccgattgagccagagctccaggctgttacaatttctgcaactgtagatacaacattaggtactaagacattaccaattactgtaacagaccagtatggtaataaattcagtactacagttgatgttgaaattacagaccgtgtgaagaaaaatgaaaatgatttcgactgggatgaagctgttgtctactttatgatgacagaccgattctttgatggtaatgaatctaacaatacagcaagtggtacagatacatacggagacaaccctggactgtatcatggtggagattttgccggtgtaacagctaagttagattacttacaggatttaggagtaaatacaatctggcttacaccaattgtaaagaatattgcaggtgtaactgtgacagatgagggtaaagaagatgttccttataatgcagcataccatggatactgggcaagtgattttacaaaattgaatcctacaatgggtacaacagaagaatttaaaactatgattagcgaagcacataaacgtggtatgcgtattatggttgatattgttgtaaaccatgcaggatatggtacagaatcaacatttgctgatatgcttagggataagagcgtcagtgaaggcgatattaaatcatggcagtctggattgccggattttgcaacagaaaaggcagatgtcagggcaaaattagtagaatggcagacatcatggatgaaggattatggtgttgactatttccgtgtagatactgtaaagcatgttgacagtacaacatgggcagcacttaaaaattctacaacagaagtaaatccgtctttcaagatgattggagaatattatggtgcaggatatgcgtcaaatggtagtaccttaggtagtggtcagatggatgcagatcttgatttcgattttaatgaccaggcaacaagctttgtaagtggcaatatttcttctgtagagaaattcctttctgcaagaaattcagcacttaataacgcatacatgacaggtcagttcttaagcagtcatgatgaagatggatttaaggcttccttaataaacggaaaaggctataccgaggatgaagcaacatcagcagcgttagttgcagctaccttacagcttactgcaaagggtattccggttatctattatggtgaagaagttggtttaagtggattaaataattatccatatcagactaatagatatgacatggatttctctaaggcaacaaaggacaatgtcacatatcagcattataagaatctgcttagcatccgtaatgcatacacagatgtatttgcaagaggaagcagaacagttgtggcaggttctgatgaggaaggctatgatgtagtttcaagatcctatggaggaacaaccttatatgttggtatgaatatcaaggataccgcaaaagaagtaaaagttccggttagcttagcagcaggaacagaggtaaaggatttatacagcggtgctacatatactgtaggaagtgataaaacagttgctgttacaattccggcagcaaaggatggtggaacagtcattcttactgaggtgaagaaaacaaaagacccgggcaagacagatccaacaccggaaaaggtttctgcaacattaattactcttgataagaaaactgcaggtaaacagcagaatgacactaaaaaagcagctccaaagagtggcgatgacaatgaagcagctacatatgtatgcttactcggacttgcaatggttgcaatcacagcagctacatatcgcaagaagagagcttgcaactaa

SEQ ID NO: 29 - DNA, 2265 bp, Bacteroides sp.
  source: /note="GH92.0-5"
atgaaacgtattctattaacttacacacttgctttcgcccttcttcccgtatatgcgggggagggtggaagtccccccgctgataagagtcttccggttgattacgtagatccttttatcggaacgaccaatttcggcacgaccaatcccggagcggtgtgtccgaacggaatgatgtccgtggttccttttaatgtgatgggctcttcggaaaacacgtatgataaagatgcacgatggtggtctactccatacgaatataccaattgtttctttacaggatatgctcatgtcaatctgagcggagtaggttgtccggaattggggtctttacttttaatgcccactaccggagagctgaatgtggattataaagaatacggaagtaaatataaggatgagcaggcttcaccgggttattattccaattatctgacaaaatatagcgtcaagacagaggtttccgctactccacgtacaagtatcgcccgttttacttttccaaaaggcaaaagccatatattgctgaatttaggagagggactgacgaacgaaagtggtgctatgctccgccgtgtcagtgattgcgaggtggaaggcatgaaactgctcggtacgttctgttataatcctcaagctgttttccctatttactttgtgatgcgggttaaaaaagtcccttctgcaaccggctactggaagaagcaacgtccgatgacgggtgtggaagccgaatgggatgcggatcaggggaagtataaactctatacccgctatggaaaagaaatagccggtgatgacatcgggacttatttttcttttgaaacggaagagggagaacaggtagaagtgcagatgggagtttcctttgtgagcattgaaaatgcccggttgaacctgaaccgtgaacaggaaggaaagaattttgagcagattcttgccgaagcgcatgctaaatggaatgacgacttgtcacgtatcactgtagagggcggaacggatgcgcagaagactgtgttttatacggcactctatcatctgctgattcatcctaatatcttgcaggatgccaacggagaatatccggcaatggaaagcgataagattatgacgacaaagggagaccgctatacagtattttctctttgggatacgtatcgcaatgttcaccaattgttgacactggtttatccggaacgccagatggagatggtacgcaccatgttggatatgtatcgtgaacatgggtggttgccgaaatgggaattgtatgggagagagacattgacaatggaaggcgaccctagcattccggtgattgtagatacatggatgaaaggtttgcgtgactttgatgtggagctggcatacgaagcaatgtacaaatcggctacactgccgggagcggacaatctgatgcgtcctgacaatgacgattatctgtcgaaaggatacgtgcccctccgcgaacagtatgacaattcggtatctcacgctttggagtattatattgcagattttgcactttcccgttttgcagaggctttgggtaagaaaaaggatgcggaactgttctataagcggtctttagggtataaacattattatagcaaggagttcggaacgttccgtccgatattgcctgacggtactttttatagtccgtttaatccgagacagggagagaacttcgagccgaatcccggttttcatgaaggcagctcctggaattatacattttatgtgccgcatgatgtatatggactggcaaagttgatggggggcaagaaacgtttcattgacaagttgcagatggtgtttgatgaaggactttatgatcctgccaacgaaccggatattgcatatccttatttgttctcttattttaaaggagaggaatggcgcacgcagaaagaaacgcaacggttgttggataagtattttacaacgaagccggatggtatccccggaaatgatgatacgggaacgatgtcttcatgggctattttcaatatgataggtttctatccggattgtccgggattgccggaatatacattgacgactccggtattcgacaaggtgactattcgcctggatccgaaatggtataaagaaaaggaattagtgattgaaagtaatcgcgcccaaccgggaactctttatatcaataaggtgttactgaatggaaagaaattcaataaatatcgtatcacacatgatgaacttgttcatggtcaacacatatattttgatttgaaatga

SEQ ID NO: 30 - DNA, 1260 bp, Bacteroides sp.
  source: /note="GH8.0-3"
atgaagaacttattttacctcctcctttgcctcatcgccgggacatcgtgcagccaggcagacccgacaaagccctgggataaaggtgcctttgaaacacagaaataccggaatctcctcgccgagatgggctacaaacaggcagatattgatgccaagctcaaatccgtctttgacggtgtattctacggtcccgacaaagtatattttgaagtaggcgactctatggcttacatcagtgacatcaaaaaccatgatgtccgcaccgaaggtatgtcttacggattaatgattgcagtccagttcgaccgtaaagatatcttcgaccgcctttggcgatggggcacaaagtacatgcagcatcaagacggtccgttgaaaggatacttcgcctggagctgcgagacagacggtacccgtaactcccaaggccccgcctccgacggagaactttactatgtaaccgccctcatcttcgcctccaaccgttggggaaacgacaccggcatcaactaccttgccgaagctcggaatatcctgaactgttccatggagaaagatggtacagaccgagtaatgccttttatcaatgtagagcataagctcatcaccttcgtccccgacatacggggcggccttttcaccgatccatcttaccacgtacccgctttctatgaagtatgggcacgctgggccgatgatggcagagccgacttctggcgtgaatgtgccgaatgcagtcgtgaatacctgcataaaagcatccaccccgtaaccggtctgaaccccgattacaacaactatgacggcagcctgctgggcaataaccgcattattggtgatgctttccgcttcgattcttggcgtgtaccgatgaatattgctttagattactcctgggcatgtgccgacaaagagtggcaacaggaatacggcaacaaaatccagaactttctctacagccagggtattgatactttcgtagaccagtacaacatagacggtacacaggtaaaagataccctccgagccggagaacacaaggcgttaagacactctttaggcttagtagccacttctgccgtcgcctcactgatgtgcactcacgagaaaagccgtgagttcgtagacaagttgtggaacgcaaaacacgagccgtatgaagacggatacttcgatgcttactatgacgggctgctccgcctcttcgcttttatgcacctgagtggaaactaccgcatcatcttccctgaaaagtaa

SEQ ID NO: 31 - DNA, 1335 bp, Ruminococcus sp.
  source: /note="GH1.0"
atgagttttcagaaggactttttatggggcgctgcagctgcctcttatcaggtagaaggtgcataccaggaggacggcaaggggttgaatatctgggacgtatacacccgggagccggggcatgtggcgttcaacgagaacggggatgtggcatgcgaccactatcaccggttcaaggaggatgtggcgctgatgaagcagatcggtctgaaggcataccgactgtccatcagctggacacgggtgatccccaacggcaccggagaggtaaatcccgccggtatcgccttctacaacgcactgatcgatgagctgctggcagcaggcatcgagccattggtgaccatcttccactgggactacccctatgccctccactgccggggcggctggctcaatcctgcatcctctgactggtttgaagcatacaccagggtgctggtagacagcttctccgaccgggtacggtactggatgaccatcaacgagccccaggtattcatcacagacggctacaagaacggaaattttgcgccctttatgaagcatccggacggggatctgatccggatgacccacaatgtgctgctggcacacggcaaggctgtccgcaccatccgggcacatgcaaagcgcacgcccatcgtaggctttgcacccaccggtccctgcgtggttcctgcaagcaatgcgccggaggatatagaacgggcacgggcggcatcctttgatttcaacaggaacaactacacctccagcaatgcctggtggggagaccccattgtgctggggcactacagccccagggcatatgaattgttcggggatctgatgccaaaggagaatccggaggaaatggctctgatctcccagaaactggatttctacggtgcaaacatctactggagcatgcaggggggcgaactgggcaccaccctcaccggctgcccgaaaagcaatctggcatggcctctgacgccggatgtgatgtactggtccatccggttcctgcatgagcgctaccagctgccgctgatgattaccgaaaacggcatggctggtcacgactgggtggcattggacggcaaggtgcatgacccggatcggatcgactatctgacccggtatctgcgtagctgcaagcgtgcagtggaggaagggctgcccctgatcggctatatgcactggtccattatggacaactttgagtgggcgcggggctatgaccagcgattcggcctcatccatgtggattacggtacccagaagcgtactctgaaggattccgcctactggtacgcatccgtcattgcggaaaatggcgaaaatctctga

SEQ ID NO: 32 - DNA, 2151 bp, Ruminococcus sp.
  source: /note="GH26.0-1"
atgaattcattcgtaaagcgactgggcagtgccctcactgccagcgcaatgatgctgaccgccggcatcttcgttccggttcaggcagccgacacaggggctgatgcagcgccgctgttcactgccgaagcggaggactgcaccctgctgaccggcgccagcgtcaccaccaatgtgtacggcacggagtatccgggctacagcggagatggtttcgtatgggcagggaacgccggcggcatgacctttgaggtggatgtaccggagaatgccatgtacgagctcaccacaagatgctggatgtacctgggtgatccgggcaccaccagaatgcagaccctggcaattgacggagatgtcaaaagctccatctacattgccaataacgaaaagtgggaggattccagcttcggcttcttttacctggaaaagggcaagcacaccattgaagtgggtgctaccggcagctggggcttcattctctacgacaccgtcacctttgactttgcagatatgccggagctgaacattgcgccggatccctgcgacaaaaatgccactgccgagaccaaggcgctgatgaagtacatgaccggtcagtacggcaaccacatcatctccggtcagcaggagatctacgggggcggcaacaacggggacaccgagctggaattccggtacatctatgagaccacaggcaaataccccgtgatccggggcttcgatttcatgaactacaatcccctctacggctgggaggacggcaccaccggccgtgtcatcaactgggtggcaaactgcggcggcattgccactgctagctggcacatcaacgtgccccaggactttgactcctacaccctgggagatcagctggactggcagaagtgtacctacaagcccacctcctctttcaacactgcaaactgcctggatcctaccacaaaggaatacaaatatctgatgctggcaatcgaggatctggctgagcagctgttaatccttcaggacgcaaatgtaccgatcattttccgtcccttccacgaggctgaaggcaacaacaataccaacggctccggcgcatggttctggtggggttcctccggcgcagaggtatacaaggagctgtggaagctgctgtacaccaccctgaccgaagaatacggcatccacaactgcatctgggaagtaaacctgtacgactatgcaaattctgcacagtggtatccggggaacgactatgtagacatggttgcatacgacaagtacgagggctctccctacacctggaacacctctgctgcaacctctgtctttctgaccctggtgaatgacaccaacgacaccaagatggtagcactggcagaaaacgacgtgatcccggacattaccaacatggtgaatgaaggcgcatggtggtcttacttctgcccctggtacggagatttcatcaccaacggtaccaccaataccaaggaaatgctggacaagatctataacagcgactatgtcgtaacactggacgaggtgcccaatgacctgtacggctatgcacggggcaacggaggcaactggaacgtggaaggtgcctatgagtgcgaggacggcaacatccagaccaacaagggcaccacgaccgttgcttacgattactgctctggtggaaaatatgtgtacctccagggagagggcgactacatcgagcagactgtaaccgtagaaaaggcaggcaagtacgccatccgctatggttatcagcagaactttgagaaaaacggcaagacccagaacctctacgtcaacggtaccgcagttggcgaggctttcttcccctattccatcctgtttggagagagcgatgccatcgtggtagagctgaaggcaggcaagaatacaatcaaggtagaaagcggcgagggctggacatattttgactacctgaccgtaagctatgtgggcgatgacattctcaccggcgatatcaatctggacggcaaactcagcgtcagcgacgtggtacttctccagaagtatctgatcaagagcggtaagctgactgccgatcaggcaaagcgtgccgatctgaacggagacggcgtgctgaatgcatatgacctggctctgctcaagcacaccatgctgggtaaataa

SEQ ID NO: 33 - DNA, 1851 bp, Ruminococcus sp.
  source: /note="GH26.0-2"
atgagaaaacagaaacgccagttgtccgtcctgctggcttctgctgtggcaatgactaccctgctcagctttcccggcggcgcagtatcctccgacacactgaccacctacgagtttgaacagggcgtgatcgaccgtgccaagcagtacgatgcaggctggacagacaccaacgatgcaggcgatacctacgactgtacggatcccaccggcagcggctttgtgtatctgaccgacaagggcagttccgttacctgtacagtggaggtggaaaaagccgggctgtacaatatgaatatccgctatctgcagcccaatgacaccaacaaaaaggtgcagtatctgaacatcaacggctccaatcaaggagaagtcaccttcccctataatctgaagtggagcgagattaccacgctggtcaccctgcgggagggcagcaacagcattgagctgaagggctactggggctatacctacctggacagctttactctgacccaggcggacgaaagcatttctcagctttctcccacggattctctgtccaatcctcacgccaacgacaccacgaagcggctctacgcttacctgcgcagtgtgtacggcaaccacattctttccggtcagcaggaaatgtgcggttcccacaactacaattacaatgcggatcctacctccggattcatcaaggacaatgaggcggagttcacctatatccaggagcagaccggcaagcagcccgccatccggggcattgatttcctcacctatcacctggatgaaaacggggagctttcctaccaggactatgccgcagagcgtgccatcgagtggaccaacaagtacggtggcatcgctaccatcagctggcactggagcgtcccctccagcaccggcaattacgctttctatgtagaatccgccaatgcaaactatacggatttcagcatctctaaagctgtcactgagggcaccaaggagcacgagattatcatgaaggatattgaactagtggcaagcaagtttcagatgctggaggatgcagacgtgtccgtcatcttccgtcccctccacgaggcagagggcgcatggttctggtggggcgctgaaggcccggagccctgcgtcaagctgtaccggctgctgtacgatcagctgaccaatgtgtacggtctggacaatattatctgggaatggacgggctacaccacccccaattcagctgcatggtacccgggggatgatgtggtggatctgattggctatgacaagtacaatgtcagcgacggcatccccaaccccagcgccatcgcctccaccttctatgggctggttgccagcaccaacggacagaaaatggttgccatgtctgagaatgacgcaattccatcattggaaaatctggtaaatgaccgggctgcttggctgtatttctgcccctggtatgggtactacctgaccggagaggtcaacaacccggtggatctgctgaacgagatctacaacagcgaatattgcattacgctggatgagctgccggatatccgcagcttcccgctggatgccccctccaccactgctgcatccaccacaggctccggaacggtcacaaccaccgctaccacaacctccctgtacggggatgtgaacgcagacggcattgtagatattgcagacacggtgctgctggcacggtacatcgcccaggacaatgcagtgaaggtcagcgaggcagggctacagaatgcggactgtgtgctggatggcaacattgacgcatcggatctgaccgccattgctcgctaccttgcccatctgaccgacgcagatcaattggggatcaagccataa

SEQ ID NO: 34 - DNA, 2229 bp, Ruminococcus sp.
  source: /note="GH43.16"
atgaaaaaacgagcatttgcatacgcagcggcggcagcattgtctctgacgctgtgcttcggaacgtatcccgcatcccggctcactgccggatccattgcagaagccgcagaggaggcgagtaccatcgcaaacagtcagatcagcaccaaccagtttaaaaatatcaattacaacaacccgatttccccggcatttttctgtgccgaccccaccgcagtggagtataacggcaggctgtacctgtttggcaccaacgaccaccagcagtttgaggtcaagggctccgaggtggataatacctatgagcagatcaagtctctggtggtgctttctacagatgatatggtaaactggacttatcatggggagattcatgtggatcaggttgctccctggatcaccaactcctgggctccctccattgtttcccgggtggaggatgacggactgacccacttttatctgtatttctccaacaacggtctgggtgtgggcgtgatcaccgcaacggatccgctgggcccctggacggatcccctgggcaagcctctgatttccacttccacccccggactgaatggctgccccaacccttttgacccgggtgcagtgatcgatgagaacggcgtgggctggctgtccttcggtgccggaaaggcacccggcggcacagattatatgcccggctctgcccggatcgtccggctaggggaggatatggtttccttcgacagcgactttcagaacattccggcaccctatttgtttgaggcaagcgagctgaattacatcaacggcacctatgtgtatacctacaatacggattggtcggatcattccaagcagtgggagtacgactgtgatcccccttccggatgcagcatggtgtacatgaccaccaagacccccttggatccggacagctgggttatgcggggcgaatgcttccagaacccggggcagagcggttttgattactccaacaaccacactcacatgcagaagttccgggatcaatactatatgttctatcataccctgatgctgaagcagggtatgggcatcaagggcagctaccgcagcatgcaggtggatcggatcagtgtggatgaggacacagtgaccatcacaaaaaccggcggcacgaaaaagggtgtacagaccatccagggggtagacccctttgcagtgcagaatgccgcttctttaaacaatacagcggatatggtatacaacactgacagcatgcagaacccatacctcattagcgatgcagccggtgcctggagcagcgtccgcagcgtgacctttaccggctccagagtacctgcacagcccacggtggatccggcggactatgtgctgaccaaggtggataccattacatatcagatctccgtgacggatgtggacaaagccactactctgtccatgcatccatccaccaaggcggggacggactgcaccggcacagcggagatcaccggcaccgggaattacaccattacctgtgacatgggtggtgcggaaggtatgttcaacatgggctactttactgcatccgatgatgcgcagatcacctttaccattgataccatgctggtaaacggcacctatgcctttgacctgtccacggagctgaccaatacccgggaatgggcggacggtctgcggaatatctggaacggcttttccgatggggacacggtatacaccggcgaaaatgctgcattccgctacagcaagtctgcggatacaattcagctttataccggagaagcatccggaggaaccggggcaaatgcacctttgctggaggattcggcagtgctgaccgcagaggtacggggtaccggcactatggaggtgcggctggatgcgcctacgggacagctgctgaccagtgtcagctttgatgctccggatgcattcgccaaggtatccggcaaggcatttaccggcatcggcggcacccacgatctgtattttgtgttctccggcaagaatattgcattccgcagctggcaggtggaaagcatcgctgagcggctgatgggggatgtgaatgcggatggcgtatgcagcgtggcagatgtggtagcactgcaaaaatatctcattaagcagacggacacgctggcagattccaaagcaggggactataatggggacggtgtattgaccggcatggatctggtacgtatgaagcgtgcattactcggataa

SEQ ID NO: 35 - DNA, 2175 bp, Ruminococcus sp.
  source: /note="GH43.37"
atgaaactacagaaattgttcaggaaatcggtttctgcattgcttgcaatggtgcttggaacgggaatgctagtcagtccatctgcttgtccggagccaacagcagcggcagttggaaacactatttacaacgatacgttttggaaggacacatccggaaacaacatctattctcagggcggcggcgtatttcaattcggggatacttattactggtacggcgtgcactacaacggcgcagacacatatgccgcaaatccgaccaaaaaggtgaacgatacttcctttcgctctgtgacttgctattcttccaaggatcttgtgaactggaagtttgagaacgatgttctgacggcaaataccaagaattttggctggacctactgggttggacgcatgggcgttgcctactgtgcaaagacgaaaaagtatgtactggtgacccagtacaatgacagcatcctctttgcctcctgtgatacgcctacgggtaatttccaagtggaaaccgtgcaggatcagattcagaatgtgctcaagcaaggcactggggatcagactttgttcgtggatgacgatgggcaggcgtatctggtttgctctaataagggcggcagaggacatcagtatatttccaaactgcggacatcggatttcctgtatgctgaacctgcagtggaagtggcgaagggaaagggcagagaaggtaattgcctgtttaaatacaaggggaagtattatttctgtgcatcggatctgcacggttggaatgcatcccacagctattacatggttgccgacaagatcacaggcccatattcagactggaaggtgatggagggaacggatgaagatttctcctatgtgacccagacgggctttttctacactgtgcatggcagtaagcaggagacagttctgtattgtggcgatcgttggagcgattttgccggaaacggaattggctataaccagtgggtgccactgacggtgaatggtgacaaggtgacattccattccctgagcgaatggagcctgaatgcacagaccggtgaatggcaggtgggcgcaggcaacaattatattctcaaccccacttttgaagcagatcgggtgtcccagactacgcttgcaggctggaaggcatccggcaccggcaacagcaacaaaaagggcggacgtacaggcaactggtgtgcacggcagtggagcgatagcgcatacaaggctactatgacacaggatgtcaagctccccaacggaacctacaccatgcgggcatgggtaagaagtacgggtggtcagaattcggctatgctgtatgtgcggggtgccggcgctgataagattatcaatgtgaatcgaaaaatagacaattgggaagaggtcactatttctgatatccaggtcaccaatggtaccgtacagattggaatttattcagatgccaaggcgggaaattggctgctagtggatgatttttccttggttcgggattcgtctcaaccaccggttgtggaaccggatcccatccccgacgggaagctgatcaagagtctgaacgtatatgacaaggagaatgcaggcgattggtcaattcagtccgggctgaatgttggcagccaggtatttggggatagaacctgtaagtttaccgcagtgccggagcttctgcaggatgcagagtggatccggacagcttgtgattcaaaaaaatatgcgggcgaggaagcatgcttcacggcagcgaaggatctgacagcctatgtggcagtggatacccgggcagagcagaatgcgtcagcatggctcagtggctgggaaaagacgaacatgactttgacggatgacggaaatccggttgtaacatatgtggtgtatcagaaagacgtaaagcaggatgcagcagtgacgctgggtgcgatcaatctgaaccaggctgtgaactatgtggtgctggctgcggagaatacagccgagccggtgatccccggggatgtaaacggggacggcatggtcaacggcatggatcttgcaaggatgcgccgggcattgctgggacagtccctgaaccggaatgccctgcgccgggcagatctgaacggcaccggcagcgtggaaatagcggatgcggttgtgttgacaaaattcctgttaggcggttcaaaaaattag

SEQ ID NO: 36 - DNA, 2256 bp, Ruminococcus sp.
  source: /note="GH43.4"
atgaacactcacacattccatcagaagactgctgcgtttcttgtgtcaagtgcaatgctgatgttcttaggggctgtccccagtctggtaagcacgaaagcagatgccgcttccaacaaatcccgtgtatccgtacatgacccatctgtaatcaagcttgcagatggcagctattacatcattggttcacatcttgctgccgcacgctcaacggatctgcaaaattggacatggacggcaaactcaaattacggcacgaaaaacaccacgtttttccgggatatttacacggatcttgcgaaacctgccggatggtccggcaccagtgaaaattatgacctttccggcaacctgtgggcacccgatattgtctggaatcccgatatgcagaagtattgtatgtacctcagcgtgaatggggacaactggcattcttcaatcgtactttgcacggctgacaacatcgatggcccgtatcaatattccgataccatcgtatactccgggtttgaaaccaatcctgccaatggggcaaaccattatgcaaacacagacgtggaaaaagtcctcggcagtcatccggatcttagccggtatctcaacagcagcggaaagtggaacgccgaatacggcacaaatgcaattgatccctgcacgttctatgatgaagaaggaaatctgtggatggtatatggttcctggttcggcggcatatatatgctggaactggatgaaaagacggggttgcgtgattatacggtgcagtataaaacggaatcttacaatggcgccgtacagtctgatgcgtatatgggcgttcatgttgcaggcggacactggacttccggtgaagggccatacattgaatatatgaagtccccgggtgcagaaaaaggatattattacatgttcctttcctatggtcatttcaacaataagggcggatacaatatgcgtgttttccgcagtgaaaacccacagggaccttatgttgaccagaacggcaattcttcaatttatgcacaagccatggataatattgcaggcaatatcggagaacgccttatgagcaattatcaatggagctgcaatacaaagccaaatacagcacagggacacaactcggcgctgatggacgacgacggcaagctgttttgcatctatcataacaaatttgacgataattatggtgggcatgaagtgcgtgtacaccagatgcttctgaacgaggacggatggccgactgcaaccgcatatgaatactccggcgaaacgctttcagcagacgggcatacaatggaagcaattgtcggcaactatgagttgatctggcacaacccgaatcagaaatttgaaaatgaaaaatccgccgatgtggaaaagccgattcacattacgctgaatgcggatggaactgtcaccggagatattgatgcaacgtggaaaatcacaaagaacggcacgccgtatatgagcttcacctggggtggtgtgacttataaaggcgcatttattgtacaggaggacgaatcggatacgccggtcaggaaaatgacttttactgcaacagggataaacatctgcatctggggcagcaaggaaacggcatataatcctgtggaggatatcgtcaatttgacaccggttgccgatggaacctataccatacagaatgtcaacagtgcgttgtatatgcatgcagacatggatatcaagaatggcagtgcagaacagaatactgatgcacaaatctggaatattaccgcagtggataacgggtggtatacgattcgcaccacacatggcaaggcactgactgttgaaaatgcaagcgctgaaaacggcgcagatattgtgattacagattacatcggcgatgcctcacaaaggttcagatttctggatacaggcggcggacaatatgcgctgctgaccgcagtttcagggggcaattcctgtgcggacgtctacaatatcagtaaggatgccggtgcgaatatctgccagtgggaatactggggcggcgatgggcagaaatttattttagagcctgcagtgccggaaaaaacggtgctcggtgatgtgaatgcagacggcagcttcaacattgcagatgcggttctcctccagaaatggctgcttgcagtgccaaacacagagcttgccgactggaaggcaggagatttttgcgaagatgacaggctgacagtttttgatttatgtctgatgaaacgagctttgattcaaaataaatga

SEQ ID NO: 37 - DNA, 1935 bp, Ruminococcus sp.
  source: /note="GH5.8"
atgagagggaagaaactacttgcatgcgctactgcatgcgcaatgatggctaccgcatctgccgcaggcacctttggtgttatggctgcggatggcctgggcggcttcgcatggtctgccacagaaggataccaggagggtaccaccggcgtgaccaacggtgcggattccgtcacagtcagctttgctgatacggacaacggtacaagcaatgcagctggattttaccacaactttgacggggcagactggtccgagtatgatacgctgagctttacgctgaccaacgaaagcgccagcgacatcagctttgcagcagcagtcaacaccggatcgtcctggaagtggcaccagagcgacaatatcaccgtcagtgccggagcatccaaggatgtgaccctgtatctgaaggcagaggagtggtggtactatgatgcagacacccagaccaattccctggtgacgattgcagacctgtataatgtacagcgtgtcaatatgatgattatgtccaccagcgagactgcaactgtcagcggttctgttactctgaacggctggaagctggagaaatccggaagcggtgaggtggttgagccgaaggatgggttctacgtagacggcacggtactgcgggatgcaaaccagaacgcatttgaaatgcggggcaccaactacgcttacacctggtacaagtgggagggcaacgaagaagccactctcaaggaaattgcggcttacggtgcaaatacagtccggatcgtactgtccgacggtcagcagtataccaagaacacagcaggcgaggttgcaaatctcatcagtctgtgcgaaaagtataagctgattgccgttctggaggttcatgatgtgaccggtaaggatgatgcaaatctgctgctgaatgctgcaaagtatttcagcgagatcaagtccgccctgatcggacacgaggatacggtcatcatcaacattgccaacgaatggcagggtaacaccaacaccagcagctgggagagtgcttacattgccgctgtaaaggagatccgtgacgctggtctgacccactgcatcatgtgtgacgcaggcggttggggtcagggttatgtgaccgttcgggacggcggcagcgcagtgctggcatccgacccggagaagaatgtgatgttctctgtacatatgtatggtaccgcaggcggcaacgctgctacgatcaagagcgtcattgacggcattatgacccggaatctttgcctggtaattggcgagtttggctataagcattccgatggcgaggttgatgaagcatacattatggaatactgtaaggatgtacagatcggctggatggcatggagctggtacggcaacggcagcccggttgagtacctggatatgtcctctgcaaatgccggcggcaccctgtctgctgactggggcgaggttgtagtaaacggcaagaatggctggaaggaaacctctaaggtatgctctgtgtatgcggatgcaccgatcacaactaccaccactgagcctgttgtgaccaccactacaacagaggagactaccacaactacaacggaagcagaaaccacaatggcagaagtaagtaccacgacgactactaccacaacagttgctgagaccagtacagaggctggcgaaaccacaaccactacaaccacccagactgtagctaccctgtacggcgatgtagactgcaacggcgtggtcgagatcaatgatatcgttctgctggctcggtacattgcacaggatcagggtattcccgcaatctccgcagaaggtcttgcaaatgcaaactgcgtccaggatacaaatgtggattcaagtgacctgacgcagatcgcacggtatctggcacatctgattactgctgaggaactggttgttactgatactacaaacaactga

SEQ ID NO: 38 - DNA, 2076 bp, Bifidobacterium sp.
  source: /note="GH42.0-2"
atggaacatagagcgttcaagtggccgcagccacttgcgggcaacaagccccgcatctggtacggcggcgattacaaccccgaccaatggcctgaggaagtgtgggacgaagatgtagccctcatgcagcaggccggcgtcaacctcgtctccgtagccatcttctcctgggccaagcttgagcccgaagaaggcgtgtacgacttcgattggctcgaccgcgtcatcgacaagctcggcaaggccggcatcgccgtcgatctcgcctccggcaccgcatccccgccgatgtggatgacccaggcccacccggagatcctctgggtcgactaccgcggcgacgtctgccagcccggtgcccgccagcactggcgcgccaccagcccggtcttccttgactacgcgctcaacctgtgccgcaagatggccgagcactacaaggacaacccctatgtggtctcttggcatgtgagcaacgagtacggctgccacaaccgcttcgactattccgaagacgccgagcgcgccttccagaagtggtgcgagaagaagtacggcaccatcgacgctgtcaacgacgcctggggcaccgccttctgggcgcagcgcatgaacaatttctccgagatcatcccgccgcgattcatcggcgacggcaacttcatgaacccgggcaagctgcttgattggaagcgtttcagctccgacgcgctgctggacttctacaaggccgagcgcgacgccctgctcgagatcgcccccaagccgcagaccaccaacttcatggtctccgcgggctgcaccgtcctcgactacgacaagtggggtcatgacgtggacttcgtgtccaacgaccattacttctcgcccggcgaggcccacttcgacgagatggcctacgcggcctgcctcaccgacggcatcgcccgcaagaacccgtggttcctcatggaacattccacgtccgccgtcaactggcgcccgaccaactaccggctcgagcccggcgagctggtgcgcgactccctggcccatctggccatgggcgccgacgccatctgctacttccagtggcgtcagtccaaggccggcgccgagaagtggcattccgccatggtgccccacgcaggccccgactcccagatcttccgcgatgtgtgcgagctgggtgccgacctcaacaagcttgctgacgagggcctgctgagcaccaagctggtcaagtccaaggtcgccatcgtcttcgactacgagtcccagtgggccaccgagcacaccgccacccccacgcaggaggtgcgccactggaccgagccgctggactggttccgcgcgctggcggacaatggcctgaccgccgacgtggtgccggtccgcggtccttgggatgagtacgaggccgtcgtgttgccgagcctggccatcctgtccgagcagaccacgcgccgcgtgcgcgagtatgtggcgaacggcggcaagctgttcgtgacctactacaccggtctggtggacgacagggatcacgtctggctgggcggctaccccggctccattcgcgacgtggtgggcgtgcgcgtcgaggaattcgccccgatgggcaccgacgcccccggcaccatggaccaccttgacttggacaacggaaccgtggcgcacgatttcgccgacgtgatcacctccgtggccgataccgctcacgtggtcgcctccttcaaggcagataagtggaccggtttcgacggcgctcccgccatcaccgtcaacgacttcggcgacggcaaggccgcatacgtcggtgcccgtctcgggcgtgagggcttggccaagagcctgcccgcgctgctggaggaactcggcatcgagacttcggctgaggacgatcgtggtgaagtgctgcgcgtcgagcgtgcggacgaaactggcgagaaccacttcgtgttcctgttcaaccgcacccacgatgttgcggtcgtggacgtggaaggcgaaccgctggtcgcctcgctggcccaggtcaacgagtccgagcacacggccgccatccagcccaacggcgtactcgtcgtcaagctgtaa

SEQ ID NO: 39 - DNA, 2133 bp, Bifidobacterium sp.
  source: /note="GH42.0-1"
atgactactcgtagagcatttaggtggccgtccctgctgacggaatccggccgcggcatcgcgttcggcggcgactacaacccggaccagtggcccgaggagacgttggacgaggatatccgtctcatgggtgaggccggcgtgaacgtcgtatcgctggcaatcttcagctgggacaagatcgagccggtcgagggcgcgttcacgttcgagtggctcgaccatgtgatcgacaggctcggcaaagccggcatcgccgtggacttggcctccgctaccgccaccgcgccgctgtggctgtacgaatcccatccagaggtgctgccggtagaccggtatggtcatatcgtcaacgcgggctcacgccagtcgtggcggcccacaagcccggtgttcaaggaatacgcgctgcgcctgtgccgcaaacttgctgaacgctacaaggacaacccgtatgtgaccgcctggcacatgggcaacgaatacggctggaacaaccgctacgactactccgacaacgccttggccgcgttccgcacgtggtgcgaggccaagtacggtaccatcgacgcgttgaacgaggcgtggggcacggccttctggtcgcagcacgtgaacagtttcgacgaggtgttgctgccgcgtcacatgggcggcgatgccatggtcaacccgccgcagcagctcgactatgagcggttcggcaacgacatgctgctcgacttctacaaggccgaacgtgacgctatcgagcagatctgccccggcaagccgttcaccacgaacttcatggtctccaccgaccagtgcgtcatggactacgccaaatgggccggcgaggtggacttcgtgtccaacgaccactacttccatgaaggcgaatcccacttggacgagctcgcctgctcggacgcgctcatggactccctcgcgctgggcaagccgtggtacgtgatggagcactccacctcagccgtgcagtggaagccgctcaacgcgcgcaaacgggccggcgaacttatgcgcgactccctggcccacgtggccatgggcgccgacgccatctgcttcttccaatggcggcagtccgtgtccggcgccgaggcgttccactccgccatgctgccccacgcgggcgccgacacgaaggtcttccgcggcgtatgcgagctcggcaaggcgctgaagaccctctccgacgccgggctgcagggcactgagctcgagcgtgccggcacggcgatcctgttcagcgcggaatccgaatgggccacacgctccgaaaccctgcccagcatgaaactcaaccattggcacgacgttcgcgactggtaccgcggcttcctggatgccgggctgcgcgcggacgtggtgccgctcgcctacgactggactgactacaaaaccatcgtgctgcccaccgtgctcagcctgtccgacgaagacgttcgccgtatcgccgacttcgcgaaggccggcggaaccgtcatcgtcggctacgccactggcctggtcgacgagtacttccacatcgggctcggcggatacccaggtgccggcaatggcctcctacgcgacatgctcggcatccgcagcgaagaattcaacatcctcggtgaagaagccgaaggcgagcccagcgaaattagcctgtccaacggtctgacgacccgcctgtggcagaacgacgtgacttccgtagccgcggacaccacagtgctcgcctcttacacaggtgagtccgccgccgactgggagctggagcgcacccccgccatcaccagccacccctatggcaacggtaccgccatctacgtgggctgcgaccttaaccgtcacgacattgcccagctgctcaaagcacttggctcccgctggcgggagctgtcggcgcagccgactgagggtggtcaaactccaacctatcccaccacagatccccgcatcctgcacaccatccgccgatccgcagacggctccacccgcttcgatttctacctcaaccgctcaaaccagcccgtcgccatcaacggtgtggaaggtgatcccatcatcgtccaccgttgcgagactgacgccgttggatatacgctgaaccgcaacgccattcttatcgctaaaacgtcctgctaa

SEQ ID NO: 40 - DNA, 1590 bp, Bifidobacterium sp.
  source: /note="GH43.10-1"
atgatgattacctcaactaatcctatggtctacacggattttcctgatccagacatcatccgggtcggggacgtgtattacatggccactacgactatgcatttcacacccgggtgcgatattctgcgcagctatgacctagtgcattgggaattcattgcgcacgcattgaatatcgtggcggatacccctgaagaacgtttggaatgtgaaggtgccaacgcctacggtcgaggcatgtgggcgccgtcactgcgttaccatcggggcacctggtatgtgttgtttgccgccaacgatacgcataccagctatctgctgacggcggacgatccatgcggcccatggcgaaagcgtgagcttgacggcttctattacgacagcggactgttctttgacgacgatgatcgagcctatgtcgtacatgggcagtcgacattgcgcatcacggagttgaatcctgaattaagcgggccgatgccgggtgggctcgaccgggtcatcgtgcaggacgatccgcaggctgaccttggttatgagggcagtcacctgtacaagcatgatggacgctattacgtcttcacctgtcacttcccgcaaggcaagggcaaaacagaagcctgcttgatggccgaatccttggatggcgctttcgaagtgcgtgaaattatcgaagacgacctgtccttccacggttacggagtcgcgcaaggcggtatggtggacactccggacggcgactggtatgcattcatgatgcaggaccgcggcggtgtgggacgcgtgccgatactgatgccgatgcggttcggcgaggacggattccccgttgtcggcgagaacggcaaagtgccgcagtcggtcagcgtgccggctgcgagctgtgccgaacctgtcacacccatcaacggcagcgaattcatagcccggtataacgccgaaggcggagtcgatgccaactgtctgcagccatactggcagttcaatcacatttcacataacgaatactggtcactgacggaacgtccgggagcattccgcctgcattccggacgcatcagctcgaatctcaatcatgcatggaacacgctgacgcagcgcacgatggggcctgtgacggtggccgaagtcaccgtcgacgcgtcgacattgcatgatggcgacttcgccggattggcggcgttccaaggatgctattcctacatcgcgcttacgcgaaggaacggccgcacgatgctgaccgtccaatacaagccggtgaatgacgattccatcttctccgacgatgattgggacagtccagccgtaacggatgcggaaatcatggcggatgcggattgcatgcgcctgcgcgcggtatatgatttcaccgattgcaaggatgaagtgacgttcttctaccgcgatgcggatacgccggaatccgaatggtgtccattggggacagcgcaccggatggtcttcaaaatggatcatttcacaggttgccgtatcggattgttcctgtattcgacaaaagagaccggtggaatcgccgatttttacgactttgcgtattcgacgccggatacgaaggaaagagagcaatga

SEQ ID NO: 41 - DNA, 1140 bp, Bifidobacterium sp.
  source: /note="GH8.0-1"
atgacaaatgcaaccgataccaacaagacattgggcgagtccatgttcgcacagtgcggatatgcccaggacgccatcgataagcgcgtgtcacaggtctggcatgaaattttcgaaggtccgaacaaattctattgggagaacgacgaaggtcttgcctatgtgatggacaccggcaacaacgatgtacgtaccgagggtatgagctatgcgatgatgatcgccctgcaatacgaccgtaaggacgtattcgacaagctgtggggctgggtaatgcgtcacatgtacatgaaggacggtcatcatgcgcattatttcgcatggtcggtcgcgccggacggtacgccgaactcgaatggtcctgcacctgacggcgaggaatatttcgcgatggacctgttcctcgcctcccgtcgctggggtgatggcgaggatatctatgaatattccgcatggggacgcgagatcttgagatattgcgttcataagggtgaacgctacgacggcgagcccatgtggaatcccgacaacaagctcatcaagttcattccggaaaccgagtggagcgatccgtcctaccatctgccgcacttctatgaagtattcgccgaagaagctgacgaagaagaccgtccattttggcatgaggcagccgccgcaagccgtcgctatctgcaggcggcctgcgacgagcggaccggcatgaacgctgaatacgcggattatgacggaaagccgcatgtcgacgagtccaatcattggcatttctattccgacgcctaccgtaccgcggcgaatatcggactggatgcagcctggaacggtcctcaggaagtgctgtgcgaccgcgtcgccgcactgcagcgattcttcctgacccacgaccgtactagcgtctacgccatcgacggcaccgccgtggacgaggtcgtgcttcatccggtcggattcctggccgcgaccgcgcaaggcgcacttgcggcggtgcattcggcccagcccgacgcggaacataatgcccgtgaatgggtgcgcatgctgtggaatacgccgatgcgaaccggcacgcgtcgttactatgacaatttcctctatgctttcgccatgctggcgttgagcggaaagtatcggtatgaatga

SEQ ID NO: 42 - DNA, 2808 bp, Blautia sp.
  source: /note="GH36.0"
atggcaattatatacaatccaaataaaagaatatttaacctgcatacggtgcatacaacttatcagatgcaggtcgatccactgggatatctgctgcatctgtactatggagctaaaacaaacagccccatggattatgttttaacctatgcagaccgtggattttccggaaatccttatgcagtgggcatggaccgcacctattcgctggatgcgctgccacaggagtatccttccattggaactggggattaccgcaatattgcgctgaatatcaaaaatgaaaaaggggtggaaagcgcagagctgctttttaaaagttatgagatccgaagcggcaaataccagttacagggacttccggctgtctgggcagacaaagaggaagcacagacactggaaattgtccttgcagacgaaaacgcacaggttgaagttcatctgctgtatggtgttttggaagaaaacgatgtcattacaaggagcgtccagattaaaaatacgggaactgggcagattacgatcgaaaaggcagcggcagcctgtctggattttgtacagggagattttgatgtcctgcggttttatggaaagcatgccatggagcgcaatctggagcgtacgccgctggggcatggaaccattgcgtttggcagccgcaggggaacgtccagccatcagtataatccggcagtgattttggcagaaaaaggaacaacagagaccgcaggcagctgctatggaatgctgtttgtatacagcggaaatttctcctgtgaggcagaaaaagatcagttcaaccagacgcgcctgcttctcggattaaatgaagaactgttttcctatccgcttgcggaaggagaaacctttacggtaccggaagtcattttgtcttattcggcagacggattgtctgcactgtcgcagcaatatcataactgcatccgcaaccatgtgtgccgcagcaaatatgtccatatgcagcgtccggtgctgattaacagctgggaggcagcatatttcgattttacgggagatacgatcgtggatctggcaaaagaagctgcttcccttggaattgatatggtagtgatggatgacggctggtttgggaaaagaaacgatgataattcttcccttggggactggcaggtcaatgaaaagaaactggggggaagcctggcagagcttattacccgtgtgcataatcagggggtgaaatttggtatttggattgagccggagatggtcaatgaagacagcgacctttaccgggcacatccagactgggcaattcagattccggggaaaaagccggtgcgctcgagaaaccagttactgcttgatttttccagaaaagaagtgcgcgactgtgtatttgatcagatttgtgccgtgctggatcagggaaaaattgattatgtcaagtgggatatgaaccgcagtatggcagatgtctatgccggaaatctttcccatgattacgtccttggtgtctatgattttatggagcgtttgtgcagccggtatccggatcttttgctggaaggatgcagcggtggcggcggcagatttgacgcaggaatactttattattcccaacagatctggtgcagtgacaataccgatgcgattaaccgcacaagaatccagtacggaacgtcgtttttctatccggtttccgcgatgggagcgcacgtttcggcggtgccgaaccaccagaccggacgggtgacaagtttccacacccgcggggtgacggcgatggcgggaaccttcggttacgaattaaacccagcgcttttatccgatgaggaaaagcagcagatccgggagcagatcaaaacgtataagaagtacgaaatgctcattaacgagggaacctactggcggctgtctgatccgtttacagatgaaattgcggcatggatgtcggtatcagaggaacaggatcatgcactggtaagtgtggtgcgtcttatggctgaggcaaatcaggcgaccgtttatgtccgcctgcgtgggttaaaaccggatgctgtgtatctggaagaacaaagcggcagacagtattccggtgcggcactgatgcatgcgggaattccgcttccgccgtttaccgaggaatatgaggcgtatcagtttgcctttaccgaactgaaagaggcgggaagattatatgaaaaagtgcagaaatggtgtgacgggaatgccgaaaaccgggtggtcatcagcatttacggtggctccggttccggaaaaacaacgcttgcaacggcattgcagcagtactttttaaatgacggaaccggatgttatctgctctcgggcgatgattatccacaccggattccaaaacgcaacgacgaagaacggctgcgtgtgtataaagaagcaggggaagacggactgcgtggatatctcggaacaaagaaagagattgatttcgcccggatcaatgaagtgcttgcggcatttcatgagggaaaagatacgatcacgttgcggcatttgggacgggaagatggcgagatttcatcagaagaaaccgatttttccggaatatctgtattgcttctggagtggacgcacggaggcagtgacgatttacatggtgtggatctatccgtctttctggaaagttccccggaggagacaaaggagcggcgcatccgcagaaaccgcgacgagaatgccgcaagcccgtttatctgtcgtgtggtggaactggaacaggaaaaactcgaagtgcagcgcaaaaatgcaggattgatcgtgggaaaggacggaagtatttatgaacagtaa

SEQ ID NO: 43 - DNA, 2523 bp, Bacteroides sp.
  source: /note="GH2.0-3"
atgattgggaaactgaaatatttgatactggggagctgtctgatgctgttgggagcatgtaacagttcttcccccatttctccacgcgagcggtctgactttaatgcggattggcgtttccacttaggagacggactacaagctgcacaacccggttttgccgacaatgactggcgggtattgaatttgcctcatgattgggcgattgagggagactttagccgtgaaaatccttccgggacagggggaggggcgcttccgggtggagttggatggtatcgcaaaacttttagtgtagacaaagcagatataggaaagatcttccgcattgagtttgacggagtatatatgaattcggaagtattcatcaacggtgtttcgttaggagtgcgtccttatggatatattagtttcagctataatctgaccccttatctgaaatgggatgaaccgaatgtgttggctgtgcgtgtagataatgccgaacaacccaattcacgttggtattcgggttgtggcatttaccggaatgtatggctaagcaagactggtccgatacacgtagccgattggggaacgtatgtcacgacatcatcggttgacaagggagaggctgtactgaatcttgttactactattgtgaatgaaagtgatacaaatgaaaatatcacggtctactcatccttacaggatgctgaaggcagagaagttgctagaacgcagtcggccggaaaaacggaaactggcagagaagctgttttcacccagcaattgactgtaaaacaaccggagctgtgggatgttgatactccttacttgtatacattggttaccaaagtgatgcgaaacgaggaatgtatggataggtatacgactcctgtcggtatccgtaccttcagttttgatgcccggaaaggatttacattgaacggtaggcaaaccaagattaacggggtatgtatgcaccatgatctgggctgtctgggggcagctgtcaacacacgtgccattgaacggcaattgcagattctgaaagaaatgggatgcaacggcatacgttgttcccataatcctcccgcacccgaactgcttgatttctgtgatcgtatgggatttatcgtgatggatgaggcttttgatatgtggcggaagaaaaaaacagcacataattatgcccgttacttcaatgaatggcacgagcgcgatttgaatgactttattttgcgtgaccgcaatcatccttctgtctttatgtggagtatcggtaatgaagtcctcgaacaatggagtgatgctaaagcggatacattgagtctggaagaggccaatttgatcctgaattttggacattcttctgaaatgttggcaaaagaaggagaggagagtgtcaactctttgctgacgaagaaattggtaagctttgtaaaagggcttgattctacccgtcctgtcactgccggatgcaatgaaccaaattccggcaatcatttattccgttccggtgcactggatgtgattggctataattatcataataaagatattcctcatgttccggctaattttccggacaagccctttatcattactgaaagtaattcggcattgatgacacgtggatactaccgtatgcccagtgaccggatgtttatctggcccgagcgttgggataaaccctttgctgattctacttttgcctgttcatcttatgagaactgtcatgtgccttggggaaacactcatgaagaaagtctgaagttagtcagagacaacgactttatcagcgggcaatatgtatggacaggatttgattatatcggagaaccgactccttacggatggcctgcacgtagttcattctttggtattgtcgatctggcaggtttcccaaaagatgtctactatctatatcagtcggaatggacagataaacaagtattgcatcttttcccgcattggaactggactccggggcaggagattgatatgtggtgctactataatcaggctgatgaagtggaattgtttgtgaatggaaagtcgcagggagtgaaatgtaaagatgctgataacctgcatgttgtttggcgtgtaaagtttgaaccgggaacggtgaaggtcgtttcacgcagaaaggatgaagtgatagcagaaaaggaaattcgtacagccggaaagcctgcagaaattcgcctgactcctgatcgtccagttctggctgctgatggaaaagatttgtgtttcgtcactgtagagatgctggatgaagaagggaatctttgtccgaatgcagataatttggtgaatttcacagtgaaaggtaatggtttcatcgcaggagtggacaatggaaacccggtatcgttggaacgctttaaggataaaaagaggaaagcattttatggaaaatgccttgttgtaattcagaatgatgggaaaccgggaaaaacggagctgacagctacttcggaagggcttcggcaagccgtggtaaaggtctcggcaaaagattgtaaactgtaa

SEQ ID NO: 44 - DNA, 2523 bp, Bacteroides sp.
  source: /note="GH2.0-4"
atgattgggaaactgaaatatttgatactggggagctgtctgatgctgttgggagcatgtaacagttcttctcccatttctccacgcgagcggtctgactttaatgcggattggcgtttccacttgggagacggactacaagctgcacaacccggttttgccgacaatgactggcgggtattgaatctgcctcatgattgggcgattgagggagactttagccgtgaaaatccttccggcacagggggaggggcgcttccgggtggagttggatggtatcgcaaaacttttagtgtagacaaagctgatataggaaagatcttccgcattgagtttgacggagtatatatgaattcggaagtattcatcaacggtgcttcgttaggagtgcgtccttatgggtatattagtttcagctataatctgaccccttatctgaaatgggatgaaccgaatgtgctggctgtgcgtgtggataatgccgaacaacccaattcacgttggtattcgggttgtggcatttaccggaatgtatggctaagcaagactggtccgatacacgtagccgattggggaacgtatgtcacgacatcatcggttgacaagggagaggctgtactgaatcttgttactaccattgtgaatgaaagtgatacaaatgaaaatatcacggtctgctcatccttgcaggatgctgaaggcagagaagttgccggaacacggtcggcaggaaaaacggaaactggcagagaagctgttttcgcccagcaattgactgtaaaacaaccggagttgtgggatattgatactccttatttgtatacattggttaccgaggtgatgcgaaacgaggaatgtatggataggtatacgactcctgtcggtatccgtacatttagttttgatgcccggaaaggatttacattgaacggtaggcaaaccaagattaacggggtatgtatgcaccatgatctgggttgtctgggggcagctgtcaacacacgtgccattgaacggcaattgcagattctgaaagaaatgggatgcaacggcatacgttgttcccataatcctcccgcacccgaactgcttgatctctgtgatcgtatgggatttatcgtgatggatgaggcttttgatatgtggcggaagaaaaaaacagcacatgattatgcccgttacttcaatgaatggcacgagcgcgatttgaatgactttattttgcgtgaccgcaatcacccttctgtctttatgtggagtatcggtaatgaagtcctcgaacagtggagtgatgctaaagcggatacattgagtctggaagaggccaatttgatcctgaattttgggcattcttctgaaatgttggcaaaagaaggagaggagagtgtcaactctttgctgacgaagaaattggtaagctttgtgaaagggcttgattctacccgtcctgtcactgccggatgcaatgaaccgaattccggcaatcatttattccgttccggtgcactggatgtgattggctataattatcataataaagatattcctcatgttccggctaattttccggacaagccttttatcattactgaaagtaattcggcattgatgacacgtggatactaccgtatgcccagtgaccggatgtttatctggcccgagcgttgggataaaccctttgctgattctacttttgcctgttcatcttatgagaactgtcatgtgccttggggaaacactcatgaagaaagtctgaagttagtcagagacaacgactttatcagcgggcaatatgtgtggacaggatttgattatatcggagaaccgactccttacggatggcctgcacgtagttcattctttggtattatcgatctggcaggtttccccaaagatgtctactatctatatcagtcggaatggacagataaacaagtgttgcatcttttcccgcattggaactggactccggggcaggagatcgatatgtggtgctattataatcaggctgatgaagtggaattgtttgtgaatggaaagtcgcagggagtgaaatgtaaagatgctgataacctgcatgttgtttggcgtgtaaagtttgaaccgggaacggtgaaggtcgttgcacgcagaaaggatgaagtgatagcagaaaaggaaattcgtacagccggaaagcctgcagaaattcgcctgactcctgatcgttcagttctggctgctgatggaaaagatttgtgtttcgtcactgtagaggtgctggatgaagaagggaatctttgtccgaatgcagataatttggtgaatttcacagtgaaaggtaatggtttcatcgcaggagtggacaatggaaacccggtatcgttggaacgctttaaggataaaaagaggaaagcattttatggaaaatgccttgttgtaattcagaatgacgggaaaccgggaaaaacggagctgacagctacttcggaagggcttcggcaagccgtggtaaaggtctcggcaaaagattgtaaactgtaa

SEQ ID NO: 45 - DNA, 1260 bp, Bacteroides sp.
  source: /note="GH8.0"
atgaaaaacttactctacctcctcctctgcctcatcgccggaacatcgtgcagccaggcagacccgacgaagccttgggacaaaggggctttcgaaacacaaaagtaccggaacctcttcgccgaaatggggtataaacaagcggatatagacgccaagctcaaatccgtcttcaacgatgtattctatggccccaataaagtctactttgaagtaggcgattctatggcttacatcagtgacatcaaaaaccacgacgtacgcaccgaaggcatgtcctacgggctgatgattgccgtccaattcaaccgccaggacatcttcgaccgcctttggagatggggcagtaagtacatgcagcatcaggacggcccgttgaaaggttacttcgcctggagttgtaaagtggacggaacccgtaactctcaaggtcccgcctccgatggggagctttattacgtcaccgctctcatcttcgcctccaacctctggggaaacaacaccggaatcgactaccttgccgaagctcaaaacatcctgaactgctccatggagaaagacggaaccgaccgcgtgatgccattcatcaacctggagcataaactcatcaccttcgttcccgacatacgcggcgggctctttaccgatccgtcctatcacgtccctgccttctacgaggtatgggcacgctgggccgatgatggcagagccgacctctggcgggagtgtgccaaacgcagccgtgaatatctgcacaagagcatccaccccataaccggactaaatcctgattacaacaactacgacggaaccctgctagacaacaaccgtatcatcggtgacgcctttcgcttcgactcttggcgcgtgcccatgaacatggctttagactactcctgggcctgtgctgataaagaatggcagcaggaatatggaaataagattcagaatttcctctacagtcagggcatcgacactttcgtggatcagtataatgtgaacgggacacaagtaagagataccctcggagccggagggtataaggcactgaggcactcattaggtcttgttgccacttccgccgccgcctcactgatgtgtacgcacgagaagagtcgggagtttgtaaataagttatggaatgccagacacgagccttatgaggatggttatttcgatgcatattatgacgggctgctccgtcttttcgccttcatgcatctgagtgggaattaccggattattttcccggaagaataa

SEQ ID NO: 46 - DNA, 1077 bp, Bacteroides sp.
  source: /note="GH43.10-1"
atgattatgctgaaaacaaaaatcaacactattctgctgtgtattctttttacattgttcttcccgctatcagccggagcacaataccgtaatcctattctttatgctgacgttcccgatatgtcggtgtgtcgcgcaggcgattacttttacatggtttctactactatgcacctgatgccgggagcgcctatcatgcgttcgccggacatgaaacattgggaaactatcagctacgtatttccccgcattgacgatggtccccgttatgatctgctcgaaggtactgcttacgggcaaggacaatgggcatcatctatccgctatcatgacggtaaattctatgtatggtttacagccaatggtgcgcccggacgtgggtttgtctatactgcgacagatccggccggtccctggaaacttctttcgcgccccccgcatttccatgacggttcgcttctgtttgatgatgacgggcgggtgtatctctttcacagtacgggacagcttacggagttgaaacctgatttgaccgatgtacttcccggtggcatcaatcagcaaatatttgaacgggatgctgacgaacaaggtctgttggaaggtagttctgtcatcaagcataatggaaaatattacttgctgatgatttctatggattggagtattcccggccgtctgcgtcgtgaagtatgttatcgtgccgataagattaccggaccttacgaaaagcgtgtcattcttgaaacagagttcgacgggcatggcggtgttggtcagggatgcatcgtagacgggaaaaacggtgaatggtacggactgatttttcaggatcgtggtggcgtagggcgtgtgccgtgtcttatgccttgtacatggacggaagatggttggcctatgctgggagacaaggatgggcacattccgaatgataccactttatcgtatatgtcaatggatggtatctgcggttcggatgatttttccgcttccgggcttccctctattggcagtggaatcataaccccgtcgatcaggcatggagccttaccgaccgtcccggatttctgcgtttga

SEQ ID NO: 47 - DNA, 2859 bp, Bacteroides sp.
  source: /note="GH31.0-4"
atgaatatgaaaaacattttctgttgcctgttgccgggacttcttttcggagcatgtgccaataaggtctatgaggaagcaggcgacagcgtgatagttaaagtacaacaggaagtaacgggaggtccccgactggttcgtctgcaagtgatgggagataaattaatccgtgtttctgctactgccgacagcaagtttgccgatccgcaaagtttgattgttgttccgcaggaaaaacaaatcccatttgccgtcatgcagaatggcgatacgattacagtgtctacagaagaagtgaaagcgtccgtactggccagtaccggagaggtgtggtttgtggataaagacggaaagttaatcctgcaggaaaacaagggaggaggaaagaagtttactccaatcgaagtagaagggacaaagggatatacgatctgtcaggtttttgaatctcctgaagatgaagcgttctacggattggggcagcatcaggcggatgaatttaattataagggtaagaacgaagaactgttccaatacaatacgaaagtctctgttccattcgttgtttcaaataagaattatggtatactgctggatagctattcattgtgtcgtttcggtaatccgaatgactactcccaattgaaccgggtctttaagctttatgataagacaggtcgggaaggtgcgcttaccggtacttatgtgccgaaaaaaggagagacgttggttcgccgggaagactccatttattttgagaatctgaaaacgattcagaatcttccggagaaattgccgttaatgggggctaaggtcacttatgaaggcgaaatagaacctgctcaaacaggagaatttaagtttattctttattacgccggatatgtcaaggtctatttgaataatgaaccggtggtgccggaacgttggcggactgcatggaatcctaatagctataagtttgctgttcatctggaagcagggaaacgtgtgccgttgaaaatcgaatggcagcctgatggtgggcagtcttattgcgggctgcgggcattgactcctgtagatccggcagaacagggaaaacagtcatggtggagcgagatggcaaagcagcttgattattattttgtggttggtgaggatatggatgaggtaatcagtggctatcggactctgaccggaaagtcacctgttatgccgaaatgggcaatgggtttctggcaaagtcgggagaagtataatacacaagatgaaatgttgggcgctctgaaaggtttccgtgatcgtaaaatcccggtggataatatcgtactggattggaatcactggccggaaaatgcctgggggagtcatgagtttgataaggcacgctttccggatcccaaagcaatggtcgattccattcatgctatgcatgggcgtatgatgatttcggtgtggcctaagttctatgttactaccgaacatttcaaggagttcgacaagaatgggtggatgtatcagcagtctgtcagggatagcttgaaagattgggtaggtcccggttaccattatggtttttatgacgcttatgatccggatgcacgtaaactgttttggaagcagatgtatgagcactattatccgttgggtatcgatgcctggtggatggatgccagcgaaccgaatgtacgtgactgtaccgacttggaatatcggaaggctttgtgcggacctacggcgttgggttcctctacggaatttttcaatgcttatgcactgatgaatgcagaagccatttatgacggtcagcgcggagtggataataataagcgtgtgttcttattgacccgttcgggatttgccgggttacagcgttattctacagctacatggagtggagatatcggtacacgttgggaggatatgaaggcacagatttctgccggactgaattttgccatgagtggaataccttactggacaatggatattggcggcttttgtgtagagaaccgttatgtagcgggacagaagcaatggaatgcgacaaagacagaaaatgccgattataaagaatggcgtgaattaaatgcccgttggtatcaattcggtgcattcgttcctctgtatcgtgcacatggacaatacccgttccgtgaaatatgggagattgctccggaagggcatccggcctatcaatcggttgtttattataccaagctacgctacaatatgatgccgtatatttattcgttggcaggcatgacctggtttaatgattatacaatcatgcgtccattagtcatggattttacagcggatacccaagtgaataatattggtgaccagtatatgttcggtccttcatttatggtatctccggtttatcgatatggtgaccgtagtcgtgagatttatttcccccaggcagaaggctggtatgatttttattccggtaaattccagcccggaggagagagaaaagtaatagaggctccttatgagcgtatcccgctgtatgtgcgtgcaggcgctatcgtaccgttcggagatgatattcagtatacggatgaaaaaccggcggatcatatccgtttatatatttatcagggggctgatggagagtttacgctatacgaagatgagggggtgaattataactatgaacagggtatgtacgccatgataccgatgaagtatgatgaggctactaagactttagtaatcggtgaacgccagggagaatttccgggtatgttgaaggaacgtactttcactgtagttacggttaataaggagaaagcacaaccgtttgatttgaatgcgaaaggagtgactgtgaagtataatggcagcgagcagacattgaaactgtaa

SEQ ID NO: 48 - DNA, 2358 bp, Bacteroides sp.
  source: /note="GH3.0-4"
atgaaaagcattaagaaaatggtattagtatcagcctttgccggtacctgccttacaactcacgcgcaggctaaccctcccgccatcccagccgatccggctattgaagctaacatccggcaatggcttcagagaatgaccctcgaacagaagatcggtcagatgtgtgaaatcaccattgatgtggtgtctgaccttgaaaccagccgtgagaaaggattctgtctaagcgaggcgatgctcgacacggttatcggtaaatataaggtaggctcactactgaatgtccctctgggagtagcacagaagaaggagaagtgggcggaagccatcaagcagatacaggagaaatcaatgaaagaaatcggtatcccgtgcatctatggagtagaccagattcatgggacgacctacacgctggacggaacaatgtttccgcaaggtatcaacatgggagccactttcaaccgggaactgacaaggaaaagtgccgaaatatctgcctatgaaaccaaagcagggtgcatcccctggacgtttgccccggttgtcgatttaggtcgtgacccgcgctgggcacgtatgtgggaaaactatggagaagattgttatgtaaatgcagaaatgggcgtgtcggccgtaaagggatttcaaggagaagacccgaaccgcatcggagcataccatgtagctgcctgtatgaagcactatatgggttacggtgtacccgtttccgggaaagaccgtactccttcttccatctcacgcagcgatatgcgtgaaaaacacttcgctcctttcctggctgccgtgcgtcatggtgcattgagcgtgatggtgaattctggcgttgacaacggcctgccttttcatgccaaccgtgaattactgaccgaatggctgaaagaagacttgaactgggacggtctgattgtaacagactgggcggacataaacaatctctgcacacgggatcatattgctgccaccaagaaagaagccatcaagattgccatcaatgccggaatcgacatgtcaatggttccttatgaagtgagtttctgcgattatctgaaagagttggttgaagaaggagaggtatctatggaacgcatcgacgatgcagtagcccgtgtgttgcgtttgaaatatcgtctgggattattcgacaatccgtattgggacattaagaagtatgacaagttcggttctaaggaatttgcggccgttgccctccaggctgccgaagaatcggaagtgttattgaagaatgacgcacataccctgccgatagcgaaaggcaaaaagattctgctgaccgggccgaacgcaaactccatgcgttgcctgaatggcggatggtcgtatagctggcagggacacgttgccgatgattacacgcaggcatatcatacaatctacgaggctttgtgtgagaaatacggaaaagagaatattatctacgaaccgggagtcacctatgctccttacaaaaacgataactggtgggaagaaaacaaaccggaaattgaaaaaccggtagcagcggcagcacaggcagatattatcatcgcctgcattggcgaaaactcttattgcgaaactcccggcaacctgacggatcttaccttatcggaaaatcagcgcaatctggtaaaagctctggccgctacgggtaaacctatcgttttggttctgaaccagggacgtccgcgtattatcaatgacatagagcctttggcaaaagctgtcgtcaacatcatgctgccaagcaattacggtggcgatgcacttgctaacttattggccggtgatgccaacttcagtggaaaaataccgtttacttatccccgcctaatcaacgctttggcgacttatgactacaagccttgtgaaaatatggggcaaatgggaggtaactacaattatgattcggtgatggatattcaatggccgttcggcttcggattaagctataccaattataaatataataacctaaaagtaaacaaaccgactttcaatgccgatgatgagctgatattcacgattgatgtaaccaatacgggcaaagttgccggaaaagaaagtgtgttgttattctctaaagacttggtggcaagcagtacaccggacaatatccgtctgcggaactttgaaaagatctctctgaaaccgggagaaacaaagactgttacgttgaagctaaaaggaagcgatttggcatttgtcgggtatgacggtaagtggagactggaaaaaggagatttcaagatcaaatgcggtgaccaatggattgatattgtatgcgatcagacgaaagtatggaatactccgaataaaaatactcttcattaa

SEQ ID NO: 49 - DNA, 2058 bp, Klebsiella sp.
  source: /note="GH42.0-2"
atgaataaatttgcacctttacatccgaaggttagtacgctgctgcatggcgcggattataatccggagcaatgggagaatgaccccgatattattgataaagacattgccatgatgcagcaggcaaaatgcaatgtgatgtcggtgggaatatttagctgggcgaaactggagccacgcgaaggggtatttaatttcgcctggctggatactatcctcgataaactgtatgccgccggcattcatgtttttctggccacgccgagcggcgcgcgtccggcgtggatgtctcagcgctatccgcaggttctgcgggtgggacgcgatcgggtgccggccctgcacggcggccgtcacaaccactgtatgtcgtcaccggtctatcgcgagaaaaccctgaaaatcaataccctgcttgcagagcgttattcttcacacccggcggtactgggctggcatatttccaatgaatatggcggtgaatgccattgcgatctctgccagaaccgttttcgcgactggctgaaggcgcgttaccagaccctggagaacctcaaccaggcctggtggagcaccttctggagtcatacctataccgactggtcgcaaattgaatcacctgcgccacagggcgaggtgtcaattcacggtctcaatcttgactggcatcgctttaacaccgctcaggtgaccgatttctgccgccatgaaattgccccgctgaaggcggctaacgcctccctgccggtgaccactaactttatggagtatttctacgattacgactactggcaactggcaaaggcactggactttatctcgtgggacagctatccgatgtggcaccgcgataaagacgaaaccgcactggcctgctacaccgcgatgtatcacgacatgatgcgcagcctgaagggcggcaaaccgtttgtgctgatggagtccacaccaggcgccaccaactggcagccgaccagcaaactgaagaagccgggaatgcatattctctcctcgctgcaggcggtggcgcatggcgccgactcggtgcagtatttccagtggcggaaaagccgcggttcggttgagaaatttcacggcgcggtggttgaccacgtcgggcacattgatacccgtattggtcgtgaagtcagccagctcggcgagatactgagcaagctaccggaggtccggggttgtcgcaccgaggcgaaagtagcgattatcttcgaccaacaaaaccgctgggcgcttgatgacgcccaggggccgcgcaatctgggtatggagtatgagaagacggtcaacgaacactaccgtccgttctgggaacagggtattgccgtcgatgtgattgacgctgatgtcgatttaacgccataccggttagtgattgccccgatgttatatatggtgcgcgacagctttgccgcgcgggcagaggcgtttgtcgccagcggcggccacctggtgaccacctactggaccggcatcgtcaatgagtccgatctctgctatctcggcggcttcccgggcccgctgcgcaatctgctggggatctgggcggaagagatcgactgtctgaatgacggcgagtttaatcttgtgcaggggcttgccgggaatcagtgcggtctgcaggggccctatcaggtgcgccatctctgtgaactaatccataccgagagcgctcagacgctggccacctaccgggatgatttctatgccggacggccggcggtgacggtgaacggtttcgggaaaggtaaagcctggcatgtcgcctcccgcaacgatttagccttccagcgcgatttctttgctgccctgagcagggagctggatctgccacgagcgatagcggcggatttaccgcccggcgtagtggctaccgcgcgcaccgacggtgagagcacgtttgtcttcctgcagaactacagcgcgcaaagtcatactctgactctgccgccggggtatcgggattgcctgaccgacgcggcggcgccggacccgctgatcctctcagcatgggattgccgtattcttcgtcgtcacgcctaa

SEQ ID NO: 50 - DNA, 2865 bp, Bacteroides sp.
  source: /note="GH31.0-3"
atgattatgaatatgaaaaacattttctattgcctgttgccgggacttcttttcggagcatgttccaataaggtctacgaggagacaggtgatagcgtgatagttaaagtacaacagaaagaaataggagggcctcgtttagttcgccttcaagtgatgggagataagttaatccgtgtttccgccactgccgacagcaagtttgccgatccgcaaagtttgattgttgttccgcaggaaaaacaaacatcctttgccgttgtgcagaatggcgatacgattatagtgtctactgaagaagtaaaagcatccgtactggctagtaccggggaagtgtggtttacggatcgaaacggagagttaatcctgcaggaaaacaagggaggaggaaagaagtttactccgatagaagtggaggggacgaaaggatatacgatctgtcaggtatttgagtctcccgaagatgaggcgttttacggattaggtcagcatcaggcggatgaatttaattataagggcaagaatgaagaattgttccaatacaatacgaaagtatctgttccgtttgttgtttcgaataaaaattatggcatactactggatagttattcgttgtgccgcttcggtaatccgaatgattattcccagttgaaccgtatctttaaactttatgataagacaggtcaggaaggggcgcttaccggtacttatgtaccgaaaaaaggagaaactctggttcgtcgggaagattccatttatttcgagaatctgaaaacgattgagaatcttccgaagaaactgccgttaatgggggctaacgtcacttatgaaggagagatagagcctgctcaaacgggagaatttaagtttattctttattatgcaggatatgtcaaggtttatttgaataatgagctggtagtgccggaacgttggcgtactgcatggaatcctaatagttataagtttgctgctcatttggaagcaggaaagcgtgtgccgttgaaaatcgagtggcagcctgatggtgggcagtcttattgcgggctgcgtgcattgacacccgttgatccgaaagaacaggggaaacagtcgtggtggagtgaaatgaccaagcagctcgattattattttatggctggtgaagatatggacgatgtgattagcggttatcgtacgctgaccggaaagtctcccgttatgccgaagtgggcaatgggtttctggcaaagtcgtgagaagtataatacacaggatgaaatgttgggagcactgaagggttttcgtgatcgtaaaattccgttggataatatcgtactggattggaatcactggccggagaatgcctggggcagtcacgagtttgataagcctcgttttccggatccgaaagcaatggtcgattcaatccatgctatgcatggtcgtatgatgatctcggtatggcctaagttctatgttactactgaacatttcaaagaattcgacgagaatggctggatgtatcagcagtctgtcagggatagcttgaaagattgggtaggtcccggttaccattatggtttttatgatgcatacgatcccgatgcacggaaattgttctggaaacagatgtatgagcattattatccgttgggtatagatgcctggtggatggatgccagcgaaccgaatgtgcgtgactgtacagacctggaatatcggaaggctttgtgcgggcctacggcattaggttcctcaacagaattcttcaatgcttatgcactgatgaatgcggaagcgatttatgacggccagcgcggggtggataataacaaacgggtgttcttattaacccgttcgggatttgccggattgcagcgttattctacggctacatggagtggggatatcggtacacgttgggaagatatgaaagcgcagatttctgcagggttgaattttgcgatgagtggaattccttactggacaatggatattggcggtttttgtgtagagaatcgttatgtggcaggacagaaacaatggaacgcgacaaagacggaaaacgccgattataaagaatggcgtgagttgaatgcccgctggtatcaattcggtgcgtttgtgcctttgtatcgtgcacacgggcaataccctttccgtgaaatatgggagattgcgtcggaagggcatccggcttatcagtcggttgtgtattataccaagttacgttataatatgatgccgtatatttattcgttggcaggtatgacctggttggatgattatacgatcatgcgtcccttagttatggatttcacagtggatgccgaagtgaataatattggtgaccagtttatgttcggtccttcgtttatggtatctcccgtttatcgatatggtgaccgcagccgtgaaatttatttccctcaatcagaaggctggtatgatttttattcaggcaaatttcaggctggaggagagagaaaggttatagaagctccttatgagcgtattccgttgtatgtgcgtgccggtgctatcgtaccattcggagatgatattcagtatacggatgaaaaaccggcggatcatatccgtttgtatatttatcagggagcggatggagagtttacgttatacgaagatgagggtgtgaattataactatgaacaagggaggtatgccatgataccaatgaagtatgatgaagctaccaagactttagtgatcggtgaacgccagggagattttccgggtatgctgaaagaacggactttcactgtaattacggtcaataaggaaaaagcccaaccgtttgatttgaatgcgaaaggggtgactgtgaagtataatggcagcaaacagacattgaaactgtaa

SEQ ID NO: 51 - DNA, 852 bp, Bifidobacterium sp.
  source: /note="GH26.0-1"
gtgcacaatctgctttatgcctactcccccggcggcgtattcaacggtgattccactgattatctcgccacctacccgggcgaccagtgggtggacgtactcggttatgacgaatacgactccgatgattccgcagacgattccagcgcatggatcaacactgtggtcaaggatatgaagatggtttccgaccaagcttcgcagcgtggcaaaatcgtggcgctcaccgaattcggacgttccggcgaacgcaagttcaaggaatccggcaccggagacaaggacaccaagttcttctccgaacttgccgaagcacttgccgaaaacgtgccaagcaccgcatatatgatgacttgggccaacttcggtggaggtggagacaatttccaggcgtatacgccgtggaagggctccgacggcgaagccgatttcaaggcgttcgcggacagcaacaagaacctcatggcctccaaggacaacgtcgactattcgaacgccccggcagccgccatgcaaaatggctccgcgcgtatcgtcactccagtggacggcaatcgtgtgaccgacaccaaggtggtcgtccgggtcaagaccgaaggtgtgaaatactccgaccttgatcttaattccgccatcgtgaccaccgatcgaggccagaacgtcaaactcaagtattcctgcaatggatatttcacgggcatactggatttgaacgcggccggtatcaatcttgaccagtccaaactcactttgactccgcaggtcaagaccaaggacggcaagacactcgcagcggccgacggcaacggttccgtcacagtaaaactggtgccaaaccagagcagacggtag

SEQ ID NO: 52 - DNA, 981 bp, Paenibacillus sp.
  source: /note="GH5.8"
atgttgatatggatgcagggatggaagtctattctagtcgcgatcctggcgtttgtgtcattaggcggtgaacttcctagttcagaagcagccacaggattttatgtaaacggtaccaagctgtatgattcaacgggcaaagcctttgtgatgaggggtgtaaatcatccccacacctggtacaagaatgatctgaacgccgctattccggctatcgcgcaaacgggagccaataccgtacgagtcgtcttgtcgaacgggtcgcaatggatcaaggatgacctgaacgccgtcaacagtatcatctcgctggtgtcgcagcatcaaatgatagccgttctggaggttcatgacgcgacaggcaaagatgatgatgcttcccttgaagcggctgtcgactattggatcggcatcaaagaggccttgatcggaaaagaagaccgcgtcatcgtcaatattgccaatgaatggtatggaaattggaacagcagcggatgggccgagggttataagcaggccattcccaaattaagaaatgcgggcattaagaatacgttgatcgttgatgcagcgggatggggtcaatacccgcaatccatcgtggatgagggggcagcggtatttgcttccgatcaactgaagaatacggtattctccatccatatgtatgagtatgccggtaaggatgccgctacggtgaaaacgaatatggacgatgttttaaacaaaggattgcctttaatcattggggagttcggcggctatcatcaaggtgccgatgtcgatgagattgctattatgaagtacgggcagcagaaggaagtgggttggctggcttggtcctggtacggaaacagcccggagctgaacgatctggatctggctgcagggccaagcggaaacctgaccggctgggggaacacagtggttcatggaaccgacggaattcaacaaacctccaagaaagcgggcatttattaa

SEQ ID NO: 53 - DNA, 2859 bp, Bacteroides sp.
  source: /note="GH31.0-2"
atgaatatgaaaaacattttctattgcctgttgccgggacttcttttcggagcatgttccaataaggtctacgaggagacaggtgatagcgtgatagttaaagtacaacagaaagaaataggagggcctcgtttagttcgccttcaagtgatgggagataagttaatccgtgtttccgccactgccgacagcaagtttgccgatccgcaaagtttgattgttgttccgcaggaaaaacaaacatcctttgccgttgtgcagaatggcgatacgattatagtgtctactgaagaagtaaaagcatccgtactggctagtaccggggaagtgtggtttacggatcgaaacggagagttaatcctgcaggaaaacaagggaggaggaaagaagtttactccgatagaagtggaggggacgaaaggatatacgatctgtcaggtatttgagtctcccgaagatgaggcgttttacggattaggtcagcatcaggcggatgaatttaattataagggcaagaatgaagaattgttccaatacaatacgaaagtatctgttccgtttgttgtttcgaataaaaattatggcatactactggatagttattcgttgtgccgcttcggtaatccgaatgattattcccagttgaaccgtatctttaaactttatgataagacaggtcaggaaggggcgcttaccggtacttatgtaccgaaaaaaggagaaactctggttcgtcgggaagattccatttatttcgagaatctgaaaacgattgagaatcttccgaagaaactgccgttaatgggggctaacgtcacttatgaaggagagatagagcctgctcaaacgggagaatttaagtttattctttattatgcaggatatgtcaaggtttatttgaataatgagctggtagtgccggaacgttggcgtactgcatggaatcctaatagttataagtttgctgctcatttggaagcaggaaagcgtgtgccgttgaaaatcgagtggcagcctgatggtgggcagtcttattgcgggctgcgtgcattgacacccgttgatccgaaagaacaggggaaacagtcgtggtggagtgaaatgaccaagcagctcgattattattttatggctggtgaagatatggacgatgtgattagcggttatcgtacgctgaccggaaagtctcccgttatgccgaagtgggcaatgggtttctggcaaagtcgtgagaagtataatacacaggatgaaatgttgggagcactgaagggttttcgtgatcgtaaaattccgttggataatatcgtactggattggaatcactggccggagaatgcctggggcagtcacgagtttgataagcctcgttttccggatccgaaagcaatggtcgattcaatccatgctatgcatggtcgtatgatgatctcggtatggcctaagttctatgttactactgaacatttcaaagaattcgacgagaatggctggatgtatcagcagtctgtcagggatagcttgaaagattgggtaggtcccggttaccattatggtttttatgatgcatacgatcccgatgcacggaaattgttctggaaacagatgtatgagcattattatccgttgggtatagatgcctggtggatggatgccagcgaaccgaatgtgcgtgactgtacagacctggaatatcggaaggctttgtgcgggcctacggcattaggttcctcaacagaattcttcaatgcttatgcactgatgaatgcggaagcgatttatgacggccagcgcggggtggataataacaaacgggtgttcttattaacccgttcgggatttgccggattgcagcgttattctacggctacatggagtggggatatcggtacacgttgggaagatatgaaagcgcagatttctgcagggttgaattttgcgatgagtggaattccttactggacaatggatattggcggtttttgtgtagagaaccgttatgtagcgggacagaagcaatggaatgcgacaaagacagaaaatgccgattataaagaatggcgtgaattaaatgcccgttggtatcaattcggtgcattcgttcctctgtatcgtgcacatggacaatacccgttccgtgaaatatgggagattgctccggaagggcatccggcctatcaatcggttgtttattataccaagctacgctacaatatgatgccgtatatttattcgttggcaggcatgacctggtttaatgattatacaatcatgcgtccattagtcatggattttacagcggatacccaagtgaataatattggtgaccagtatatgttcggtccttcatttatggtatctccggtttatcgctatggtgaccgtagtcgtgagatttatttcccccaggcagaaggctggtatgatttttattccggtaaattccagcccggaggagagaggaaagtaatagaggctccttatgagcgtatcccgctgtatgtgcgtgcaggcgctatcgtaccgttcggagatgatattcagtatacggatgaaaaaccggcggatcatatccgtttatatatttatcagggagctgatggaaagtttacgctatatgaagatgagggggtgaattataactatgaacagggtatgtacgccatgataccgatgaagtatgatgaggctactaagactttagtgatcggtgaacgccagggagaatttccgggtatgttgaaggaacgtactttcactgtagttacggttaataaggagaaagcacaaccgtttgatttgaatgcgaaaggagtgactgtgaagtataatggcagcgagcagacattgaaactgtaa

SEQ ID NO: 54 - DNA, 1788 bp, Bacteroides sp.
  source: /note="GH43.12-3"
ttgcagaaaaagatcagtaattcatatttgattataaagaaaataagaggtattatgaagaatacacaggtaatacaattaatgtcaatcgtccggttctccatatttatgttggggataacaatgatgtcatgtaactcaaagaaagaacaacaattatcggctattggaaaatctgtggctctctttgattatttttcttataagggaaatgatgatttctatatttccaatcctctgtcaggtgaagactatttctataatcctattttgccgggatggtattctgatcctagtgtttgtacaaatggaaaaggtgattattttctagtaacatctacattcacttatttccccggtgttcctatttttcacagcaaggacttggtgaattggaaacagatagggcatgtgttgaatcgtgcttcgcaattagtgaatatggaagggcagaaagtgagtggcggtatttttgctccggctatttcctataatccgcataataagacctattatatggtgactaccaatgtaggggccggaaatttctttgttaagacacaaaatccgtttggtgaatggtcagagcctgtcatgttgccggaagttggtggtattgatccttctttcttttttgatgaagatggtaaggcgtatatcgtgaataacgatgaggctccggataataagcctgaatatagcggacaccgtaccatacgcatacaagagtttgatgtgaaaacagataagacgatcggtccccgtaaaattcttgtaaacaaaggagctcaaccggcagacaaaccaatttggatagaaggacctcatttatataaaataaatggaaagtacttcttgatgtccgccgaaggtggaacgggaaactggcattcggaagtgattttccgtggtgattctccgatgggtaagtttcttccatggaaaaacaatccgattttgacgcaaagacatttgaattctgaccgtcctaattcggtaacctgtgctggtcatgcagacttgattcaaacaaaggagggagattggtgggctgtttttctggcttgtcgccctattaataatcagtttgagaatttgggacgtgaaacatttatgatgccggtgaaatggagtgaagacggattcccgtacatgacacaaggagatgatttagtacctatgattgtaaaacgtgaaggtgcgaaacgcgatacgacagttacttatggtaatttcgagttaatagagaactttgattctcctgtacttgatatgccatggatgactttaagagcttctgcttccgatttatattcattgacggaaacgcccggatatctgaccttgaagtgtgcagatattagcgctacggaaaagaaaactccggcatttgtttgccgtcggttacaacatcataaatttgaatgtgctacccgtatgttgttcaatccttctaacgataaggaaacagccggaatgctgttgtttaaagatgagacgcgtcaatatttcttctgcttgaataaagtgggtgagaataaaaatatttctctgaaacaaatcggtgaaaaggaacagacattggcttcagatgaaatagacgcagatacaaatgaagtatatttgaaattagtatctcaaggaattggttacgatttctattattctattgatggtgaaaaaagctggaaactgctttgtaaagatgtagcccctagttatctctctactacaacggctggtggatttaccggtactacaattggattatacgctacttgcaaataa

SEQ ID NO: 55 - DNA, 1410 bp, Bifidobacterium sp.
  source: /note="GH26.0-2"
gtggaggacttcgactcctatgacaacgaagccgaattacagtccgtctattcgccgagccacagcacgaaatcgaatctcacgctggtggacatccccgaggacaatggcaccaaggccggtaacatccactatgatttcgtgagctatccggagtataacggcttccagcgttcccatacgccgaagcaggactggtccggcttctccaagctgaacatgttcctcaaggccgacggttcggatcacaagtttgtggtgcaggtcaatgccggcggcgtgaccttcgaagcctatccgaagatcgatggcacggacggacacgtcgtctcactgaacttcggtgacgccgacggcaacggaggcgacttcgcaccggcatcctgggacaccgcgcatgcgggcatgaaactctcgcagaagctgctgtccaaagtcggttcgttcgccctgtacatcaacgacaatggcggcaaccgtccgaagagcggcgatttgacgctcgactccatcaagctcgacggcaaacgcgacgcttacgcgccgaacaccaatccgacgccgggcaacacagccaaagcgcaatccgtggatgatttctcaggctattcggatgatgccgcagcacaatcggcttggggcaaccgcggacatacggaagtcctatccctcgatgaaggcccgaccgatgggtccaaggcgcttcgcttcaagtacgacttctccaatggaggctggtacgatgtggcgaaatatcttgacggcgcgaactggtccggcgaatccgtattggctttccaagtcaagggggatggttccgacaacgccatcggcctgcagatcggcacaagcgatggcaaatacttcctcgccagcgtcaaacttgacttcaccggctggaagcagattgagattccattggtcgataacgccaatctgacccaatcctggccggaggacgccaataaagacaatccgatgaccgaagatgatctggcctccatcaaggaactggtgttcgcctcccagcaatggaatagcgaaagcgatgggcttgatttctccatcgccgatatcaaggtcgagcccgccgagaatacgtccaacgagcaaaccccgaaggacgaaagcaaaaccgaggtcaaggccgacaaggagcaggaacagtccgaggacacctccgcggatgtgaccgcccaagatccggccacttgcccgatttcagacgaagattccaagggctcgaccggcaatacgacggttacggtcaagcccacgcccgacgccaaggaaccggccgacaacaccggcaaagatggcctgtcccgcaccggttcaaacataatctctgccattgctgccgtggccgtgctgatcgcacgcaagcggaagggaggcgatatcgaatag

SEQ ID NO: 56 - DNA, 2361 bp, Bacteroides sp.
  source: /note="GH3.0-2"
atgaaaaacattaagaaaatggtattagtatcagcctttgccggtacttgtcttacgcctcatgcacagactgcctctcctgtcatcccgaccgatccggctattgaaactcatatccgggaatggcttcagaaaatgactctcgaacaaaagatcggtcagatgtgtgaaatcacgattgatgtggtatctgatcttgaaaccagtcgtaagaaaggattctgccttagcgaggcaatgctcgacacggttatcggtaaatataaagtaggttcactgttgaatgttcctttaggggtagcacagaaaaaggaaaagtgggcggaagccatcaaacagatacaggagaaatcgatgaaggagatcggtattccctgcatctatggggtagatcagattcatggaacgacctacacacaggacggaacgatgtttccgcaaggcatcaacatgggagccactttcaaccgggaactgacccgaaaaggtgctgaaatctctgcttatgaaaccaaggctggctgcatcccctggacgtttgctccggtagtcgacttaggacgtgatccgcgctgggcacgtatgtgggaaaattatggtgaagattgttatgtaaatgcagaaatgggcgtatcggccgtgaagggttttcagggagagaacccgaaccgtatcggagaataccatgtagccgcatgtatgaagcactacatgggctatggtgtacctgtctccggtaaagaccgtactccgtcttccatctcacgcagcgatatgcgtgaaaaacatttcgctcctttccttgctgccgttcgtcagggtgcattgagcgtgatggtgaattccggtgttgacaacggactaccttttcacgctaaccgtgaattactgaccgaatggctgaaagaagacctgaactgggacggtctgattgtaacagactgggcggacattaacaatctctgtacccgggatcacattgctgccaccaagaaagaagctatcaagattgccatcaatgccggaatcgacatgtcgatggttccttatgaagtgagtttctgcgattatctgaaagagttggttgaagaaggagaggtatctatggagcgcattgacgatgcagtagcccgtgtgttgcgtctgaaatatcgcctgggattatttgacaatccgtattgggacattaagaagtatgacaagttcggttctaaagaatttgcagccgttgccctccaggctaccgaggaatcggaagtgttattgaagaatgacgcccataccctgccgatagcgaaaggcaaaaagattctgctgaccggtccgaacgcaaactccatgcgttgtctgaacggcggatggtcgtatagctggcagggacacgttgccgatgaatatgcgcaggcatatcataccatctacgaggctttgtgtgagaaatacggaaaagagaatattatctacgaaccgggagtgacctatgctccttacaagaacgataattggtgggaagaaaacaaaccggaaattgaaaaaccggtggcagcggcagcacaagcggatattatcatcgcctgcatcggcgaaaactcttattgcgaaactccgggcaacctgacggatcttaccttatcggaaaaccagcgcaatctggtaaaagctctggccgctacgggcaaacctatcgttttggttctgaatcagggacgcccgcgtattatcaacgatatagaacctttggcaaaagctgttgtcaacatcatgctgccaagcaactatggtggagacgcacttgcaaacttattggcaggcgacgccaacttcagtggaaagatgccattcacttatccacgacttatcaacgctttggcaacttatgacttcaagccttgcgaaaacatagggcaaatgggaggcaactacaactatgactcggtgatggatattcaatggccgttcggtttcggattaagctatacgaattacgaatacagcaacttaaaagtaaataaaccgacttttaatgctgacgacgaactgatattcacggttgacgtaaccaacacgggcaaagttgtcggaaaagagagtgtgttattgttctctaaggacttagtggcaagcagcacaccggacaatatccgtttacgaaacttcgaaaaggtttctctgaaaccgggagaaacaaagacggttacgctgaaactgaaaggaagcgacttggcatttgtgggatatgacggtaagtggagactggaaaaaggagatttcaagattaaatgtggtgaccaatggatggatattgtatgcgatcagacaaaagtatggaatactccgaataagaatacggcccacaaataa

SEQ ID NO: 57 - DNA, 2232 bp, Unknown
  source: /note="Description of Unknown: Lachnospiraceae sequence"
  source: /note="GH36.0-2"
atgagcatttgttatcacgaaggatcccgggaatttcatctttccaacagggatatcagttatattatcacagtcttaaaaaacggacagttaggacagctgtattttgggaaaaaactgcatgacagggagagttttgcccatctgctggagctgcgtcaccgcccaatggctgtatgtacttacgaaggagattccacattctcgatggaacatatcaagcaggaatatccgtcctatggagcaggggatatgcggtatccggcggtggagattctgcaggaaaacggaagccggatcacggattttgtgtatcagacacatcggatttatgacgggaagcccgcgcttgcaggactgccggctacctataccgaagattccaaagaggcacagacactggaaatcgaactgaaagatgagctgattcacaccacactgatcttgtactatacgatttttgaagagcttccggcgattacaagaagtgcaaaggtgatttaccacggaacagagaagatcgtgctggaacgtgcaatgagctgcagtgtggatctgccggatcacgactatcaaatgatcgagctgacgggagcctggggaagagagcgtgcggtgactgagcgaaagctgcagtatggaattcagggaatttatagtatgcgcggatgcagcagcagtaactttaatccgtttctggcactgcgtcgggagaataccacggaagcgtgcggggaagtgtatggcttcagtcttgtttacagcgggaattttctggcgcaggcagaggtggatacatacgatgtcacaagagtgacgctgggaattcatccggaccggttttcctgggaaatgaaaaacggagatgagtttcagacaccggaggcggtgatggtctattccaatcgcggactgaacgggatgagtcaggcattccacagtctgtatcgtgcacgcctggcaagaggatactggagagaccgaccgagaccgattctcatcaataactgggaagcgacttattttgatttcaatgaggaaaagattctggagatcgtgcgcacggcaaaacagcttggaatcgaattgtttgtactggatgacggatggttcggaaaacgggaggatgatcattcttctctgggagactggtatccgaatctggaaaagctgccggatggcattgcaggaatcgcgaagaaggtagcggcggaaggcatgaaattcggtctctggtttgagccggaaatggtcaacaaggacagcaatctctatagagagcatccggactggattttgtctactccgggacgtcatatttcccatggaagaaatcagtatattctggatttttccagagccgaagtggtggatgccatttatggacaaatggaaaaaatcctggaggatgcgccgatttcttatatcaaatgggatatgaaccgctgtatgtcagaagtatactctcatacagccagtgccgcagatcagggtaaggtcatgcatcagtatattctaggtgtttatcggttatatgagaagctgacgggcagatttcctgaaattttatttgaatcctgtgcaagcggcggttcccgttttgatccgggattgctgtattatgcgccgcaggcatggacatcggatgatacggatgcagtggaacgttgtaagatccagtatggaacgtcccttgtctatccagtgagcagtatgggatctcacgtatcagcagtgccgaatcatcaggtgcttcgcaacacatctttgaaaatgcgtgcggatgtagcgtatttcggaacattcggatatgagctgaacccgaacagtctgacagaggcagagcgggaggcaatcaaaaagcagacggcatttatgaaagaacacagaagcctgatccagtatggaacattctatcgacttcagagcccgtttgcaggaaatgaaatggcatggatggttgtgtctgaggacaaaaaagaagcgattgtgggctggtatcgcttcctggagccgatcaatatcggatatcggagcgtcagactgcagggactggatccgaagcttccgtatcagatttcggatatggaaatggcattgtacggagatgagctgatgcaggccggactgatcgtatcagacgtggcgtccggacaaaatccggagcagtataatggagagaacggagatttccagtctcgtctttatctgctgaaagcaaaggaagaataa

SEQ ID NO: 58 - DNA, 1578 bp, Bacteroides sp.
  source: /note="GH76.0-6"
atgaaagcaatattcaaactgtttatattgaacctcttggctttggcattacttccgtcctgtagtgatgatgatcagtcaaactcagaacagaatgatcccatcagtggaaatatttctccggtaggttcatttgcggtagaagctaccaataacgagaatgaacttctggtgaaatggaccaatcccagtaatcgcgacgtggatatggtagaactctcttacagggacgtggaagcgagcttgtctcgtgctaccgacttctcgccgggacatatcatcatacaggtagagcgtgatgttacacaagaatatctcttgaaagttccttattttgctacttacgaagtttctgccgtagctatcagcaaagccggcaagcgatcggtgcccgaaagccgtattatgatgccttatcatgaaaaggtggatgagccggaactgaaactgccggagatgctggaccgtgcacattcttacatgacttctgtcattggatattatttcggcaagagttccaggagctgctggcgtggtaattatccatatgatggaaaaggttattgggatggtgatgcgttggtctggggacaaggcggcggtctttcggcatttgtcgctatgcgtgatgcaaccaaagagagcgaagtggagaatatctatggcgcaatggatgatatgatgttcaaaggaatacagtatttctgtcagctggatcgtggaatcctggcttattcctgctacccggctgccggtaacgaacgcttttacgatgataacgtatggatcgggctcgatatggtcgactggtatacggaaacgaaagagatgcgttatctgacacaggcaaaggtggtatggcgctatctgatcgatcacggttgggatgagacttgcggaggaggtgtacactggagggagttgaacgaacacactaccagcaagcactcttgctctaccggacctactgctgtgatgggctgtaagatgtatctggcaactcaggaacaggaatatctcgactgggcgatcaaatgttacgactatatgctggatgtattgcaagacaagtccgaccatttattctatgacaatgtacgtccgaataaggatgatcccaatctgccgggcgatcttgaaaagaacaagtattcttacaattccggacagccgttgcaggcagcctgtctcttatataagattaccggcgaacagaaatatctggatgaagcgtatgcgattgctgaaagctgtcataagaaatggtttatgccctatcgttccaaagagctgaatcttactttcaacatccttgctccgggacacgcctggttcaatacgatcatgtgtcgcggattctttgaactttattctatagacaatgaccgtaaatatatcgatgacattgagaagtcaatgattcatgcgtggagcagtagctgtcatcagggcaacaacttgctgaatgacgatgatctgagagggggaacgaccaagaccggttgggaaatactccatcagggagcattggttgaattgtatgcccggttggcagtactggaacgtgaaaaccgatag

SEQ ID NO: 59 - DNA, 1551 bp, Bacteroides sp.
  source: /note="GH76.0-7"
ttgaacttcttggctttggcattacttccatcttgtagtgatgatgatcagtcaaactcagaacagaatgatcccatcagtggcaatatttctccggtaggttcattttccgtagaagctaccaataacgagaatgaacttctggtgaaatggaccaatcccagtaatcgcgatgtggatatggtagaactctcttacagggacgtggaagcgagcttgtctcgtgctaccgacttctcgccgggacatatcatcatacaggtagaacgtgatgttacacaggaatatctgttgaaagttccttattttgctacttacgaagtttctgccgtagctatcagtaaagccggcaagcgatcggtacccgaaagccgtattatgatgccttatcatgaaaaggtggatgagccggaactgaaactgccggaaatgctggaccgtgcacattcttacatgacctctgtcattggatattatttcggcaagagttccagaagctgctggcgtggtaattatccttatgatggaaaaggttattgggatggtgatgcgttagtttggggacaaggtggcggtctttcggcatttgtcgctatgcgtgatgcaaccaaagagagcgaagtggagaatatctatggcgcaatggatgatatgatgttcaaaggaatacagtatttctgtcagctggatcgtggaatcctggcttattcttgctacccggctgccggtaacgaacgtttttacgatgataacgtatggatcgggctcgatatggtcgactggtatacggaaacgaaagagatgcgttatctgacacaggcaaaggtggtatggcgctacctgatcgatcacggttgggatgagacttgcggaggaggtgtacactggagggagttgaacgaacacactaccagcaagcactcttgctctaccggacctactgctgtgatgggctgtaagatgtatctggcaactcaggaacaggaatatctcgactgggcgatcaaatgttacgactatatgctggatgtattgcaagacaagtccgaccatttattctatgacaatgtacgcccgaataaggatgatcccaatctgccgggtgatcttgaaaagaacaagtattcttacaattccggacagccgttgcaggcagcctgtcttttatataagattaccggcgaacagaaatatctggatgaagcgtatgcgattgctgaaagctgtcataagaaatggtttatgccctatcgttccaaagaactgaaccttactttcaatattcttgctccgggacatgcttggttcaatacgatcatgtgccgcggattctttgaactttattctatagacaatgaccgtaaatatatcgatgatatcgaaaagtcaatgattcatgcgtggagcagtagctgtcatcagggtaacaacttgctgaatgacgatgatctgagagggggaacgaccaagaccggttgggaaatactccatcagggggcattggttgaattgtatgcccggttggcagtattggaacgtgaaaaccgatag

SEQ ID NO: 60 - DNA, 1788 bp, Bacteroides sp.
  source: /note="GH43.12-2"
ttgcagaaaaagatcagtaattcatatttgattataaagaaaataagaggtattatgaagaatacacaggtaatacaattaatgtcaatcgtccggctctccatatttatgttggggataacaatgatgtcatgtaactcaaagaaagaacaacaattaccggctattggaaaatctgtggctctctttgactatttttcttataaaggaaatgatgatttttatatttccaatcctctgtcagatgaagactatttctataatcctattttgccgggatggtattctgatcctagtgtttgtacaaatggagaaggtgattatttcctagtaacatctacattcacttatttccccggtgttcctatttttcacagcaaagacttggtgaattggaaacagatagggcatgtgttgaaccgtgcttcgcaattagtgaatatggaaggacagaaagtgagtggcggtatttttgctccggctatttcttataatccgtataacaagacatattatatggtaacaaccaatgtcggagccggaaatttctttgttaagacgcaagacccgtttggtgaatggtcggaacccgtcatgttgccggaggtcggaggtattgatccttctttcttttttgatgaagatggtaaggcatatattgttaataatgatgaggctccggataataaacctgaatatagcggccaccgtactatacgcatacaagagtttgatgtgaaaacagataagacgatcggtcctcgtaagattcttgtaaacaaaggagctcaaccggcagacaaaccaatttggatagaaggtcctcatttatataaaataaatggaaagtatttcttgatgtccgccgaaggtggaacgggtaactggcattcggaagtgattttccgtggtgattctccgatgggtaaatttcttccatggaaaaacaatccgattctgacgcaaagacatttgaattctggccgtcctaattcggtaacctgtgctggtcatgcagacttgattcaaacaaaagagggagattggtgggctgtttttctggcttgtcgccctattaataatcagtttgagaatttgggacgtgaaacatttatgatgccggtgaaatggagtgaagatggattcccgtacatgacacaaggcgatgatttagtacctatgattgtaaaacgtgaaggtgcgaaacgcgatacgacagttacttatggtaacttcgagttaatagcgaactttgattctcctgtacttgatatgacttggatgactttgagagcttctgcttccgatttatattcgttgacggaaacacccggatacctgaccttgaagtgtgtagatattagcgctaccgaaaagaaaactccggcatttgtttgtcgtcggttacaacatcataaatttgaatgtgctacacgtatgttgttcaatccttctaacgataaggaaacagccggaatgctgttgtttaaagatgagacacatcaatatttcttctgcttgaataaagtgggtgagaataaaaatatttctctgaaacaaatcggtgaaaaggaacagacattggcttcagatgaaatagacgcagatacaaatgaagtatatttgaaattagtatctcaaggaattggttacgatttctattattctattgatggtgaaaaaagctggaaactgctttgtaaagatgtagatcccagttatctctctactacaacggctggtggatttaccggtactacaattggattatacgctacttgcaaataa

SEQ ID NO: 61 - DNA, 1734 bp, Bacteroides sp.
  source: /note="GH43.12-5"
atgaagaatacacaggtaatacaattaatgtcaatcgtccggttctccatatttatgttggggataacaatgatgtcatgtaactcaaagaaagaacaacaattatcggctattggaaaatctgtggctctctttgattatttttcttataagggaaatgatgatttctatatttccaatcctctgtcaggtgaagactatttctataatcctattttgccgggatggtattctgatcctagtgtttgtacaaatggaaaaggtgattattttctagtaacatctacattcacttatttccccggtgttcctatttttcacagcaaggacttggtgaattggaaacagatagggtatgtgttgaatcgtgcttcgcaattagtgaatatggaagggcagaaagtgagtggcggtatttttgctccggctatttcctataatccgcataataagacctattatatggtgactaccaatgtaggggccggaaatttctttgttaagacacaaaatccgtttggtgaatggtcagagcctgtcatgttgccggaagttggtggtattgatccttctttcttttttgatgaagatggtaaggcgtatatcgtgaataacgatgaggctccggataataagcctgaatatagcggacaccgtaccatacgcatacaagagtttgatgtgaaaacagataagacgatcggtccccgtaaaattcttgtaaacaaaggagctcaaccggcagacaaaccaatttggatagaaggacctcatttatataaaataaatggaaagtacttcttgatgtccgccgaaggtggaacgggaaactggcattcggaagtgattttccgtggtgattctccgatgggtaagtttcttccatggaaaaacaatccgattttgacgcaaagacatttgaattctgaccgtcctaattcggtaacctgtgctggtcatgcagacttgattcaaacaaaggagggagattggtgggctgtttttctggcttgtcgccctattaataatcagtttgagaatttgggacgtgaaacatttatgatgccggtgaaatggagtgaagacggattcccgtacatgacacaaggagatgatttagtacctatgattgtaaaacgtgaaggtgcgaaacgcgatacgacagttacttatggtaatttcgagttaatagagaactttgattctcctgtacttgatatgccatggatgactttaagagcttctgcttccgatttatattcattgacggaaacgcccggatatctgaccttgaagtgtgcagatattagcgctacggaaaagaaaactccggcatttgtttgccgtcggttacaacatcataaatttgaatgtgctacccgtatgttgttcaatccttctaacgataaggaaacagccggaatgctgttgtttaaagatgagacgcgtcaatatttcttctgcttgaataaagtgggtgagaataaaaatatttctctgaaacaaatcggtgaaaaggaacagacattggcttcagatgaaatagacgcagatacaaatgaagtatatttgaaattagtatctcaaggaattggttacgatttctattattctattgatggtgaaaaaagctggaaactgctttgtaaagatgtagcccctagttatctctctactacaacggctggtggatttaccggtactacaattggattatacgctacttgcaaataa

SEQ ID NO: 62 - DNA, 1734 bp, Bacteroides sp.
  source: /note="GH43.12-6"
atgaagaatacacaggtaatacaattaatgtcaatcgtccggctctccatatttatgttggggataacaatgatgtcatgtaactcaaagaaagaacaacaattaccggctattggaaaatctgtggctctctttgattatttttcttataagggaaatgatgatttttatatttccaatcctctgtcaggtgaagactatttctataatcctattttgccgggatggtattctgatcctaatgtttgtacaaatggagaaggtgattatttcctagtaacatctacattcacttatttccccggtgttcctatttttcacagcaaagacttggtgaattggaaacagatagggcatgtgttgaaccgtgcttcgcaattagtgaatatggaaggacagaaagtgagtggcggtatttttgctccggctatttcttataatccgtataacaagacatattatatggtaacaaccaatgtcggagccggaaatttctttgttaagacgcaagacccgtttggtgaatggtcggaacccgtcatgttgccggaggtcggaggtattgatccttctttcttttttgatgaagatggtaaggcatatattgttaataatgatgaggctccggataataaacctgaatatagcggccaccgtactatacgcatacaagagtttgatgtgaaaacagataagacgatcggtcctcgtaagattcttgtaaacaaaggagctcaaccggcagacaaaccaatttggatagaaggtcctcatttatataaaataaatggaaagtatttcttgatgtccgccgaaggtggaacgggtaactggcattcggaagtgattttccgtggtgattctccgatgggtaaatttcttccatggaaaaacaatccgattctgacgcaaagacatttgaattctgaccgtcctaattcggtaacctgtgctggtcatgcagacttgattcaaacaaaagagggagattggtgggctgtttttctggcttgtcgccctattaataatcagtttgagaatttgggacgtgaaacatttatgatgccggtgaaatggagtgaagatggattcccgtacatgacacaaggagatgatttagtacctatgattgtaaaacgtgaaggtgcgaaacgcgatacgatagttacttatggtaacttcgagttaatagagaactttgattctcctgtacttgatatgacttggatgactttgagagcttctgcttccgatttatattcattgacggaaacacccggatacctgaccttgaagtgtgcagatattagctctacggaaaagaaaactccggcatttgtctgccgtcggttacaacatcataaatttgaatgtgctacccgtatgttgttcaatccttctaacgataaggaaacagccggaatgttattgtttaaagatgaggcgcatcaatatttcttctgcttgaataaagtgggtgagaataaaaatatttctctgaaacaaatcggtgaaaaggaacagacattggcttcagatgaaatatacgcagatacaaatgaggtatatttgaaattagtatctcaaggaattggttacgacttctattattctattgatggtgaaaaaaactggaaactgctttgtaaagatgtagattccagttatctctctactacaacggctggtggatttaccggtactacaattggattatacgctacttgcaaataa

SEQ ID NO: 63 - DNA, 1027 bp, Escherichia sp.
  source: /note="GH42.0"
tggcgccgactcggtgcagtatttccagtggcggaaaagccgcggttcggttgagaaatttcacggcgcagtggtcgaccacgtcggacatattgatacccgcattggccgcgaagtctgccagctcggcgagatcctcagtaagttgccggaggtgaggggctgtcgcaccgaggcgaaagtagcgattatcttcgaccagcagaaccgctgggcgctggatgacgcccaggggccgcgcaatcttgggatggaatatgagaagacggtcaacgagcactaccgcccgttctgggagcagggcatcgccgtcgatgtgattgacgccgatgtcgatttaacgccgtaccagttagtgattgccccaatgttatatatggtgcgcgacggctttgccgggcgggcggaggcgtttgtcgccaacggcggccacctggtgaccacctactggaccggcatcgtcaatgagtccgatctctgctatctcggcggcttcccgggcccgctgcgcaatctgctggggatctgggcggaagagatcgactgcctgaatgacggcgagtttaatctggtgcagggacttgccgggaatcagtgcggtctgcagggcccttatcaggtgcgccatctctgcgaactaatccatacagagagcgcccaggcgctggccacctaccgggatgatttttatgccggccggccggctgtgacggtgaacgagttcgggaaaggcaaagcctggcatgtggcctcccgcaacgatttagccttccagcgcgatttctttaccaccctgagcaaggagctggccctgccgcgggcgatagcgacggagttaccacccggcgtggtggctactgcgcgcaccgacggtgacaactcttttatcttcctgcagaactacagcgcccaaaaccataccctgaccctgccgcaaggatattgggattgcctgaccgacgcggcggtgtcggctccactgaccctgtcggcatgggattgccgtattctccgtcgtcacgcgtaa

SEQ ID NO: 64 - DNA, 2361 bp, Bacteroides sp.
  source: /note="GH3.0-3"
atgaaaagcattaagaaaatggtattagtatcagcctttgccggtacttgtcttgcgccccatgcacagacaacctctcctgccatcccggctgatccggctattgaagctaacatccgggaatggcttcagaaaatgactctcgaacaaaagatcggtcagatgtgtgaaatcaccattgatgtggtttctgatcttgaaaccagtcgcaaaaaggggttctgccttagcgaggcaatgctcgacactgttatcggcaaatataaagtaggctccctgttgaatgttcctttaggggtagcacaaaaaaaggagaagtgggcggaagctatcaaacagatacaggaaaaatcgatgaaggagatcggtattccctgcatctatggggtagatcagattcatggaacgacttacacattggacggaacgatgtttccgcaaggcatcaacatgggagccaccttcaaccgcgagctaacgagaagaggtgccgaaatctccgcttatgaaacgaaagcaggctgcatcccctggacgttcgccccggtagtcgacttaggccgcgacccgcgctgggcacgtatgtgggagaactatggtgaagattgttatgtaaacgcagaaatgggtgtatcggccgtgaaaggttttcagggagaagacccgaaccgtatcggagaatacaatgtagctgcgtgcatgaagcattatatgggttacggtgtacctgtttccggtaaagaccgtactccatcttccatctcacgcagtgatatgcgtgaaaaacatttcgctcctttccttgccgctgtacgtcagggtgcattgagcgtaatggtaaactccggcgttgacaacggactgccttttcacgccaaccgtgagttgctgaccgaatggctgaaagaagacttgaactgggacggactgattgttacagactgggcggacattaacaatctctgtacccgggatcacatcgctgccaccaagaaagaggctgtcaagattgccatcaatgctggtatcgacatgtcgatggttccttatgaagtgagtttctgcgattatctgaaagagttggttgaagaaggagaggtatctatggagcgtatcgatgatgcagtagcccgtgtgttgcgtctgaaatatcgtctgggattatttgaccatccatattgggacattaagaagtatgacaagttcggttctaaggaatttgcagctgttgccctgcaggctgccgaggaatcggaagtgttgctaaagaatgacggaaatatcctgccgatagcgaaaggcaaaaagattctgctgaccggtccgaacgcaaactcgatgcgttgtctgaacggcggatggtcgtatagctggcagggacacgttgccgatgaatatgcgcaggcatatcataccatctacgaggctttgtgtgagaaatacggaaaagagaatattatctacgaaccgggagtgacctatgctccttacaagaacgataattggtgggaagaaaacaaaccggaaattgaaaaaccggtggcagcggcagcacaagcggatattatcatcgcctgcatcggcgaaaactcttattgcgaaactcccggtaacctgacggatcttaccttatcagaaaaccagcgcaatctggtaaaagctctggccgctacgggcaaacctattgtcctggttctgaatcagggacgtccgcgtattatcaacgatatagaacctttggcaaaagctgttgtcaacatcatgctgccaagcaattacggtggcgacgcacttgctaacttattggccggtgatgccaacttcagtggaaaaatgccgttcacctatccccgacttatcaacgctttggcaacttatgactacaagccttgcgaaaacatggggcaaatgggaggtaactacaattatgattcggtgatggatattcaatggccattcggtttcggattaagctatacgaattataagtacagcaatttaaaagtaaataaaccgacttttaatgctgacgacgaactgatattcacggttgacgtaaccaacacgggcaaagttgccggaaaagagagtgtgttattgttctctaaggacttagtggcaagcagcacaccggacaatatccgtttacgaaacttcgaaaaggtttctctggaaccgggagaaacaaagacggttacgctgaaactgaaaggaagcgacttggcatttgtgggatatgacggtaagtggagactggaaaaaggagatttcaagattaaatgcggtgaccaatggatggatattgtatgcgatcagacaaaagtatggaatactccgaataagaatacggcccacaaataa

SEQ ID NO: 65 - DNA, 1545 bp, Bacteroides sp.
  source: /note="GH51.0-2"
atgaaagcaaaactattagtcagcacggcttttctggcagcatccgtatctctttctgcacaaaagagtgctaccataaccgtacatgccgaccaaggcaaagaaatcataccgaaggaaatttacggccagtttgccgaacacctgggttcatgtatctacggcggtctttgggtaggcgaaaactcggatattcccaatattaagggataccgcacagatgtattcaatgcactgaaagacttgtccgttcccgtccttcgctggccgggcggatgctttgccgatgaataccactggatggacggcattggtccgaaagagaaccgtccgaagatggtgaacaacaactggggcggaaccattgaagataacagtttcggaacacacgagtttttgaatctttgcgaaatgctgggttgcgaaccatacgtgagtggaaatgtaggtagcggtaccgtagaagaactcgccaaatgggtggaatacatgacctccgacggggactctcccatggccaatcttcgtcgtaagaatggtcgtgacaaagcatggaaactcaaatatctgggagtaggaaatgaaagctggggctgtggtggcagcatgcgtccggaatattatgcggacttataccgtcgttattctacttattgccgtaactatgacggcaaccgtctgttcaaaattgccagtggtgcaagtgactatgactacaactggacagacgtattgatgaatcgtgtaggacatcgcatgcagggactttctctccactattacaccgtaaccggatggagcggcagcaaaggggcagccactcaattcaacaaggatgactattattggacaatgggtaaatgcctggaagtggaagatgtgctcaagaagcattgtgccatcatggataaatatgacaagaacaaaaagatcgctcttttactcgacgaatggggaacctggtgggatgaagaaccgggaaccatcaaaggacacctatatcagcagaatacattgcgcgatgctttcgttgcttctttaagccttgacgtattccacaaatatacagaccgtctgaagatggcaaacatcgcacagattgtcaatgtacttcaatccatgattctgacgaaagacaaagaaatggtgctcactcctacttattatgtcttcaagatgtataaagtacatcaggatgccacttatcttcccatcgacctgacttgcgaaaagatgagtgtacgtgataaccgcaccgttccgatggtaagcgccacagcttccaaaaacaaagatggagtgatccacatttctctgtccaatgtagatgctgacgaagcacaggaaatcaccatcaatctgggtgatacgaaagcaaaaaaagcagtcggagagattctgacctctgcaaaactgaccgattacaattcttttgaaaaccctaatattgtaaaaccggcacctttcaaagaggtaaaaatcaataaaggtacaatgaaggtaaaacttcctgctaagtccattgttactttagagttacagtaa

SEQ ID NO: 66 - DNA, 2445 bp, Bacteroides sp.
  source: /note="GH31.0-9"
atgaaaatacatcatctattttggggtatatgtttatgcttcagcacaaatattttattcgcacagaactatcagaaaacatcgtccggcatcaaaaccactgtaaatgcagtggatatagaagtacaattctttgcgcctgctgtggcgagagtaataaaatcgccggaaggtgttgcctatgaaaaacagagtctttctgtaattgccaaacccgaaaaggtaagtttcaaggctgatatacaagataataagattgtattgaacaccagcgaactaagtgtcagtgtggacaccgggacgggaattgtttcttatttctcaaaggatggcaagtcgttattggcagagaaatccggtatgcagtttatcaatttcgatgatgccgggacaaaaacttatcaggtttatcaaccttttatattagataaggaggaagccatttatggtttgggacaattgcaaaatggaaagatgattcagcggaacatgactaaaaatctgatacagggaaatgttgaagatgtgtcacctttcttccagtctactaaaggatatggtgtgttttgggataactattcgccgactctttttacggataacgaagttgaaacatctttccgttctgaagtaggtgactgtgtggattattacttcatgtatgggaaaaatgccgacggtgttatagcacaggtacgcagcttgaccgggcaagcaccgatgtttccattatggacttatggttactggcaaagtaaagaaagatataagagccaggaggaagtggtagatgttgttcgcaagtatcgtgagttgggggttcctttggacggtattattcaggactggcaatattgggggcataactatttgtggaatgcgatggattttcagaatccgactttcaataatcctcaaaagatgattgaggatgtccatgcgatgaacgcacacatggctatatctatctggtcgtcattcggaccgatgactaaaccttatagagaattggacaaaaaagggatgttgtttaacttcactacttggccgcaatcgggattggagtcatggccccccaacatggaatacccttccggtgtaagagtgtatgatgcttacaatcccgaagcgcgtgacatttattggaaatatctgaatgatggaattttcaagctgggaatggatgcctggtggatggactctaccgaacccgatcatttggattggaagccggaggatatggataccaaaacctatctgggctcgttccgtaaggtgcgcaatgcttatccgttgatgactgtcggaggggtttacgaccatcagcgtgcagtgacttcggacaaacgggtgtttattttaactcgttcgggattcttggggcagcaacgttatggtgcaaatgtatggagtggtgatgtcgcttccacatgggagagttttagaaatcagattcctgccggattaaacttttctttgtgtggtatgcctcactggaatagtgatattggtggcttttttgcaggacattataataaaagctggaatgatgatagtgcttcaaaaaatccattgtatcaggagctttatgtgcgttggttgcagtttggaacgttcaatccgatgatgcgttcgcacgggacggatgtttatagggaaatctataagttcggaaagaagggtgagcctgtatatgatgctatcgagaagatgataggtttgcgttactctttgttgccttatatttattctacttcttgggaggtgagcaatcgccaatcgagttttatgcgcgctttgatgatggattttgtagatgacagaaaggtgtgggatatcaatgacgaatatatgtttggaaaatcaatccttgtagctccgattgctcatgcacaatatacaccggaagctgtggtaaaagtctccgaagaagaaggatggaacagagatggagtgaaaaaagcaaaaactgacgttgctgtggatttcatggaaacgaaatctactaaaatatacttaccggcaggaacgctatggtatgacttctggacgaacgagaaacacgaaggcggaaaggaaattaccaaagagactacacttgatgttattccattgtatgtaaaagcgggtagtattattcctgtcggtccacaagttcagtatgcaactgaaaaaccgtgggatcatcttgaactgaaggtgtatgcgggtgcgaatggaaacttcattttatatgaagatgaatttgataattacaactacgaaaaaggcgtttatacggaaattccaatctcgtggaataatacatcttgtaaattgacgataggagcaagaaaaggtgcgtatgagggaatgttgaagaactgtaagtttactgtaactctccaggacgggactcaaaaaaacgtcgattataatggaaaggctatttctgtaaagttttga

SEQ ID NO: 67 - DNA, 1734 bp, Bacteroides sp.
  source: /note="GH43.12-4"
atgaagaatacacaggtaatacaattaatgtcaatcgtccggctctccatatttatgttggggataacaatgatgtcatgtaactcaaagaaagaacaacaattaccggctattggaaaatctgtggctctctttgattatttttcttataaaggaaatgatgatttttatatttccaatcctctgtcagatgaagactatttctataatcctattttgccgggatggtattctgatcctagtgtttgcacaaatggagaaggtgattatttcctggtaacatctacattcacttatttccccggtgttcctatttttcacagcaaagacttggtgaattggaaacagatagggcatgtgttgaaccgtgcttcgcaattagtgaatatggaaggacagaaagtgagtggcggtatttttgctccggctatttcttataatccgtataacaagacatattatatggtaacaaccaatgtcggagccgggaatttctttgttaagacgcaagacccgtttggtgaatggtcggaacccgtcatgttgccggaggtcggaggtattgatccttctttcttttttgatgaagatggtaaggcatatattgttaataatgatgaggctccggataataaacctgaatatagcggccaccgtactatacgcatacaagaatttgatgtgaaaacagataagacgatcggtccccgtaaaattcttgtaaacaaaggagctcaaccggcagacaaaccaatttggatagagggccctcatttatataaaataaatggaaagtatttcttgatgtccgccgaaggtggaacggggaactggcattctgaagtgattttccgtggtgattctccgatgggtaaatttcttccatggaaaaacaatccgattttgacgcaaagacatttgaattctgaccgtcctaattcggtaacctgtgctggtcatgcagacttgattcaaacaaaggagggagattggtgggctgtttttctggcttgtcgccctattaataatcagtttgagaatttgggacgtgaaacatttatgatgccggtgaaatggagtgaagacggattcccgtacatgacacaaggagatgatttagtacctatgattgtaaaacgtgaaggtgcgaaacgcgatacgacagttacttatggtaacttcgagttaatagagaactttgattctcctgtacttgatatgccatggatgactttaagagcttctgcttccgatttatattcattgacggaaacacccggatacctgaccttgaagtgtgcagatattagctctacggaaaagaaaactccggcatttgtctgccgtcggttacaacatcataaatttgaatgtgctacccgtatgttgttcaatccttctaacgataaggaaacagccggaatgttattgtttaaagatgaggcgcatcaatatttcctctgcttgaataaagtgggtgagaataaaaatatttctctgaaacaaatcggtgaaaaggaacagacattggcttcagatgaaatagacgcagatacaaatgaggtatatttgaaattagtatctcaaggaattggttacgacttctattattctattgatggtgaaaaaagctggaaactgctttgtaaagatgtagatcccagttatctctctactacaacggctggtggatttaccggtactacaattggattatacgctacttgcaaataa

SEQ ID NO: 68 - DNA, 3810 bp, Bifidobacterium sp.
  source: /note="GH13.28"
atgaaacatcggaaacccgcaccgacctggcataggctggggctgaagattagcaagaaagtggtggtcggcattaccgccgcggcgaccgccttcggcggactggcaatcgccagcaccgcagcacaggccagcaccgatcgcgacagctacgccgacaccgttgaaaacaccacgttcgaacaggcgcgcaagcattacggactggcgcagcaaatgagcgagggcgccaccctgcatgcatgggagtggagcttcaaaaccattgaggaaaacatccccgctattgccgaagcgggttacacctccgtgcagaccgagccgatttccgctattcataacggcggcaagggcatgatcttcaccgagaactggtactacgtgtatcagccgaccgacaccaccatcggcaactgggtgatgggtaccgaagatgatctgaagagcctgtgcaacacggctcacaagtacggcgtgcgtatcatcgtcgatgtggtagccaaccatatgaccgcgacttggggcgccatcgccgatcgttggaagaagtccgagtactaccaccacgactgcaatgacggtgatgtgcaggattggaacaaccgctatcaggtgacccactgcaagctgctcggcctgtatgacatcaacactgagaacaccgaaaccgccaacatgatgcacgatttcctcgtgcaagcggtcaacgacggtgtggacgggttccgtttcgatgcggccaagcacatcgaactgccggacgagtataacggctcccagtattggaacatcattcttaacaatggcgcgcagttccaatacggcgaagtgttgcaggattccatctcccgcgatagcgactatgcaaagctgttctccagccacagcaagaacggcggcggcgtcaccgcatcctcctacggcagcaagctgcgcggagccctgaattcgaagaacctgaacgccggcaccctgtccgattggagcaactccgccagcccgagcaatcttgtctcttgggtggaatcgcatgataactattccaatagcgatagggaatccaccggcatgagcgagtggcagatgaccatgggctggggcgtcatcggttcccgctcccagaccatgccgctgtacttcgaccgcccggtcggttccggcggcagccagccacagttctccgaggagagcaagctcggcgatgccggtgcggattcttggaaggatgcgcaggttgtggcggtgaaccacttccgcaatactatgaacaacaacaaggcttcggagtatctgcgcaactgcggcgcgaattcctgcctcatggtggaacgctacatcaaggacggcaacttcaagaacgacggcgtgaccatcaccaacatgggtgatacgcaagagctgtccggcactgccaccaaccttgacgacggcacctacaaggaccaggtctccggcggtaccatcaccgtttccggcggcaagattacttccggctctgctcccggcggcaagatcagtgtgttcttcaccgacaattccggttcggtctccgcaaccccgggcgacagctcgttcaagacggacaccactaccgttaccctgaatgcgaacaacgtcaccgatgccatctacaccacttcggagggcaagtccggctcgtatcaggatggcgacaccatcaccatcggcgcttccacggcgatcggtgacaccatcaccgtgaagctgcagggcaaggatgcggatggccaaacggtctccgcaacatacaagtacacgaagaaggatccggccgccaccagcacggcttatgcgaagaagccgagtgcgtggagcaacctgtacgcctatgtgtatgtagacgattcgagcgccaccactttgaaggaaaacgcgaagtggccgggcgaaccgatgacacaggtcgcttcgggagacacttgcggcaaggatggtgagtacaagtatgagattcccgacgatctcgagggaagcaatactcgcatcatcttcaacgatggcaatgccacgaatacccagaagtaccctgccgacgccaccgaaggcgtagatgccgctggcctcaagatcgacggcaattacgcttgggacggcaacacttcatccggcacctgggaggctcgcaattgtgtggtcaccccgaccaagtccgtgaggattgatcagtcggattacagcgtggacctgtccgatggcgtggccacgaagcagttgacagccacgaccgatccgaagggcgcgtccgtgagctggagctcgtccgacaaggacgtggcgaccgtcagcccgaagggcgtggtcaccccgaggaaggccggcaaggccacgatcaccgcgaagtccgggaccaagaccgcgtcgatcaccgtgaccgtgaccggtgagcttccgcctgacccggtcgcgaagaacaccgtctacgcttcgaagccctcgggctggggcaagatctacgcgtacgtgtacacgggcgacggcgcgaccgcggcgaacaacgcggcctggccgggcgtggagatgaccgccccgagcgcgaccgacggctgccagcagaccgacctgtacaagtacgaggtcccggacagcctcgccaagggcgcgaaggtgatcttcaacgacggcggcagccagcagtatccgggatcccgccagccgggcctggactacaacggcggcatcgtgaagtgggacggctcctccgcggccctggccgcggtcgagtgcgagaccaccatcccggtcacgtccgtgtcggtctctggtgatggtgtgagcggcggcaagctctcgctgaagtccggggcgagcgtgcagctgaccgcgacggtcaagcccgacaacgcgacggaccgcaaggtcacgtggacgagctcggactcgagcgtcgcgaacgtgatgggcaccggcgtggtcacggccggctcgaaggccggcaaggccacggtcaccgcgaccgccggcggcgtgagcgcgtccgtcgaggtcacggtcgaggcgcaggatccgtacgccgagctggacgcgttggcgaaggcccacgcgtcggatctggaggacggcacgtacgcggtgtcgaccgcgctgaaggacggcatggtccttgacgtggcggacggatcgaggaaggacggcgcgaacgtgcggctgtggtcgtcgaacgggacgaaggcgcagcagtggacggtttcgcacgactcgaagggctacgtgacgctgaggaacgtgaattccggcaaggcgctggatgtgaaggacggcaaggccgcgaacggttcgaacgtgcatcagtacgcgccgaactcctaccgttcgcagaagtgggtggcggtcaggagcggatcggtgtacaaactggtgtccgcgctctccccgtccatggcgctggacgtgaaggacggcaaggccgcgaacggttcgaacgtgcagatctacaccgccaacgggtaccgttcccagcagtggacgttcaaaacggtcgcccagccgttgaagtcggcgacggtctggtaccgtccctcgtccgcgcagtcgcgcgtgcgcgtgcagtggcgcgtgtacggcagtccggacacgaccggcggcatggagatgacgcaggcgtgcggaggctggtggaaggccacggtgccttccgcgggctccacgagggtcggtctgtcgttctcgtatggttccacgacggatgacaacggcgggaagctgtacgacgtgaagggcgagtccgcggccgtctcgggcgggcaggccgtgaccgacgtcacaccaaactgcgcggtaaccaacaaatga

SEQ ID NO: 69 - DNA, 2445 bp, Bacteroides sp.
  source: /note="GH31.0-5"
atgaaaatacatcatctattttggggtatatgtttatgcttcagcacaaatatcttattcgcacagaactatcagaaaacatcgtccggcatcaaaaccactgtaaatgcagtggatatagaagtacaattttttgcgcctgctgtggcgagagtaataaagtcaccggaaggtgttgcctatgaaaaacagagtctttctgtaattgccaaacctgaaaaggtgagtttcaaagctgatatacaagataataagattgtattgaacaccagtgaactaagtgtcagtgtggacaccgggacgggaattgtttcttatttctcaaaggatggcaaatcattattggcagagaaatccggtatgcagtttatcgatttcgatgatgccgggacaaaaacttatcaggtttatcaaccttttgtattagataaggaggaagccatttatggtttgggacaattgcaaaatggaaagatgattcagcggaacatgactaaaaatctgatacagggaaatgttgaagatgtgtcacctttcttccagtctactaaaggatatggtgtgttttgggataactattcgccgactctttttacggataacgaagttgaaacatctttccgttctgaagtaggtgactgtgtggattattacttcatgtatgggaaaaatgccgacggtgttatagcacaggtacgcagcctgaccgggcaagcaccgatgtttcctttatggacttatggttactggcaaagtaaagaaagatataagagccaggaggaagtggtagacgttgttcgtaaatatcgtgaattgggtgttcccttggatggtattattcaggattggcaatattgggggcataactatttgtggaatgcgatggatttccagaatccgactttcaatcatcctcaaaagatgattgaggatgtccatgcgatgaacgcacacatggctatatctatctggtcgtcattcggaccgatgaccaagccttatagagaattggataaaaaaggaatgttgtttaacttcactacctggccgcaatcgggattggagtcatggccccccaacatggaatatccttccggtgtaagagtgtatgatgcttacaatcccgaagcgcgtgatatttattggcaatatctgaatgatggaattttcaagctgggaatggatgcctggtggatggactctaccgaacccgatcatctggattggaagccggaggatatggataccaaaacctatctgggctcgttccgtaaggtgcgcaatgcttatccgttgatgactgtcggaggggtttacgaccatcagcgtgcaatgacttcggacaaacgtgtgtttattttaacccgttcgggattcttggggcaacaacgttatggtgcaaatgtatggagtggtgatgtcgcttccacatgggagagttttagaaatcagattcctgccggattaaacttttctttgtgtggtatgcctcactggaatagtgatattggtggcttttttgcaggacattataataaaagctggaatgatgatagtgcttcgaaaaatccattgtatcaggagctttatgtgcgttggttgcagtttggaacgttcaatccgatgatgcgttcgcacgggacggatgtttatagggaaatctataagttcggaaagaagggtgagcctgtatatgatgctatcgagaagatgataggtttgcgttactctctgttgccttatatttattctacttcttgggaggtgagcaatcgccaatcgagttttatgcgcgctttgatgatggattttgtagatgacagaaaggtgtgggatatcaatgacgaatatatgtttggaaaatcgctccttgtggctccgattgctcatgcacaatatacaccggaagctgtggtaaaagtctccgaagaagaaggatggaacagagatggagcgaaaaaaacaaaaactgacgttgctgtggatttcatggaaacgaaatctactaacatatacttaccggcaggaacgctatggtatgacttctggacaaacgagaaacatgaaggcggaaaggaaattaccaaagagactacactggatgttattccattgtatgtaaaagcgggtagtattattcctgtcggtccacaagttcagtatgcaactgaaaaaccgtgggatcatcttgaattgaaggtgtatgcgggtgcgaatggaaacttcattttatatgaagatgaatttgataattacaattacgaaaaaggagcttatacggaaattccaatctcttggaataatgtatctcgtaaattgacgataggggcaagaaaaggtacgtatgagggaatgttgaagaaccgtaaatttactgtaactcttcaggacgggactcaaaaaaacgtcgattataatgggaaagcgatttctgtaaagttttga

SEQ ID NO: 70 - DNA, 2445 bp, Bacteroides sp.
  source: /note="GH31.0-8"
atgaaaatacatcatctattttggggtatatgtttatgcttcagcacaaatatcttattcgcacagaactatcagaaaacatcgtccggcatcaaaaccactgtaaatgcagtggatatagaaatacaattctttgcgcctgctgtggcgagagtaataaagtctccggaaggggttgcctatgaaaaacagagtctttctgtaattgccaaacccgaaaaggtgaatttcaaggctgatatgcaagataataagattgtattgaacaccagtgaactaagtgtcagtgtggacaccggaacgggaattgtttcttattgctcaaaggatggcaagtcgttattggcagagaaatccggtatgcagtttatcgatttcgatgatgccgggacaaaaacttatcaggtttatcaaccttttgtattagataaggaggaagccatttatggtttgggacaattgcaaaatggaaagatgattcagcggaacatgactaaaaatctgatacagggaaatgttgaagatgtgtcacctttcttccagtctactaaaggatatggtgtgttttgggataactattcgccgactctttttacggataacgaagttgaaacatctttccgttctgaagtaggtgactgtgtggattattacttcatgtatgggaaaaatgccgacggtgttatagcacaggtacgcaacctgaccgggcaagcgccgatgtttcctttatggacttatggttactggcaaagtaaagaaagatataaaagccaggaggaagtggtagacgttgttcgtaaatatcgtgaattgggtattcctttggatggtattattcaggattggcaatattgggggcataactatttgtggaatgcgatggattttcagaatccgactttcaataatcctcaaaagatgatggaggatgtccatgcgatgaacgcacacatggctatatctatctggtcgtcattcggaccgatgaccaaaccttatagagaattggacaaaaaaggtatgttgtttaacttcactacctggccgcaatcgggattggagtcatggccccccaacatggaatatccttccggtgtaagggtgtatgatgcttacaatcccgaagcacgtgatatttattggaaatatctgaatgatggaattttcaagctgggaatggatgcctggtggatggactctaccgaacccgatcatctggattggaagccggaggatatggataccaaaacctatctgggctcgttccgtaaggtgcgcaatgcttatccgttgatgactgtcggaggggtttacgaccatcagcgtgcagtgacttcggacaaacgcgtgtttattttaacccgttccggattcttggggcagcaacgttatggtgcaaatgtatggagtggtgatgtcgcttccacatgggagagttttagaaatcagattcctgccggattaaacttttctttgtgtggtatgcctcactggaatagtgatattggtggcttttttgcaggacattataataaaagctggaatgatgatagtgcttcaaaaaatccattgtatcaggagctttatgtgcgttggttgcagtttggaacgttcaatccgatgatgcgttcgcacgggacggatgtttatagggaaatctataagttcggaaagaaaggcgagcctgtatatgatgctatcgagaagatgataggtttgcgttactctctgttgccttatatttattctacttcttgggaggtgagcaatcgccaatcgagttttatgcgcgctttgatgatggattttgtagatgacagaaaggtgtgggatatcaatgacgaatatatgtttggaaaatcgatccttgtggctccgattgctcatgcacaatatacaccggaagctgtggtaaaagtctccgaagaagaaggatggagcagagatggagcgaaaaaaacaaaaactgacgctgctgtggatttcatggaaacgaaatctactaacatatacttaccggcaggaacgctatggtatgacttctggacaaacgagaaacatgaaggcggaaaggaaattaccaaagagactacacttgatgttattccattgtatgtaaaagcgggtagtattattcccgtcggtccacaagttcagtatgcaactgaaaaaccgtgggatcatcttgaattgaaggtgtatgcgggtgcgaatggaaacttcattttatatgaagatgaatttgataattacaattacgaaaaaggagcttatacggaaattccaatctcttggaataatgcatctcgtaaattgacgataggggcaagaaaaggtacgtatgagggaatgttgaagaaccgtaaatttactgtaactcttcaggacgggactcaaaaaagcgtcgattataatgggaaggcaatttctgtaaggttttga

SEQ ID NO: 71 - DNA, 1707 bp, Bacteroides sp.
  source: /note="GH43.12-12"
atgtcaatcgtccggctctccatatttatgttggggataacaatgatgtcatgtaactcaaagaaagaacaacaattaccggctattggaaaatctgtggctctctttgattatttttcttataaaggaaatgatgatttttatatttccaatcctctgtcagatgaagactatttctataatcctattttgccgggatggtattctgatcctagtgtttgcacaaatggagaaggtgattatttcctggtaacatctacattcacttatttccccggtgttcctatttttcacagcaaagacttggtgaattggaaacagatagggcatgtgttgaaccgtgcttcgcaattagtgaatatggaaggacagaaagtgagtggcggtatttttgctccggctatttcttataatccgtataacaagacatattatatggtaacaaccaatgtaggagccggaaatttctttgttaagacgcaagacccgtttggtgaatggtcggaacccgtcatgttgccggaggtcggaggtattgatccttctttcttttttgatgaagatggtaaggcatatattgttaataatgatgaggctccggataataagcctgaatatagcggacaccgtactatacgtatacaagagtttgatgtgaaaacagataagacgataggtccccgtaaaattcttgtaaacaaaggagctcaaccggcagacaaaccaatttggatagaaggccctcatttatataaaataaatggaaagtatttcttgatgtccgccgaaggtggaacggggaactggcattcagaagtgattttccgtggtgattctccgatgggtaaatttcttccatggaaaaacaatccgattctgacgcaaagacatttgaattctgaccgtcctaattcggtaacctgtgctggccatgcagacttgattcaaacaaaagagggagattggtgggctgtttttctggcttgtcgccctattaataatcagtttgagaatttgggacgtgaaacatttatgatgccggtgaaatggagtgaagacggattcccgtacatgacacaaggcgatgatttagttcctatgattgtaaaacgtgaaggtgcgaaacgcgatacgacagttacttatggtaacttcgagttagtagcgaactttgattctcctgtacttgacatgacttggatgactttgagagcttctgcttccgatttatattcattgacggaaacacccggatacctgaccttgaagtgtgcagatattagtgctacggaaaagaaaactccggcatttgtttgtcgtcggttacaacatcataaatttgaatgtgctacacgtatgttgttcaatccttctaacgataaggaaacagccggaatgctgttgtttaaaaatgagacgcatcaatatttcttctgcttgaataaagtgggtgagaataaaaatatttctctgaaacaaatcggtgaaaaggagcagacattggcttcagatgaaatagacgcagatacaaatgaggtatatttgaaattagtatctcaaggaattggttacgatttctattattctattgatggtgaaaaaagctggaaactgctttgtaaagatgtagatcctagttatctctctactacaacggctggtggatttaccggtactacaattggattatacgctacttgcaaataa

SEQ ID NO: 72 - DNA, 2808 bp, Unknown
  source: /note="Description of Unknown: Lachnospiraceae sequence"
  source: /note="GH36.0-1"
atggcaattatatacaatccaaataaaaaaatatttaccctgcatacggcgcatacaacttatcagatgcaggttgatccactgggatatctgttgcatttgtactacggagaaaaaacaaacagttccatggactatgtcctaacctatgcagaccgcggattttccggaaatccttatgcagccggtatggaccgcacctattcgctggatgcgctaccacaggaatatccgtcccttggcaccggagattaccgcaatattgcactgaatatcaaaaatgaaaaaggggtggaaagtgcggatctgctttttaaaagctatgaaatccgaaacggtaaataccggttgcagggacttccggctgtctgggcagacgaaaaggaagcgcagacactggaaattgtcctcgcagatgaaaacgcacaggttgaagtacatctgctgtacggtgttttggaagaaaacgatgtcattacaagaagtgtccggattaaaaatacaggaaccgggcagattacgatcgaaaaggcagcggcagcctgtctggattttgtacagggagagtttgatgtcctgcggttttatggaaaacatgccatggagcgcaatctggagcgtacgccgctgggacatggaaccattgcgtttggtagccgcaggggaacatccagccatcagtataatcctgccgtgattctggcagaaaaagggacaacggagaccgcaggcagctgctatggaatgctgtttgtatacagcgggaatttctcctgtgaggcagaaaaagaccagttcaaccagacgcgcctgcttctcggattaaatgaagaactgttttcctatccgcttgcgtcgggagaaacctttacggtgccggaagttattttatcttattcggcagagggattgtcggcattgtcgcagcagtatcataactgcatccgcaaccatgtgtgccgtagcaaatatgtccatatgcaacgcccagtactgatcaacagttgggaggcagcttattttgattttacgggagatacgatcgtggatctggcaaaagaagccgcttcccttggaattgatatggtagtgatggatgacggctggtttggaaaaagaaatgatgacaattcttccctgggggactggcaggtcaatgaaacgaaactgggaggcagtctggcagagcttattacccgtgtgcatgagcagggtatgaaatttggcatctggattgagccggagatgatcaatgaagacagtgacctttaccgggcgcatccggactgggcgatccggattcaggggaaaaagccggtgcgctcgagaaaccagttactgcttgatttttccagaaaagaagtgcgtgactgtgtctttgaccagatctgtgtcgtgctcgatcagggaaaaattgactatgtcaagtgggatatgaaccgcagcatggcagatgtttatgccggaaatctttcccatgattacgtccttggtgtctatgattttatggagcgtttgtgcagccggtatccggatcttttgctggaaggatgcagcggtggcggcggcagatttgacgcaggaatactttattattcccaacagatctggtgcagtgacaataccgatgcgatcaaccgcacaagaatccagtacggaacttcgtttttctatccggtttccgcgatgggagcgcacgtttcggcggtgccgaaccaccagaccggacgggtgacaagtttccacacccgcggggtgacggcgatggcgggaaccttcggttacgaattaaacccagcgcttttatccgatgaggaaaagcagcagatccgggagcagatcaaaacgtataagaagtacgaaatgctcattaacgagggaacctactggcggctgtctgatccgtttacagatgaaattgcggcatggatgtcggtatcagaggaacaggatcatgcactggtaagtgtggtgcgtcttatggctgaggcaaatcaggcgaccgtttatgtccgcctacgtgggttaaaaccggatgctgtgtatctggaagaacaaagcggcagacagtattccggtgcggcactgatgcatgcgggaattccgcttccgccgtttaccgaggaatatgaggcgtatcagtttgcctttaccgaactgaaagaggcgggaagattatatgaaaaagtgaagaaatggtgtgacgggaatgccgaaaaccgggtggtcatcagcatttacggtggctccggttccggaaaaacaacgcttgcaacggcattgcagcagtgctttttaaatgacggaaccggatgttatctgctctcgggcgatgattatccacaccggattccaaaacgcaacgacgaagaacggctgcgtgtgtataaagaagcaggggaagacggactgcgtggatatctcggaacaaagaaagagattgatttcgaccggatcaatgaagtgcttgcggcatttcatgagggaaaagatacgatcacgttgcggcatttgggacgggaagatggcgagatttcatcagaagaaaccgatttttccggaatatctgtattgcttctggagtggacgcacggaggcagtgacgatttacatggtgtggatctatccgtctttctggaaagttccccggaggagacaaaggagcggcgcatccgcagaaaccgcgacgagaatgccgcaagcccgtttatctgtcgtgtggtggaactggaacaggaaaaactcgaagtgcagcgcaaaaatgcaggattgatcgtgggaaaggacggaagtatttatgaacagtaa

SEQ ID NO: 73 - DNA, 1728 bp, Bacteroides sp.
  source: /note="GH43.12-7"
atgagaacattaaaattgattttgtcgggctggcaatccgtgggtcttgtcgtattttttatgctgttttttaatatggaggtgagtggcaagggtaaaataacaaaaaatgctcctgtctttacgcaatttatttatcagggggaggatgctatttatcaaaacaatcctttaaagccgggtgagttctataatcctattttgcagggttgctatcccgatccgagtataacgcggaaagggaatgattattatttagtgtgctcatcttttgctatgtttcccggggtgcctattttccattctaatgatctggtcaactggaaacaaatcggtcatgtgctggacagaacgtcacaattaaaggttgaagattgtggtattagtgctggtgtatatgctcctgctataagatataatcccaataatgatacgttttatatgataaccactcaattttccggtggctttggaaatatggtggtaaagacaaagaatccggagaatggctggagtgatccggtcaaacttcaatttgaaggcattgatccttctcttttctttgatgataatggcaaggcatacgtggtacataatgatgctcctgctaaagcaaatgagcgttactcgggacaccgtgtcataaaaatatgggattatgatgtggagaatgataaagtggttccgggaacggaccggatcatcgtaaacggtggcgtcaatatagaagaaaaaccgatatggattgaagctcctcatatctataagaaagatggacgttattatttaatgtgtgccgaaggaggaaccggaggctggcatagcgaagtcatttttgtaagtgatcatccgaaaggaccttatcttccggcaaataataatcctattttaactcaacgttattttcctgcaaaccgggcgaataaagtagactgggctggtcatgcagacttagtggagggacccgacggaaaatattatggtgtatttttgggaatacgccctaatgagaagaacagagtgaataccggacgcgaaacttttattcttccggtggactggagcggaacatttcctgttttcgaaaatgggcttatccctatgaaacctacattgaagatgccttcgggagtagagaaccaaacagggaaaaacggttatttgcctagtggcaactttgtctttaaggatgatttctccgataaaacattagacttaagatggattggtcttagagggcctcgtgaagaattcgttgatatgaccgataaagggttgcggatcatcccttttacctcaaatattaatgaagtgaaacctacttctactttgttctaccgtcagcagcataatcaatttacagcagcagcaaccatggagtacaaaccgaaaaatgagaaagattttgccggtataacatgttatcagaatgaaagatatcactatgttttcggtatcactaaaaagggaaaggactattacctgatactgcaaagaaccgaaaaaggacaagcgagtgtcctaggtgaggtgaagatagaaacagagaaacctgtgacactgcaagtaacagctaatggagatgattatcgttttaattattcgattgatggcaagggtttcctaaatttaggaggaaccgtttccggcgatattctttctactaatgaggctggtggctttacaggagcaatgattggactgtatgcaacatctgttggtaattaa

SEQ ID NO: 74 - DNA, 1728 bp, Bacteroides sp.
  source: /note="GH43.12-9"
atgagaacattaaaattgattttgtcgggctggcaatccgtggcgcttgtcgtattttttatgctgttttttaatatggaggtgagtggcaagggtaaaataacgaaaaatgctcctgtctttacgcaatttatttatcagggggaggatgctatttatcaaaacaatcctttaaagccgggtgagttctataatcctattttgcagggttgctatcccgatccgagtataacgcggaaaggtaatgattattatttggtgtgctcatcttttgctatgtttcccggggtacctattttccattctaatgatctggtcaactggaaacaaatcggtcatgtgctggacagaacgtcacaattaaaggttgaagattgtggtattagtgctggtgtatatgctcctgctataagatataatcccaataatgatacgttttatatgataaccactcaattttccggtggctttggaaatatggtagtaaagacaaagaatccggagaatggctggagtgatccggtcaaacttcaatttgaaggcattgatccttctcttttctttgatgataatggcaaggcatacgtggtacataatgatgctcctgctaaagcaaatgagcgttactcgggacaccgtgtcataaaaatatgggattatgatgtggagaatgataaagtggttccgggaacggaccggatcatcgtaaacggtggcgtcaatatagaagaaaaaccgatatggattgaagctcctcatatctataagaaagatggacgttattatttaatgtgtgccgaaggaggaaccggaggctggcatagcgaagtcatttttgtaagtgatcatccgaaaggaccttatcttccggcaaataataatcctattttaactcaacgttattttcctgcaaatcgggcggataaagtagactgggctggtcatgcagacttagtggagggacccgacggaaaatattatggtgtatttttaggaatacgccccaatgagaagaacagagtgaataccggacgcgaaacttttattcttccggtggactggagcggaacatttcccgttttcgagaatgggcttatccctatgaaacctacattgaagatgccttcgggagttgagaaccaaacagggaaaaacggttatttgcctagtggcaactttgtctttaaggatgatttctccgataagacattagaccttagatggatcggtcttagaggtcctcgtgaagatttcgttgatatgaccgataaagggttgcggatcatcccttttacctcaaatatcaatgaagtgaaacctacttctaccttgttctaccgtcagcagcataatcaatttacagcggcagcaaccatggagtacaaaccgaaaaatgagaaagattttgccggtataacatgttatcagaatgaaagatatcactatgttttcggtatcactaaaaaggggaaagactattacctgatactgcaaagaaccgaaaaaggacaagcgagtgtcctgggtgaggtgaagatagaaacagagaaacctgtgacactgcaagtaacagccaatggagatgattatcgttttaattattcgattgatggcaagggtttcctaaatttaggaggaaccgtttccggcgatattctttctactaatgaggctggtggctttacaggagcaatgatcggactgtatgcaacatctgttggttattaa

SEQ ID NO: 75 - DNA, 2445 bp, Bacteroides sp.
  source: /note="GH31.0-6"
atgaaaatacatcatctattttggggtatatgtttatgcttcagtacaaatgttttattcgcacaaaattatcagaaaacatcgtcgggtatcaagaccacagtgaatgcagtggatatagaagtacaattttttgcgcctgctgtggcgaggataataaagtctccggaaggtgttgcctatgaaaaagagagtctttctgtaattgcaaaacctgaaaaggtaagtttcaaagctgatataaaagataataagattgtattgaataccagtgaactaagtgtcagtgtggacaccgggacgggaattgtttcttatttctcaaaggatggcaaatcattattggcagagaaatccggtatgcagtttatcgatttcgatgatgccgggacaaaaacttatcaggtttatcaaccttttatattagataaggaggaagccatttatggtttgggacaattgcaaaatggaaagatgattcagcggaacatgactaaaaatctgatacagggaaatgttgaagatgtgtcacctttcttccagtccactaaaggatatggtgtgttttgggataactattcgccgactctttttacggacaacgaagttgaaacatcttttcgttctgaagtaggtgattgtgtagactattatttcatgtatgggaaggatgccgatggtgtaatagcacaagtacgcagcttgaccgggcaagcaccgatgtttcctttatggacttatggttactggcaaagtaaagaaagatataagagccaggaggaagtggtagacgttgttcgtaaatatcgtgaattgggtattcccttggatggcattattcaggattggcaatattgggggcataactatttgtggaatgcgatggattttcagaatccgactttcaataatcctcaaaagatgattgaggatgtccatgcgatgaacgcacacatggctatatctatctggtcgtcattcggaccgatgaccaagccttatagagaattggataaaaaagggatgttgtttaacttcactacctggccgcaatcgggattggagtcatggccccccaacatggaatatccttccggtgtaagagtgtatgatgcttacaatcccgaagcgcgtgatatttattggaaatatctgaatggcggaattttcaagctgggaatggatgcctggtggatggactctaccgaacccgaccatttggactggaagccggaggatatggataccaaaacctatctgggctcgttccgtaaggtgcgcaatgcttatccgttgatgactgtcggaggggtttacgaccatcagcgtgaagtgacttcggacaaacgtgtgtttattttaacccgttcgggatttttggggcaacaacgttatggtgcaaatgtatggagtggtgatgtcgcttccacatgggagagttttagaaatcagattcctgccggattaaacttttctttgtgtggtatgcctcactggaatagtgatattggtggcttttttgcaggacactataataaaagctggaatgatgatagtgcttcaaaaaatccattgtatcaggagctttatgtgcgttggttgcagtttggaacgttcaatccgatgatgcgttcgcacgggacggatgtttatagggaaatctataagttcggaaagaagggtgagcctgtatatgatgctatcgagaagatgataggtttgcgttactctctgttgccttatatttattctacttcttgggaggtgagcaatcgccaatcgagttttatgcgcgctttgatgatggattttgtagatgacagaaaggtgtgggatatcaatgacgaatatatgtttggaaaatcaatccttgtagctccgattgctcatgcacaatatacaccggaagctgtggtaaaagtctccgaagaagaaggatggaacagagatggagcgaaaaaaacaaaaactgacgctgctgtggatttcatggaaacgaaatctactaacatatacttaccggcaggaacgctatggtatgacttctggacgaacgagaaacatgaaggcggaaaggaaattaccaaagagactacactggatgttattccattgtatgtaaaagcgggtagtattattcctgtcggtccacaagttcagtatgcaactgaaaaaccgtgggatcatcttgaattgaaggtgtatgcgggtgcgaatggaaacttcattttatatgaagatgaatttgataattacaattatgaaaaaggagcttatacggaaattccaatctcttggaataatgcatctcgtaaattgacgataggggcaagaaaaggtgcgtatgagggaatgttgaagaaccgtaagtttactgtaactcttcaggacgggactcaaaaaaacgtcgattataatgggaaagcgatttctgtaaagttttga

SEQ ID NO: 76 - DNA, 1131 bp, Bacteroides sp.
  source: /note="GH76.0-5"
atgttattttgccttacttctgcagtgggaaagacaccgggaaatacccgttatctttctattgccgactcgattctatctaatgtattgaatctctatcagacgaatgacggactactaacagaaacgtatcctgtcaatcccaaccaaaaaatcacttatctggcgggcggaacgcagcagaacggaacgctgaaggcttcttttctatggccgtattccgggatgatgtcgggttgtgtggctttatacaaagcgaccggaaacaagaagtacaaaaagattctcgagaaaagaattctaccgggaatggagcagtattgggataacagtcgcttgccggcctgttatcagtcataccccaccaagtacgggcagcacggacgttattatgacgataacatctggattgcactggactattgcgattattaccaactgactcacaagcctgcatctttggaaaaagccgttgcattgtatcaatatatctacagtggatggagcgacgagatgggtggtggtattttttggtgtgaacagcagaaggaagcgaagcatacttgttccaatgcaccgtctactgtgctcggtgtcaagttgtaccggctgacgaaggatgccaaatacctcgaaaaagcaaaagagacgtatgcctggacgaaaaagcatctgtgcgaccctaccgaccatctttactgggataacatcaacctgaaagggaaagtttccaaagagaagtacgcctacaacagtggacagatgattcaggcgggtgtattgctctatgaggaaacgggagatgaacagtatttgcgcgatgcacagcagacagccgcaggaactgatgcttttttccgcacaaaagccgacaagaaagacccgactgtcaaagtgcataaagacatggcctggtttaacgtgatcttattcagaggactgaaagctctgtataagattgacaagaatccgacgtatgtcgatgcgatggtggaaaatgcgcttcacgcctgggaaaactaccgggatgaaaacggattattaggcagggattggtcgggacataacaaggagcagtataaatggctgctcgacaatgcctgtcttattgaattctttgcagagatttaa

SEQ ID NO: 77 - DNA, 1728 bp, Bacteroides sp.
  source: /note="GH43.12-10"
atgagaacattaaaattgattttgtcgggctggcaatccttggggcttgtcgtatttattatgctgttttttaatatggaggtgagtggcaagggtaaaataacaaaaaatgctcctgtctttacgcaatttatttatcagggggaggatgctatttatcaaaacaatcctttaaagccgggtgagttctataatcctattttgcagggttgctatcccgatccgagtataacgcggaaagggaatgattattatttagtgtgctcatcttttgctatgtttcccggggtgcctattttccattctaatgatctggtcaactggaaacaaatcggtcatgtgctggacagaacgtcacaattaaaggttgaagattgcggtattagtgctggtgtatatgctcctgctataagatataatcccaataatgatacgttttatatgataacgactcaattttccggtggctttggaaatatggtggtaaagacaaagaatccggagaatggctggagcgatccggtcaaacttcaatttgaaggcattgatccttctcttttctttgatgataatggcaaggcatacgtggtacataatgatgctcctgctaaagcaaacgagcgttactcgggacaccgtgtcataaaaatatgggattatgatgtggaaaatgataaagtggttccgggaacggaccggatcattgtaaacggtggcgtcaatatagaagaaaaaccgatatggattgaggctcctcatatctataagaaagatggacgttattacttaatgtgtgcggaaggaggaaccggaggctggcatagcgaagttatttttgtaagtgatcatccgaaaggaccttatcttccggcaaataataatcctattttaactcaacgttattttcctgcaaaccgggcggataaagtagactgggctggtcatgcagacttagtggagggacccgacggaaaatattatggtgtatttttaggaatacgccccaatgagaagaacagagtgaataccggacgcgaaacttttattcttccggtggactggagcggaacatttcccgttttcgagaatgggcttatccctatgaaacctacattgaagatgccttcgggagtagagaaccaaacagggaaaaacggttatttgcctagtggcaactttgtctttaaggatgatttctccgataagacattagattttagatggatcggtcttagaggtcctcgtgaagaattcgttgagatgaccgataaagggttgcggatcatcccttttacctcaaatatcaatgaagtgaaacctacttctaccttgttctaccgtcagcagcataatcaatttacagcggcagcaaccatggagtacaaaccgaaaaatgagaaagattttgccggtataacatgttatcagaatgaaagatatcactatgttttcggtatcactaaaaagggaaaagactattacctgatactgcaaagaaccgaaaaaggacaagcgagtgtcctgggtgaggtgaagatagaaacagagaaacctgtgacactgcaagtaacagccaatggagatgattatcgttttaattattcgattgatggcaagagtttcctaaatttaggaggaaccgtttccggcgatattctttctactaatgaggctggtggctttacaggagcaatgattgggctgtatgcaacatctgttggttattaa

SEQ ID NO: 78 - DNA, 1158 bp, Bacteroides sp.
  source: /note="GH76.0-3"
atgagaaatatatgttttgtagcctgtatgttattttgccttacctccgcagtgggaaagacaccgggaaatacccgttatctttctattgccgactcgattctatctaatgtattgaatctctatcagacgaatgacggactactaacagaaacgtatcctgtcaatcccaaccaaaaaatcacttatctggcggacggaacgcagcagaacggaacgctgaaggcttcttttctatggccgtattccgggatgatgtcgggttgtgtggctttatacaaagcgaccggaaacaagaagtacaaaaagattctcgagaaaagaattctaccgggaatggagcagtattgggataacagtcgcttgccggcctgttatcagtcataccccaccaagtacgggcagcacggacgttattatgacgataacatctgggttgcactggattactgcgattattaccaactgactcacaagcctgcatctttggaaaaagccgttgcattgtatcaatatatctacagtggatggagcgatgagataggcggtggcatcttttggtgtgaacagcagaaggaagcgaagcatacttgttccaatgcaccgtctactgtgctcggtgtcaagttgtaccggctgacgaaggatgccaaatacctcgaaaaagcaaaagagacgtatgcctggacgaaaaagcatctgtgcgaccctaccgaccatctttactgggataacatcaacctgaaagggaaagtttccaaagagaagtacgcctacaacagtggacagatgattcaggcgggcgtattgctctatgaagaaacgggagatgaacagtatttgcacgatgcacagcagacagccgcaggaactgatgcttttttccgcacaaaagccgacaagaaagacccgactgtcaaagtgcataaagacatggcctggtttaacgtgatcttattcagaggactgaaagctctgtataagattgacaagaatccggcgtatgtcaatgcgatggtggaaaatgcgcttcacgcctgggaaaactaccgggatgaaaacggattattaggcagggattggtcgggacacaacaaggaacagtataaatggctgctcgacaatgcctgtcttattgaattctttgcagagatttaa

SEQ ID NO: 79 - DNA, 2556 bp, Bacteroides sp.
  source: /note="GH2.0-2"
atgatgattggtaaactaaaatatttgatgctggggggctgccttatactggggagctgcttggcattgggaggctgtctgatgttattaggagcatgtagcagttctccccttgtatctccgcgggagcgatccgactttaatgcagactggcgttttcatttgggagacgggctgcaagcggcacaacctggttttgccgacaatgactggcgtgtactggatttgccccacgactgggcgattgaaggagacttcagtcaggaaaatccttccggtacaggaggaggggcacttccgggaggagtcggttggtatcgcaaaatctttagtgtagacaaagcggatgcaggaaagatatttcgcattgagtttgacggagtatatatgaactcggaggtatttatcaatggtgtttcattgggagtacgtccttatggatatattagtttcagctatgacctgactccttatctgaaatgggatgaaccgaatgtgctggctgtacgtgtggataatgcggagcaacctaattcacggtggtattcaggttgtggcatttaccggaatgtgtggctaagcaagaccggcccaatacatgtgggtggatggggaacgtatgtcacaacctcgtcagttgacgaaaaacaggctgtactgaatctcgctactacccttgtgaatgaaagtgatacgaacgaaaatgttactgtctgttcttccttgcaggatgctgaaggcagagaagttgctgaaacccggtcgagcgggaaagcggaagccggtaaggaagttgtttttacccagcaactgactgtaaagcaacctcaactgtgggatattgatactccttatctgtatacactggttaccaaagtgatgcgaaacgaagaatgtatggataggtatactactcctgttggtattcgcacatttagttttgatgcccggaaaggattcacgttgaatggcaggcagacaaaaattaatggtgtgtgtatgcatcatgacctgggctgtttgggagcggcagtcaacacacgtgccattgaacggcaattgcaaattctgaaagaaatggggtgtaacggcatacgttgttcccataatcctcccgcacccgaactgcttgatctttgtgaccgtatgggatttatcgtgatggatgaggcttttgatatgtggcggaagaaaaaaacggcacatgattatgcccgttacttcaatgaatggcacgagcgcgatttgaatgactttattttgcgtgaccgtaatcatccttctgtctttatgtggagtatcggtaatgaagtcctcgaacaatggagtgatgccaaagcggatacgttgagtctggaagaggccaatctgatcttaaatttcggacattcttctgaaatgttagccaaagaaggagaggagagtgtcaactctttgctgacgaaaaaactggtaagctttgtaaaagggcttgatcctgcccgtcctatcactgccggatgcaatgaaccgaattccggcaatcatttattccgttccggcgtactggatgtgattggctataattatcataacaaggatattcccaatgttccggctaatttcccggacaagccgtttatcattactgaaagcaattcagcgttgatgactcgcggatattaccgtatgcccagcgacaggatgtttatctggcccgagcgttgggacaaatcctttgccgattccacatttgcctgttcatcttatgaaaactgtcatgtgccttggggaaacactcatgaggaaagcttgaaattagtcagggacaacgactttatcagcgggcaatatgtatggacgggatttgattatatcggggaaccgactccttatggatggcctgcgcgtagttcgtactttggtattgtagatctggctggtttcccgaaagatgtctactatttgtatcagtcggaatggacggataagcaggtgttgcaccttttcccgcactggaactggactccgggacaggagattgatatgtggtgctactataatcaggctgatgaagtggaactgtttgtgaatggaaagtcgcaaggagtgaagcgtaaagaccttgataatctgcatgtagcttggcgtgtgaagtttgaaccgggaacggtgaaggtcattgcacgagagagtggtaaggtagtggcggaaaaggaaatctgcacagccggaaaacccgcagagattcgtctgactcctgatcgttctattctgactgctgatggaaaagatttgtgttttgtcactgtggaggtgttggatgagaaaggaaatctttgccctgatgctgacaatctagtgaatttcacagtacaaggtaatggctttatcgcaggggtagacaacggaaacccggtatcgatggaacgctttaaggatgaaaagaggaaagcattttatggaaaatgccttgttgtcattcagaacgatggaaaaccgggaaaagcaaagctgacggctacttcagagggacttcggcaagctgtactaaagatttcggcagaggaattgtaa

SEQ ID NO: 80 - DNA, 1728 bp, Bacteroides sp.
  source: /note="GH43.12-11"
atgagaacattaaaattgattttgtcgggctggcaatctgtgggtcttgtcgtatttattgtgctgttttttaatatggaggtgagtggcaagggtaaaataacaaaaaatgctcctgtctttacgcaatttatttatcagggggaggatgctatttatcaaaacaatcctttaaagccgggtgagttctataatcctattttgcagggttgctatcccgatccgagtataacgcggaaaggtaatgattattatttagtgtgctcatcttttgctatgtttcccggggtgcctattttccattctaatgatctggtcaactggaagcaaatcggtcatgtgctggacagaacgtcacaattaaaggttgaagattgtggtattagtgctggtgtatatgctcctgctataagatataatcccaataatgatacgttttatatgataaccactcaattttccggcggctttggaaatatggtggtaaagacaaagaatccggagaatggctggagtgatccggtcaaacttcaatttgaaggcattgatccttctcttttctttgatgataatggcaaggcatacgtggtacataatgatgctcctgctaaagcaaacgagcgttactcgggacaccgtgtcataaaaatatgggattatgatgtggaaaatgataaagtggttccgggaacggaccggatcatcgtaaacggtggcgtcaatatagaagaaaaaccgatatggattgaggctcctcatatctataagaaagatggacgttattacttaatgtgtgcggaaggaggaaccggaggctggcatagcgaagtcatttttgtaagtgatcatccgaaaggaccttatcttccggcaaataataatcctattttaactcaacgttattttcctgcaaaccgggcggataaagtagactgggctggtcatgcagacttagtggagggacccgacggaaaatattatggtgtatttttaggaatacgccccaatgagaagaacagagtgaataccggacgcgaaacttttattcttccggtggactggagcggaacatttcctattttcgagaatgggcttatccctatgaaacctacattgaagatgccttcgggagtagagaaccaaacagggaaaaacggttatttgcctagtggcaactttgtctttaaggatgatttctccaataagacattagattttagatggattggtcttagaggccctcgtgaagaattcgttgatatgaccgataaaggattgcggatcgtcccttttacctcaaatatcaatgaagtgaaacctacttctaccttgttctaccgtcagcagcataatcaatttacagcggcagcaaccatggagtacaaaccgaaaaatgagaaagattttgccggtataacatgttatcaaaatgaaagatatcactatgttttcggtatcactaaaaaggggaaagactattacctgatactgcaaagaaccgaaaaaggacaagcgagtgtcctgggtgaggtgaagatagaaacagagaaacctgtgacactgcaagtaacagccaatggagatgattatcgttttaattattcgattgatggcaagggtttcctaaatttaggaggaaccgtttccggcgatattctttctactaatgaggctggtggctttacaggagcaatgatcggactgtatgcaacatctgttggttattaa

SEQ ID NO: 81 - DNA, 2244 bp, Bacteroides sp.
  source: /note="GH92.0-6"
atggctttcacccttctccccgtatttgggggagagggtaaggccccccctatgaataaggaaaagagtctgttgatagattatgtagatccttttattggaacgacaaatttcggtaccactaatcccggagctgtttgcccgaatggaatgatgtccgtagtaccttttaatgtgatgggttctgctgataatacttatgataaagatgcacgttggtggtccacgccttatgaatataccaattgtttctttacaggatattctcatgtaaatctgagtggtgtcggttgtcctgaactgggttctttattgctgatgcctactaccggagaactgaatgtagactataaggaatatgggagcaaatataaggatgaacaggcttctcccggctattattccaattatctgacgaagtataatataaagacagaagtctctgctactccgcgtacaggtattgcccgtttcacttttcctagaggaaagagtcatatacttctgaatttgggcgaaggcctgaccaatgagagtggagccatgcttcgtcgtgtaagtgacagcgaaatagagggaatgaaactattgggtactttctgttataatccccaagctgtatttcccatctattttgtgatgagagtgaacaaagttcccaccacaaccggatattggaaaaagcaacgtccgatgacaggtgtggaagcagaatgggatcgagaccaaggcaaatataaattgtatacccgctatggaaaagaaatagcaggtgacgatgtgggcgcttacttcacttttgaaacagaggaaggagaacaggtcgaagtacagatgggagtttcctttgtaagcatagagaatgcccgtttgaatttggataaagaacagtcgggaaaaaactttgaacaggtgctttccgatgcccgtgcacagtggaacgatgacttgtcacgtatcactgtagaaggaggaacggatgcacagaaaacagttttttatacggcactttatcatttgttgattcatccgaacgttctgcaggatgtaaatggtgaatatccggctatggagagcgatcagattttgacaacgaaaggtacccgatatactgtattctctttgtgggatacatatcgtaacgtacatcagcttttgactttggtttatcccgaacgtcagatggaaatggtacgtaccatgctcgatatgtatcgtgaacatggttggtttcctaaatgggaattgtatggaagagagactcttacgatggaaggtgatccaagtatcccagtgattgtggatacatggatgaaaggattgcgtgactttgacgtagatctggcttatgaagctatgtacaagtcggctacattacccggggcggaaaatctgatgcgtccggacaatgatgactatatgtcaaaaggatacgtgccgcttcgtgaacaatatgataactccgtatctcatgcactggaatattatatcgcagactttgccctttcccgttttgcggatgctttaggaaagaagaaagatgcggaaatgttctataaacgctctttgggatataagcattattatagtaaggagttcggtacattccgacctattcttccggacggaactttctacagtccgttcaatccgaggcagggagagaactttgaaccgaatcccggtttccacgaaggtaattcttggaattatactttctatgtaccacatgatgtatatggattggctaaactgatgggtggaaagaaaccttttgtcaataagctgcaaatggtgtttgatgaaggactatatgatccggctaacgaaccggatattgcttacgctcatctgttctcttactttaaaggtgaagaatggcgtacacagaaagagacacagcgactgctggataagtactttacgaccaaaccggacggtatccctggaaatgatgacacaggtacgatgtctgcatgggctattttcaatatgataggtttttatcccgactgtccgggattgccggaatatacattgactactccggtatttaataaagtaacgatccgcttggatcctaaatggtataaggaaaatgagctggtaattgagagtaatcgtaccggatcggaaactctttatataaataaggtgttattggatggtaagaagttcaataaataccgcattacccacgatgaacttgttcatggtaaacgcttgatatttgatttgaaataa

SEQ ID NO: 82 - DNA, 1701 bp, Bifidobacterium sp.
  source: /note="GH51.0-4"
atgaccactcacaacagccagtattccgccgaaaccacccatcccggcaagcaggaaagcagcccggcgccgaccgccgccggcaccacggccagtaacgtctccacaactggcaacgcaaccacgccggacgccagcatcgccctcaacgccgacgccactccggtagccgacgttcccccgcgtctgttcggctcattcgtagaacatctgggccgctgcgtctacggcggcatctacgagcccagccatcccaccgccgacgaaaacggcttccgccaagacgtgcttgacctggtcaaggagctgggcgtcacctgcgtgcgctaccccggcggcaatttcgtatccaactacaactgggaagacggcatcggtccacgcgagaatcgccccgtgcgccgcgacctggcctggcattgcaccgaaaccaacgagatgggcatcgacgacttctaccgctggagccagaaagccggcaccgaaatcatgcttgccgtcaacatgggcacccgggggctgaaagccgcgctcgacgagctcgagtatgtcaacggcgcgcccggcaccgcttgggcggatcagcgcgtggccaacggcatcgaggagccgatggatatcaagatgtggtgcatcggcaacgaaatggacggcccgtggcaggtgggccacatgagcccggaagaatatgccggcgcggtggataaggtggcccacgccatgaagctcgccgagtccggtctcgaactcgtggcctgcggttcctcgggtgcctatatgccgaccttcggcacgtgggagaagaccgtgctcaccaaggcttacgagaatctcgacttcgtctcctgccatgcctactacttcgaccgcggccataaaacccggaccgccgcctccatgcaggacttcctggcctcttccgaagacatgaccaagttcatcgccaccgtctcggacgcggccgatcaggcgcgagaagccaacaacggcgccaaagacatcgccctgtccttcgacgaatggggcgtatggtattcggacaagtggaacgagcaggaagaccagtggaaggcggaggccgcgcagggtttgcaccacgagccatggcctaagtctccgcatttgctggaagacatctacaccgcggccgacgcggtggtcgaaggttccctgatgatcaccctgctcaagcactgcgatcgcgtgcgttccgcctcgcgcgcccagctggtcaacgtcatcgcccccatcatggccgaggaacacggcccggcatggcggcagaccacgttctacccgttcgccgaagccgcccttcacgcgcgcggccaggcctacgctccggccatcagctcccccaccatccataccgaggcatatggcgacgtgccggccatcgacgcggtagtcacgtgggatgaacaggcccgcaccggtctgctgcttgccgtcaaccgtgacgccaacaccccgcacacgctcaccatcgacctttccgggctgcccggcctgcccggtctcggcacgctcgcgctcagcaaggcgcaactgttgcatgaggacgatccgtaccgcaccaacaccgccgaagcgcccgaagccgtcacgccgcaaccgctcgacattgcaatgaacgccaccggcacctgcacggcaacgcttcccgccatctcctggatcagcgtggaattccacggctaa

SEQ ID NO: 83 - DNA, 2058 bp, Klebsiella sp.
  source: /note="GH42.0-3"
atgaataaatttgcacctttacatccgaaggttagtacgctgctgcatggcgcggattataatccggagcaatgggagaatgaccccgatattattgataaagacattgccatgatgcagcaggcaaaatgcaatgtgatgtcggtgggaatatttagctgggcgaaactggagccacgcgaaggggtatttaatttcgcctggctggatattatcctcgataaactgtataccgccggcattcatgtctttctggccacgccgagcggcgcgcgtccggcgtggatgtcgcagcgctatccgcaggttctgcgggtggggcgcgatcgggtgccggccctgcacggcggccgtcacaaccactgtatgtcgtcaccggtctatcgcgagaaaaccctgaaaatcaacaccctgctggcagaacgttattcctcacacccggcggtgctgggctggcatatttccaacgaatatggcggtgaatgccattgcgatctctgccagaaccgttttcgcgactggctgaaggcgcgttaccagaccctggagaacctcaaccaggcctggtggagcaccttctggagtcatacctatactgactggtcgcagattgaatcgcctgcgccgcagggcgagatgtcgatccacggtcttaatcttgactggcatcgctttaataccgctcaggtgaccgatttctgccgccatgaaattgctccgctgaaggcggcgaatgcctccctgccggtgactaccaactttatggagtatttctacgattacgactactggcagctggcggaggcgctggatttcatctcctgggacagctatccgatgtggcaccgcgataaagacgaaaccgcgctggcctgctacaccgcgatgtatcacgacatgatgcgcagcctgaagggcggcaaaccgtttgtgctgatggagtccaccccgggcgccaccaactggcagccgaccagcaaactgaagaagccgggaatgcatattctttcctcgctacaggcggtggcgcatggcgccgactcggtgcagtatttccagtggcggaaaagccgcggttcggttgagaaatttcacggcgcagtggtcgaccacgtcggacatattgatacccgcattggccgcgaagtctgccagctcggcgagatcctcagcaagctgccggaggtgagaggctgtcgcaccgaggcgaaagtagcgattatcttcgaccagcagaaccgctgggcgctggatgacgcccaggggccgcgtaatcttgggatggaatatgagaagacggtcaacgagcactaccgcccgttctgggagcagggcatcgccgtcgatgtgattgacgccgatgtcgatttaacgccgtatcagttagtgattgccccgatgttatatatggtgcgcgacggctttgccggtcgggcggaggcgtttgtcgccaacggcggccacctggtgaccacctactggaccggtatcgtcaatgagtccgatctctgctatctcggcggcttcccgggcccgctgcgcaatctgctggggatctgggcggaagagatcgactgcctgaatgaaggcgagtttaatctggtgcaggggcttgccgggaatcagtgcggtctgcagggcccttatcaggtgcgccatctctgcgaactgatccatatcgagagcgcccaggcgctggccacctaccgggatgatttttatgccggacggccggctgtgacggtgaacgcgttcgggaaaggcaaagcctggcatgtggcctcccgcaacgatttagccttccagcgcgatttctttaccgccctgagcaaggagctggccctgccgcgggcgatagcgacggagttaccacccggcgtggtggcgactgcgcgcaccgacggtgacaacgcatttatcttcctgcagaactacagcgcgcaaaaccataccctgaccctgccgcaagggtatcgggattgcctgaccgacgcggcggtatcggctccactgaccctgtcggcatgggattgccgtattctccgtcgtcacgcgtaa

SEQ ID NO: 84 - DNA, 2058 bp, Klebsiella sp.
  source: /note="GH42.0-4"
atgaataaatttgcacctttacatccgaaggttagtacgctgctgcatggcgcggattataatccggagcaatgggagaatgaccccgatattattgataaagacattgccatgatgcagcaggcaaaatgcaatgtgatgtcggtgggaatatttagctgggcgaaactggagccacgcgaaggggtatttaatttcgcctggctggatattatcctcgataaactgtatgccgccggcattcatgtctttctggccacgccgagcggcgcgcgtccggcgtggatgtcgcagcgctatccgcaggttctgcgggtggggcgcgatcgggtgccggccctgcacggcggccgtcacaaccactgtatgtcgtcaccggtctatcgcgagaaaaccctgcaaatcaataccctgctggcagaacgttattcctcacacccggcggtgctgggctggcatatttccaacgaatatggcggtgaatgccattgcgatctctgccagaaccgttttcgcgactggctgaaggcgcgttaccagaccctggagaacctcaaccaggcctggtggagcaccttctggagtcatacctatactgactggtcgcagattgaatcgcctgcgccgcagggcgagatgtcgatccacggtcttaatcttgactggcatcgctttaacaccgctcaggtgaacgatttctgccgccatgaaattgctccgctgaaggcggcgaatgcctccctgccggtgactaccaactttatggagtatttctacgattacgactactggcagctggcggaggcgctggatttcatctcctgggacagctatccgatgtggcaccgcgataaagacgaaaccgcgctggcctgttacaccgcgatgtatcatgacatgatgcgcagcctgaagggcggcaaaccgtttgtgctgatggagtccaccccgggcgccaccaactggcagccgaccagcaaactgaagaagccgggaatgcatattctttcctcgctgcaggcggtggcgcatggcgccgactcggtgcagtatttccagtggcggaaaagccgcggttcggttgagaaatttcacggcgcagtggtcgaccacgtcggacatattgatacccgcattggccgcgaagtctgccagctcggcgagatcctcagcaagctgccggaggtgagaggctgtcgcaccgaggcgaaagtagcgattatcttcgaccagcagaaccgctgggcgctggatgacgcccaggggccgcgtaatcttgggatggaatatgagaagacggtcaacgagcactaccgcccgttctgggagcagggcatcgccgtcgatgtgattgacgccgatgtcgatttaacgccgtatcagttagtgattgccccgatgttatatatggtgcgcgacggctttgccggtcgggcggaggcgtttgtcgccaacggcggccacctggtgaccacctactggaccggtatcgtcaatgagtccgatctctgctatctcggcggcttcccgggcccgctgcgcaatctgctggggatctgggcggaagagatcgactgcctgaatgacggcgagtttaatctggtgcaggggcttgccgggaatcagtgcggtctgcagggcccttatcaggtgcgccatctctgcgaactgatccatatcgagagcgcccaggcgctggccacctaccgggatgatttttatgccggacggccggctgtgacggtgaacgcgttcgggaaaggcaaagcctggcatgtggcctcccgcaacgatttagccttccagcgcgatttctttaccgccctgagcaaggagctggccctgccgcgggcgatagcgacggagttaccacccggcgtggtggcgactgcgcgcaccgacggtgacaacgcatttatcttcctgcagaactacagcgcgcaaaaccataccctaaccctgccgcaagggtattgggattgcctgaccgacgcggcggtatcggctccactgaccctgacggcatgggattgccgtattctccgtcgtcacgcgtaa

SEQ ID NO: 85 - DNA, 1158 bp, Bacteroides sp.
  source: /note="GH76.0-1"
atgagaaatatatgttttgtagcctgtatgttattttgccttacttccgcagtgggaaagacaccgggaaatacccgttatctttctattgccgactcgattctatctaatgtattgaatctctatcagacgaatgacggactactaacagaaacgtatcctgtcaatcccgaccaaaaaattacttatctggcgggcggaacgcagcagaacggaacgctgaaggcttcttttctatggccgtattccgggatgatgtcgggttgtgtggctttatacaaagcgaccggaaacaagaagtacaaaaagattctcgagaaaagaattctaccgggaatggagcagtattgggataacagtcgcttgccggcctgttatcagtcataccccaccaagtacgggcagcacggacgttattatgacgataacatctggattgcactggactattgcgattattaccaactgactcacaagcctgcatctttggaaaaagccgttgcattgtatcaatatatctacagtggatggagcgatgagataggcggtggcatcttttggtgtgaacagcagaaggaagcgaagcatacttgttccaatgcaccgtctactgtgctcggtgtcaagttgtaccggctgacgaagaatgccaaatacctcaaaaaagcaaaagagacgtatgcctggacaaaaaagcatctatgcgaccctaccgaccatctttactgggataacatcaacttgaaagggaaagtttccaaagagaaatacgcctacaacagtggacagatgattcaggcgggtgtattgctctatgaggaaacgggagatgagcagtatttgcacgatgcacagcagacagccgcaggaacagatgcctttttccgcacaaaagccgataagaaagacccgactgtcaaagtacataaagacatggcctggtttaacgtgatcttattcagaggactgaaagctctgtataagattgacaagaatccggcgtatgtcaatgcgatggtggaaaatgcgcttcacgcctgggaaaactaccgggatgaaaacggattattaggcagggattggtcgggacataacaaggagcagtataaatggctgctcgacaatgcctgtcttattgaattctttgcagagatttaa

SEQ ID NO: 86 - DNA, 1158 bp, Bacteroides sp.
  source: /note="GH76.0-2"
atgagaaatatatgttttgtagcctgtatgttattttgccttacctccgcagtgggaaagacaccgggaaatacccgttatctttctattgccgactcgattctatctaatgtattgaatctctatcagacgaatgacggactactaacagaaacgtatcctgtcaatcccaaccaaaaaatcacttatctggcggacggaacgcagcagaacggaacgctgaaggcttcttttctatggccgtattccgggatgatgtcgggttgtgtggctttatacaaagcgaccggaaacaagaagtacaaaaagattctcgagaaaagaattctaccgggaatggagcagtattgggataacagtcgcttgccggcctgttatcagtcataccccaccaagtacgggcagcacggacgttattatgacgataacatctggattgcactggattactgcgattattaccaactgactcacaagcctgcatctttggaaaaagccgttgcattgtatcaatatatctacagtggatggagcgatgagataggcggtggcatcttttggtgtgaacagcagaaggaagcgaagcatacttgttccaatgcaccgtctactgtgctcggtgtcaagttgtaccggctgacgaaggatgccaaatacctcgaaaaagcaaaagagacgtatgcctggacgaaaaagcatctgtgcgaccctaccgaccatctttactgggataacatcaacctgaaagggaaagtttccaaagagaagtacgcctacaacagtggacagatgattcaggcgggcgtattgctctatgaagaaacaggagatgaacagtatttgagcgatgcacagcagacagccgcaggaactgatgcttttttccgcacaaaagccgacaagaaagacccgactgtcaaagtgcataaagacatggcctggtttaacgtgatcttattcagaggactgaaagctctgtataagattgacaagaatccggcgtatgtcaatgcgatggtggaaaatgcgcttcacgcctgggaaaactaccgggatgaaaacggattattaggcagggattggtcgggacataacaaggagcagtataaatggctgctcgacaatgcctgtcttattgaattctttgcagagatttaa

SEQ ID NO: 87 - DNA, 2271 bp, Bacteroides sp.
  source: /note="GH92.0-4"
atgagacgtatattattaacttgcacaatggctttcacccttctccccgtatttgggggagagggtaaggccccccctatgaataaggaaaagagtctgttgatagactatgtagatccttttattggaacgacaaatttcggtaccactaatcccggagctgtttgtccgaatggaatgatgtccgtagtaccttttaatgtgatgggttctgctgataatacttacgataaagatgcacgttggtggtctacgccttatgaatataccaattgtttctttacaggatattctcatgtaaatctgagtggtgtcggttgtcctgaactgggttctttattgctgatgcctactaccggagaactgaatgtagactataaggaatatgggagcaaatataaggatgaacaggcttctcccggctattattccaattatctgacgaagtataatataaagacagaagtctctgctactccgcgtacaggtattgcccgtttcacttttcctaaaggaaagagtcatatacttctgaatttgggcgaaggcctgaccaatgagagtggagccatgcttcgtcgtgtaagtgacagcgaaatagagggaatgaaactattgggtactttctgttataatccccaagctgtatttcccatctattttgtgatgagagtgaacaaagttcccaccacaaccggatattggaaaaagcaacgtccgatgacaggtgtggaagcagaatgggatcgagaccaaggcaaatataaattgtatacccgctatggaaaagaaatagcaggtgacgatgtgggcgcttacttcacttttgaaacagaggaaggagaacaggtcgaagtacagatgggagtttcctttgtaagcatagagaatgcccgtttgaatttggataaagaacagtcgggaaaaaactttgaacaggtgctttccgatgcccgtgcacagtggaacgatgacttgtcacgtatcactgtagaaggaggaacggatgcacagaaaacagttttttatacggcactttatcatttgttgattcatccgaacgttctgcaggatgtaaatggtgaatatccggctatggagagcgatcagattttgacaacgaaaggtacccgatatactgtattctctttgtgggatacatatcgtaacgtacatcagcttttgactttggtttatcccgaacgtcagatggaaatggtacgtaccatgctcgatatgtatcgtgaacatggttggtttcctaaatgggaattgtatggaagagagactcttacgatggaaggtgatccaagtatcccagtgattgtggatacatggatgaaaggattgcgtgactttgacgtagatctggcttatgaagctatgtacaagtcggctacattacccggggcggaaaatctgatgcgtccggacaatgatgactatatgtcaaaaggatacgtgccgcttcgtgaacaatatgataactccgtatctcatgcactggaatattatatcgcagactttgccctttcccgttttgcggatgctttaggaaagaagaaagatgcggaaatgttctataaacgctctttgggatataagcattattatagtaaggagttcggtacattccgacctattcttccggacggaactttctacagtccgttcaatccgaggcagggagagaactttgaaccgaatcccggtttccacgaaggtaattcttggaattatactttctatgtaccacatgatgtatatggattggctaaactgatgggtggaaagaaaccttttgtcaataagctgcaaatggtgtttgatgaaggactatatgatccggctaacgaaccggatattgcttacgctcatctgttctcttactttaaaggtgaagaatggcgtacacagaaagagacacagcgactgctggataagtactttacgaccaaaccggacggtatccctggaaatgatgacacaggtacgatgtctgcatgggctattttcaatatgataggtttttatcccgactgtccgggattgccggaatatacattgactactccggtatttaataaagtaacgatccgcttggatcctaaatggtataaggaaaatgagctggtaattgagagtaatcgtaccggatcggaaactctttatataaataaggtgttattggatggtaagaagttcaataaataccgcattacccacgatgaacttgttcatggtaaacgcttgatatttgatttgaaataa

SEQ ID NO: 88 - DNA, 5676 bp, Bifidobacterium sp.
  source: /note="GH2.0-1"
atgagctccacgccggaggtggtctactccagcgccgtggattccaagcagaatcgcacctcggatttcgacgccaactggaagttcatgctgtccgattccgtgcaggcgcaggatccggcgttcgacgattcggcctggcagcaggtcgacctgccgcatgactacagcatcacgcagaagtactcgcagagtaatgaggccgaaagcgcgtaccttcccggcggcaccggctggtaccgcaagtccttcaccatcgaccgggacctcgccggcaagcgcatcgccatcaacttcgacggcgtgtacatgaacgccaccgtctggttcaacggcgtcaagctcggcacccatccgtacggctactcgccgttctccttcgacctgaccggcaacgccaagttcggtggggagaacaccatcgtcgtcaaggtcgagaacaggctgccgtccagccgctggtactccggctccggcatctaccgcgacgtcaccctcaccgtcaccgacggcgtgcacgtcggcaataacggcgtggccatcaagaccccgagcctcgccacccaaaacggcggcaacgtgacgatgaacctcaccaccaaggtcgccaacgacaccaaggccgcggcgaacatcaccctcaagcagaccgtgttccccaagggaggcaagaccgacgccgccatcggcaccgtcaccaccgcatccaagtccatcgcggccggtgccagcgcggacgtgacctccacgatcaccgccgcctcgcccaagctgtggagcatcaagaacccgaacctgtacaccgtgcgcaccgaagtgctcaacggcggcaaggtgctcgacacttacgacaccgaatacggcttccgctggaccggcttcgatgcgaccagcggtttctcgctcaacggcgagaaagtcaagctcaagggcgtctcaatgcatcatgaccagggatcgctcggtgcggtcgccaaccgccgcgccatcgagcgccaggtcgagattctccagaagatgggcgtcaactcgatccgcaccacgcacaaccccgcagccaaggcgctgattgacgtctgcaacgagaagggcgtcctcgtggtcgaagaggtcttcgacatgtggaaccggtcgaagaacggcaacaccgaggattacggcaagtggttcggccaggccatcgccggtgacaacgccgtcctgggtggcgacaaggacgagacctgggccaagttcgacctgaccagcaccatcaaccgtgacaggaacgccccgtccgtcatcatgtggtcgctcggcaacgagatgatggaaggcatcagcggcagcgtctcgggcttcccggctacctccgccaagctggtcgcatggacgaaggccgcggacagcacccgcccgatgacctacggcgacaacaagatcaaggccaactggaacgagtcgaacaccatgggcgacaacctgaccgccaacggcggcgtggtcggcaccaactactccgacggcgcgaactacgacaagatccgcacgacccacccctcatgggccatctacggttccgagacggcgtccgccatcaacagccgaggcatctacaaccgcaccaccggcggcgcccagtcaagcgacaagcagctgaccagctatgacaattccgcagtcggctggggtgccgtcgccagctccgcctggtacgacgtggtccagcgcgatttcgtcgccggcacatacgtgtggaccggcttcgactatctcggcgaacccaccccgtggaacggcaccggctccggcgccgtgggctcctggccgtcgccgaagaactcgtacttcggcatcgtcgacaccgcaggattcccgaaggacacctattacttctatcagagccagtggaacgacgacgtgcacacgctgcacatcctccccgcatggaacgagaacgtcgtcgccaagggctccggcaacaacgtgccggtcgtcgtctacaccgacgcggccaaggtcaagctgtacttcacaccgaagggcagcaccgaaaagcgactgatcggagagaagtccttcaccaagaagaccaccgcggccggatacacctatcaggtctacgagggcgccgacaaggactccaccgcccacaagaacatgtacctgacctggaacgtgccgtgggccgagggcaccatctccgccgaagcatacgacgagaacaacaggctgatccccgaggggtccaccgagggcaacgcgtcggtgaccaccaccggcaaggccgcgaagcttaaagccgatgccgaccgcaagacgatcaccgcggacggcaaggacctgtcgtacatcgaggtcgacgtgaccgacgccaacggccatatcgtccccgatgccgccaaccgcgtcaccttcgacgtcaagggcgccggcaaactggtcggcgtcgacaacggcagctcgccggatcacgactcctatcaggccgacaaccgcaaggcgttcagcggcaaggtgctcgccatcgtccagtccaccaaggaggcgggcgagatcaccgtcaccgccaaggccgacggtctgcaatcatccacagtgaagatcgccaccaccgccgtccccggcaccagcaccgagaagacggtccgcagcttctactactcgcgcaactactacgtcaagaccggcaacaagccgattttgccgagtgatgtcgaggtgcgctactccgacggcacgtcggaccgtcagaacgtcacatgggacgcagtcagcgacgaccagatcgccaaggccggttcgttcagcgtggccggcacggtcgccgggcagaagatctccgtgcgcgtgacgatgatcgacgagatcggtgcgctgctcaactattcggccagcacaccggtcggcacgcccgccgtgctgcctggctcgcgtccggccgtgctgcccgacggcaccgtgaccagcgcgaacttcgccgtcgactggaccaagcccgctgacaccgtgtacaacacggccggcaccgtcaaggtccccggcaccgccaccgtcttcggcaaggagttcaaggtcaccgcgacgatccgcgtgcagcggtcgcaggtcaccatcggcagcagcgtctccggcaatgcgctgcgcctgactcagaacatccccgccgacaagcagtccgacacgctggacgccatcaaggacggctccacgaccgtcgacgccaataccggcggcggcgcgaacccgtcagcatggaccaactgggcgtactcgaaggccggccacaacaccgccgagatcaccttcgagtacgcgaccgagcagcagctcggccagattgtcatgtacttcttccgcgacagcaacgcggtgaggttccccgacgccggcaagacgaagatccagatctccgcggacggcaagaactggacggatctcgctgccacggagaccatcgcggcccaggagtcgtccgaccgagtcaagccgtacacctatgacttcgctccggtgggagccacgttcgtcaaggtcacggtcaccaacgccgacaccacaacccccagcggcgtggtctgcgccggcctgaccgagatcgagctgaagaccgcgaccagcaagttcgtcacgaacacgtccgccgcgctctcgtcgctgacggtgaacggcacgaaggtctccgactccgtgctcgccgccggctcctacaacacgcccgcgatcatcgcggacgtcaaagccgagggcgaaggcaacgccagcgtcaccgtgctgcccgcgcacgacaacgtgatccgcgtgatcaccgagtccgaggaccacgtcacgcgcaagaccttcactatcaacctgggcacggagcaggaattccccgcagactccgatgaacgcgactacccggccgccgacatgacggtcaccgcgggtagcgaacagacgtccggcaccgcgaccgaaggcccgaagaaattcgcggtcgacggcaacaccagcacgtactggcattccaactggacgcccaccaccgtgaacgacctgtggatcgccttcgagctccagaaacccaccaagctcgacgcgctgcgctacctgccgcgccccgcgggcagcaagaacggctccgtcaccgaatacaaggttcaggtcagcgatgacggcaccaactggaccgacgcgggctccggcacatggaccaccgattacggctggaagctcgccgagttcaatcagccggtgaccaccaagcacgtgcggctcaaggccgtccacacctatgcggattccggcaacgacaagttcatgtccgcctccgaaatccgcctgcgcaaggccgtcgacaccaccgacatcagcggcgcgaccgtgaccgtgcccgccaagctgaccgtcgaccgggtggacgccgaccatcccgccaccttcgccacgaaggacgtgacggtgacgttgggcgacgccacgctgcgctacggcgtggactacctgctcgactacgcgggcaacaccgccgtcggcaaggccacggtgaccgtgcgcggcatcgacaagtactccggcaccgtcgccaagacgttcaccatcgaactgaagaacgccccggcgccggaaccgacgctgacctcggtgagcgtcaagaccaagccttccaagctgacctacgtggtcggcgacgcgttcgacccggcaggactggtgctgcagctcaactatgacgacgacagcaccggcaccgtgacctggaacacgcagacggccggcgacttcacgttcaagcctgcgctcgacgcgaagctcaaggtcaccgacaagaccgtcaccgtcacctaccagggcaagtccgcggtcatcgacatcaccgtctcgcagcccgccccgaccgtcagcaagacggatctggacaaggccatcaaggcgatcgaggccaagaacccggattcgtccaagtacacggccgactcgtggaagaccttcgcggacgccatggcgcatgccaaggccgtcatcgcggatgattccgccacccagcaggacgtcgataaggcgctcaaggcgctgaccgacgcctacgccgggctgaccgagaagacgcccgaacccgcccccgtcagcaagtccgagctggacaagaagatcaaggcgatcgaggccgagaagctggacgggtcgaagtacacggccgagtcgtggaaggcgttcgagaccgccctggcgcatgccaaggccgtcatcgccagcgattccgccacccagcaggatgtggacgcggcccttggcgccctgacctccgctcgcgacggactgaccgagaagggcgaggtcaagcccgacccgaagcccgaaccgggcaccgtcgacaaggcggcgctggataaggcggtcaagaaggtcgaggccgagaagctggacgggtcgaagtacacggccgactcgtggaaggcgttcgagaccgccctggcgcatgccaaggccgtcatcggcaacgccaactccacgcagttcgacatcgacaacgcgctgtcgatgctcaacgacgcccgcgccgcgctcaaggagaagcccggccgcatcatcgccatcatcgatggcggcgcactgagcaagaccggcgcatccgtcgccatcatcgcctccgtcgcggccgcgatgctggcggtcggtgccggcgtcatggcgttgcgccgcaagcgctcctga

SEQ ID NO: 89 - DNA, 1701 bp, Bifidobacterium sp.
  source: /note="GH51.0-5"
atgaccactcacaacagccagtattccgccgaaaccgcccatcccgacaagcaggaaagcagcccggcgccgaccgccgccggcaccacggccagtaacgtctccacaactggcaacgcaaccacgccggacgccagcatcgccctcaacgccgacgccactccggtagccgacgttcccccgcgtctgttcggctcattcgtagaacatctgggccgctgcgtctacggcggcatctacgagcccagccatcccaccgccgacgaaaacggcttccgccaagacgtgcttgacctggtcaaggagctgggcgtcacctgcgtgcgctaccccggcggcaatttcgtatccaactacaactgggaagacggcatcggcccacgcgagaatcgccccgtgcgccgcgacctggcctggcattgcaccgaaaccaacgagatgggcatcgacgacttctaccgctggagccagaaagccggcaccgaaatcatgcttgccgtcaacatgggcacccgggggctgaaagccgcgctcgacgagctcgagtacgtcaacggcgcgcccggcaccgcttgggcggatcagcgcgtggccaacggcatcgaggagccgatggatatcaagatgtggtgcatcggcaacgaaatggacggcccgtggcaggtgggccacatgagcccggaagaatatgccggcgcggtggataaggtggcccacgccatgaagctcgccgagtccggtctcgaactcgtggcctgcggttcctcgggtgcctatatgccgaccttcggcacgtgggagaagaccgtgctcaccaaggcttacgagaatctcgacttcgtctcctgccatgcctactacttcgaccgcggccataaaacccggaccgccgcctccatgcaggacttcctggcctcttccgaagacatgaccaagttcatcgccaccgtctcggacgcggccgatcaggcgcgagaagccaataacggcaccaaagacatcgccctgtccttcgacgaatggggcgtatggtattcggacaagtggaacgagcaggaagaccagtggaaggcggaggccgcgcagggtttgcaccacgagccatggcctaagtctccgcatttgctggaagacatctacaccgcggccgacgcggtggtcgaaggttccctgatgatcaccctgctcaagcactgcgatcgcgtgcgttccgcctcgcgcgcccagctggtcaacgtcatcgcccccatcatggccgaggaacacggcccggcatggcggcagaccacgttctacccgttcgccgaagccgcccttcacgcgcgcggccaggcctacgctccggccatcagctcccccaccatccataccgaggcatatggcgacgtgccggccatcgacgcggtagtcacgtgggatgaacaggcccgcaccggtctgctgcttgccgtcaaccgcgacgccaacaccccgcacacgctcaccatcgacctttccgggctgcccggcctgcccggtctcggcacgctcgcgctcagcaaggcgcaactgttgcatgaggacgatccgtaccgcaccaacaccgccgaagcgcccgaagccgtcacgccgcaaccgctcgacattgcaatgaacgccaccggcacctgcacggcaacgcttcccgccatctcctggatcagcgtggaattccacggctaa

SEQ ID NO: 90 - DNA, 1878 bp, Bacteroides sp.
  source: /note="GH43.4"
ctggcagcgtgcagcgacgacgatgaaaactccgcatcaggagctttaagcatcacaacgccggcatatacgaatgtggggtataacaaagcaaccttatccgccaatatcagcggaacggaaggagtgaatatcgtcaaacggggattctgctacgccacggcatcccatccggacatttatgacacgacctccgaagtcagaggatcggaaatcagtacgaccctgaccggcctgactccacaaacgacgtattacgtaagagcctttgtcaccctttacaacgaagagcccagatactcggaggaaacttctttcacgactccagccgagacactgagcgatgaactggcagcgtacgaaccacccacgtatgtagacgactacaccagtttctcagcctggagcaaccgttatgactggaaccttgccaacgtacacgaccctacggtaatgaaagccgatgacggatattactatatgtatcagacagacgcttcttacggcaacgcgcacagcggaaacggacacttccacgcacggcgctccaaagacctcgtaaactgggagtatctgggagcaaccatgagtgaaacgcccccgacatggatcaaagaaaagctgaatgcctaccgtcaggagatgggactggaaccgattgacaatccgtcttacggatactgggcacctgttgcacgaaaagtatcgaacggaaaataccgtatgtattattccatcgtaatcacgaactacatccaaaccggaaaaccggaaattgagaacaacggcaactttgacggttcatggaccgaacgcgcgtttatcggactgatggaaacttccgatccggcaagtaatatatgggaagacaaaggattcgttgtctgctctgccagcgataagggaaagacggattatgggcgcagcagcatcaatgactgggaagggtattttaaaatcaatgcgatcgaccctacttatataataacggaaaatggcgaacactggctgatctatggttcatggcacagcggtatcgctgccctacaggtaaatccggaagacggcaagccgctgaatgctttgggaaatccctgggacatcacaggagaagacaattcgggttatggaaagataatcgccacacgtggcaccagccgctggcaggcatccgaaggtcccgaagtgatctatcgtgacggttattactatctgttcctggcttacggttcactgtcggtagaatataatacacgtgtctgccgttccagaaacatcgacggcccttatgtagacatacacggaaattccgctatgggaagcgcgcaactatatccgatactgactgctccttaccggttcgacaacagctacggctgggtaggaatttcccattgcggcatcttcgatgacggagccggcaactggttctatacttcacaaggacgtttccccgtgaacgtaggcggcaatgaatactccaacgccatcatgatgggacatgtacgcagcatccgctgggatgccaacggctggcctctcgttatgcccgaacgttacggagccgttccgcaagcgcctatcacggaaaatgaaatagccggagactgggaacatctggcattgaccaccagtacgggcacccaacgaacgtccgaaacgatgacttatgatctcggtacgcataagataacttccggcagctggaaaaatgctacatggacatttgatgcagcgactcaaaccatcacgacaagcgccggagtagtactctatctgcaacgtgaagtcgactgggaagccagtccgcggacacatacgattgtgtatgcggcccagggtaatcaaaagacatattgggggaagaaactccaataa

SEQ ID NO: 91 - DNA, 1477 bp, Bacteroides sp.
  source: /note="GH51.0-3"
atgaaagcaaaactattagtcagcacggcttttctggcagcatctgtatctctttctgcacaaaagagtgctaccataaccgtacatgccgaccaaggcaaagaaatcataccgaaggaaatttacggccagtttgccgaacacctgggttcatgtatctacggcggtctttgggtaggcgaaaactcgaatattcctaatatcaagggatatcgcacagacgtattcaatgcactgaaagacttgtccgttcccgttcttcgctggccgggcggatgctttgccgatgaataccactggatggacggcattggtccgaaagagaaccgtccgaagatggtgaacaacaactggggcggaaccattgaagacaacagtttcggaacccacgagtttttgaatctttgcgagatgctgggttgcgaaccatacgtgagtggaaatgtaggtagcggcacagtggaagagcttgccaaatgggtggaatatatgacttctgacggagactcgcctatggccaaccttcgccgtaagaatggtcgcgacaaagcatggaaattgaaatatctcggcgtaggaaatgaaagctgggggtgcggtggcagcatgcgtccggaatattacgcagacttatatcgtcgttattctacttattgccgtaattatgacggcaaccgtctgttcaagattgccagtggcgcaagtgactatgattacaaatggacagatgtattgatgaatcgcgtaggacaccggatggacggtctttctctgcactattataccgtaaccggatggagtggcagcaaaggatcagccactcaattcaacaaggatgattattactggacgatgggcaaatgtctggaagtggaagatgtactcaagaaacattgtaccatcatggacaaatatgacaaggacaagaaaatcgccctcttactggacgaatggggaacctggtgggatgaagaaccgggaaccatcaaaggacatctgtatcagcagaacacacttcgtgatgctttcgtggcttctttaagtcttgatgtattccataaatatacagaccgcctgaagatggcaaatatcgcacaaattgtcaacgtacttcaatcgatgattctgacgaaagacaaagaaatggtattgacgcctacttattatgtcttcaagatgtataaagtacaccaggatgccacttatcttcctatcgacctgacctgcgaaaagataagtgtacgtgataatcgcactgtaccgatggtgagcgccacagcttccaaaaataaagatggggtgatccatatttctctttccaatgtagatgctgatgaagtgcaggaaatcaccatcaatctgggtgatacgaaagccaagaaagctattggagagattctgaccgcttctaaactgaccgattacaattcttttgaaaaacctaatattgtaaaaccggcacctttcaaagaggtaa

SEQ ID NO: 92 - DNA, 2058 bp, Klebsiella sp.
  source: /note="GH42.0-1"
atgaataaatttgcacctttacatccgaaggttagtacgctgctgcatggcgcggattataatccggagcaatgggagaatgaccccgatattattgataaagacattgccatgatgcagcaggcaaaatgcaatgtgatgtcggtgggaatatttagctgggcgaaactggagccacgcgaaggggtatttaatttcgcctggctggatattatcctcgataaactgtatgccgccggcattcatgtctttctggccacgccgagcggcgcgcgtccggcgtggatgtcgcagcgctatccgcaggttctgcgggtggggcgcgatcgggtgccggccctgcacggcggccgtcacaaccactgtatgtcgtcaccggtctatcgcgagaaaaccctgcaaatcaataccctgctggcagaacgttattcctcacacccggcggtgctgggctggcatatttccaacgaatatggcggtgaatgccattgcgatctctgccagaaccgttttcgcgactggctgaaggcgcgttaccagaccctggagaacctcaaccaggcctggtggagcaccttctggagtcatacctataccgactggtcgcagattgaatcgcctgcgccgcagggcgagatgtcgatccacggtcttaatcttgactggcatcgctttaacaccgctcaggtgaccgatttctgccgccatgaaattgctccgctgaaggcggcgaatgcctccctgccggtgactaccaactttatggagtatttctacgattacgactactggcagctggcggaggcgctggatttcatctcctgggacagctatccgatgtggcaccgcgataaagacgaaaccgcgctggcctgctacaccgcgatgtatcacgacatgatgcgcagcctgaagggcggcaaaccgtttgtgctgatggagtccaccccgggcgccaccaactggcagccgaccagcaaactgaagaagccgggaatgcatattctttcctcgctgcaggcggtggcgcatggcgccgactcggtgcagtatttccagtggcggaaaagccgtggttcggttgagaaatttcacggcgcagtggtcgaccacgtcggacatattgatacccgcattggccgcgaagtctgccagctcggcgagatcctcagcaagctgccggaggtgaggggctgtcgcaccgaggcgaaagtagcgattatcttcgaccagcagaaccgctgggcgctggatgacgcccaggggccgcgcaatcttgggatggaatatgagaagacggtcaacgagcactaccgcccgttctgggagcagggcatcgccgtcgatgtgattgatgccgatgtcgatttaacgccgtatcagttagtgattgccccgatgttatatatggtgcgcgacggctttgccggtcgggcggaggcgtttgtcgccaacggcggccacctggtgaccacctactggaccggtatcgtcaatgagtccgatctctgctatctcggcggcttcccgggcccgctgcgcaatctgctggggatctgggcggaagagatcgactgcctgaatgacggcgagtttaatctggtgcaggggcttgccgggaatcagtgcggtctgcagggcccttatcaggtgcgccatctctgcgaactgatccatatcgagagcgcccaggcgctggccacctaccgggatgatttttatgccggacggccggctgtgacggtgaacgcgttcgggaaaggcaaagcctggcatgtggcctcccgcaacgatttagccttccagcgcgatttctttaccgccctgagcaaggagctggccctgccgcgggcgatagcgacggagttaccacccggcgtggtggcgactgcgcgcaccgacggtgacaacgcatttatcttcctgcagaactacagcgcgcaaaaccataccctgaccctgccgcaagggtattgggattgcctgaccgacgcggcggtatcggctccactgaccctgtcggcatgggattgccgtattctccgtcgtcacgcgtaa

SEQ ID NO: 93 - DNA, 2058 bp, Klebsiella sp.
  source: /note="GH42.0-5"
atgaataaatttgcacctttacatccgaaggttagtacgctgctgcatggcgcagattataatccggagcaatgggagaatgaccccgatattattgataaagacattgccatgatgcagcaggcaaaatgcaatgtgatgtcggtgggaatatttagctgggcgaaactggagccacgcgaaggggtatttaatttcgcctggctggatattatcctcgataaactgtatgccgccggcattcatgtctttctggccacgccgagcggcgcgcgcccggcgtggatgtcgcagcgctatccgcaggttctgcgggtggggcgcgatcgggtgccggccctgcacggcggccgtcacaaccactgtatgtcgtcaccggtctatcgcgagaaaaccctgcaaatcaataccctgctggcagaacgttattcctcacacccggcggtgctgggctggcatatttccaacgaatatggcggtgaatgccattgcgatctctgccagaaccgttttcgcgactggctaaaggcgcgttaccagaccctggagaacctcaaccaggcctggtggagcaccttctggagtcatacctatactgactggtcgcagattgaatcgcctgcgccgcagggcgagatgtcgatccacggtcttaatcttgactggcatcgctttaacaccgctcaggtgaccgatttctgccgccatgaaattgctccgctgaaggcggcgaatgcctccctgccggtgactaccaactttatggagtatttctacgattacgactactggcagctggcggaggcgctggatttcatctcctgggacagctatccgatgtggcaccgcgataaagacgaaaccgcgctggcctgttacaccgcgatgtatcatgacatgatgcgcagcctaaagggcggcaaaccgtttgtgctgatggagtccaccccgggcgccaccaactggcagccgaccagcaaactgaagaagccgggaatgcatattctttcctcgctacaggcggtggcgcatggcgccgactcggtgcagtatttccagtggcggaaaagccgcggttcggttgagaaatttcacggcgcagtggtcgaccacgtcggacatattgatacccgcattggccgcgaagtctgccagctcggcgagatcctcagcaagctgccggaggtgagaggctgccgcaccgaggcgaaagtagcgattatcttcgaccagcagaaccgctgggcgctggatgacgcccaggggccgcgcaatcttgggatggaatatgagaagacggtcaacgagcactaccgcccgttctgggagcaaggcatcgccgtcgatgtgattgacgccgatgtcgatttaacgccgtatcagttagtgattgccccgatgttatatatggtgcgcgacggctttgccggtcgggcggaggcgtttgtcgccaacggcggccacctggtgaccacctactggaccggtatcgtcaatgagtccgatctctgctatctcggcggcttcccgggcccgctgcgcaatctgctggggatctgggcggaagagatcgactgcctgaatgacggcgagtttaatctggtgcaggggcttgccgggaatcagtgcggtctgcagggcccttatcaggtgcgccatctctgcgaactgatccatatcgagagcgcccaggcgctggccacctaccgggatgatttttatgccggacggccggctgtgacggtgaacgcgttcgggaaaggcaaagcctggcatgtggcctcccgcaacgatttagccttccagcgcgatttctttaccgccctgagcaaggagctggccctgccgcgggcgatagcgacggagttaccacccggcgtggtggcgactgcgcgcaccgacggtgacaacgcatttatcttcctgcagaactacagcgcgcaaaaccataccctgaccctgccgcaagggtatcgggattgcctgaccgacgcggcggtatcggctccactgaccctgacggcatgggattgccgtattctccgtcgtcacgcgtaa

SEQ ID NO: 94 - DNA, 3876 bp, Bifidobacterium sp.
  source: /note="GH2.0-2"
atgttcattccccggtactacgagagtctcggccatctacatgtcggcacgcagccgaaccgcgcgtattacgtgcccgcgtccacgccgatggacacggtcggcgagaatcgcgtgaattccgaccgtttcatgctgctgaacggcgactgggatttcaagtattatgcgagcatctacgacttggacgccgaggtctcccgactgcgcgccgccggccgcccggtgttctatgacgtggatttcggcggggatgacgcaccggagaacgccgatccgcgcactgccgccacgggtgcgctggcggcggacggcttcacgacgacgccggtgccgagcgtgtggcagaaccatggtttcgaccgccaccagtacacgaatttcgactatccgttcccgttcgacccgccgttcgtgccgcaggacaacccgtgcggcgtgtacctgtgcgatttcatgcatacgtccgatcctgacgcaccctgcacgtacctgaatttcgagggcgtggattcggcgttctatgcgtgggtgaacggcgagttcgtcgggtattcgcaggtgtcgcattcgaccagcgagttcgatgtgaccgacgtgctggaggacggcgtgaacacgctggccgtgctggtgctgaagtggtgcgacggcagctatcaggaggatcaggacaagttccgcatgagcggcatcttccgtgacgtgtatctgctggaccgtcccgagtatgcgattcgtgacatgttcgtgcatacgtcgatttggcgcaatgtcgattccgcgctggttgaggccggcatcagcgatgacgaatatgatgcgtcgccggtcgatcacgcgacggtcgacgtggatttcgcgttcttcgacgatgcggatgtgccggtcaaggtgcagctgttcgatgaggatggcgagctggtggcagagacggcctcggagccgatcgatgatccgatggccggggacgaggacgacgtgacggttcggacacagcccgacgcgagcgaagccgacgacgcgaccggcactggcagcgacgacaccgccgcggacgacgaagaagaaggcgtcatcgagtcgaccgacgacgtggccgccatcgacgatgactccacggacgcacaggccgcactgcgcatcgcgtcggtgaccggcacgctcgccggcggcgcgaacggcaccggattcaccggagacagcgcgttcgccccgaccgcgcacgcatccctggcggtcgacgacccgcatctgtggaccgccgagacgccgtacctgtacaccatcgtgtacaccaccgcgaacgaggtcatcaccgcgctcgtcggcatccgcgaggtcagcgtggatggcaatgtggtcaaggtcaacggcaagccgatcaagctccacggcgtcaaccggcacgacagcgacccggtgaccggcccggtcatcagcgaggagcagctcatgcgcgacctcacgctgatgaaggagcacaacgtcaacgcgatccgcaccagccattacccgaacgcgccgcacttctacgacctgtacgaccgtctcggcttctacgtggtggccgaggctgacaacgagagccacggcgcgatgcgcggcgtgcatccggacgagagcgacgcggctgtcaacaagcgctggaaccggcctatcgccgacaaccccgcgtggatcgcgccgaccgttgaccgcgcgcagcgcagcgtggagcgcgacaagaaccatgcgagcatcatcttctggtcgatgggcaacgagtgtgcgtacggctgtacgttcgaggcggcgctgctgtggacgcagaccttcgatccgagccgcctgacgcactatgagagcgcccggtatgtggatgagggacaggagtgcgattacagctatcttgacgtacacagccgcatgtacccgtccgtcgaggagatcgaccagtacttctccgaggaggggccgcgcacgccggacgggctgcgcgacggcagcaacggcgatgacggcgacaacggcgtcaagccgtacgtgctgtgcgaattctgccatgcgatgggcaacggcccgggcgatctggaggattatttcacgcgcatccagcgttatgacggcctggccggcggcttcatctgggagtggtgcgaccatgcgatcgaccgtggcacgaacgcggccggcaagcgcgagtacgcgtacggcggcgattcgggcgagtacccgcatttcggcaatttctgcatggacggcttggtgtacccggaccgcacgccgcataccgggctgctggagttcaagaacgtgtatcggccggtgcgcgtgaccggtttcgacgcggccgcgggcacggtgacgctgcacaattacctggacttcctggatgccgccgacgcggtgttcatgacgttcgagctgctggtggatggcgtggagaccgcatgggctgcgtgggagagcgaccctgcggcgggcgcggcgttccgggaggagcatcccggcaattacacgccgtcgatgccatcgatcgcgccgcatggtgacgcggtcgtcgacataccggctgagatccttgatgccatacccgaggccgggaacgtgacgatgctggtgaagtactatcaggcgactgacaccgagacactgccgatcggcttcgagctcggcttcgacgaggtcgccgtgccgaccgcggatccgcgcaatcagacggtcgtcgccgcgctggccgatatcgccgatggcatcggctcggatgacgatgtcgacgacgttgccgatgacggcaccgatagcgtagaaggcgccgacgatggggcgaacgatgccgcggatgccggctacgacgacgtgctggcagacccgctgaccgtcatgcagaccgatgcctcgatcaccgtggaaggctcgacgttccggtatgtgctcgaccgccgtaccggcctgttctcgtcgatgtcgttcgcgaaccggtcgctgcttaacaggccgatggagctgaacgtgtggcgcgctcccaccgacaacgaccagtacatcaaggccgattggatccgcgcccagtatgaccgcgctcaggcgcgcgcgtacgaggtcggtgtactggtcgatgaggatgacgtcatcgccaagcccgagtcgattgagctgcgtgcggacgatgaggatgcgccggtcgcctcgtttggagacgatgcgatcctcgacgacggcaacgtcgacgccggcgacgtgagcgccatagcgacgtccgaggacggctcggtggtggtcgacggccaggtgacgatccatgcgacgatggcgctggtggcgccgattgtgcagcgcatcgccgacatcgacgccgactggaccatcgcgcccgacggttcggtggcgctgcgcatgcatgtgatgcgcgacaccgatttcccgttcctgccgcgtttcggcctgcgcctgttcgtgccgaagccgatgcggcagatcgcctattgcggtctcggcccgaacgaaagctacatcgacaagcgccggtccagctatcatggcgtgttctccggcactcccgaatcgctgttcgagccgtatatcaagccgcaggagaacggcaaccatcacgactgcgattgggcgagcgtcgccagcgatgacaccgagctgctggtgctccgtgccggtgaccacgccttcgacttccaggcgctgccttacacccaggaggagctgaccgccaaggctcacaacagcgagctgaagccggcggattcgacggtggtgtgcgtggattacatgcagtccggcgtcgggtccaacagctgcggtcccaagctgcacgagaaataccgcctcgacgacgcggagttcgatttcgatctcgtcctgcgcccgcaggcgctctga

SEQ ID NO: 95 - DNA, 1701 bp, Bifidobacterium sp.
  source: /note="GH51.0-2"
atgaccactcacaacagccagtattccgccgaaaccacccatcccgacaagcaggaaagcagcccggcgccgaccgccgccggcaccacggccagtaacgtctccacaaccggcaacgcaaccacgccggacgccagcatcgccctcaacgccgacgccactccggtagccgacgttcccccgcgtctgttcggctcattcgtagaacatctgggccgctgcgtctacggcggcatctacgagcccagccatcccaccgccgacgaaaacggcttccgccaagacgtgcttgacctggtcaaggagctgggcgtcacctgcgtgcgctaccccggcggcaatttcgtatccaactacaactgggaagacggcatcggtccacgcgagaatcgccccgtgcgccgcgacctggcctggcattgcaccgaaaccaacgagatgggcatcgacgacttctaccgctggagccagaaagccggcaccgaaatcatgcttgccgtcaacatgggcacccgggggctgaaagccgcgctcgacgagctcgagtatgtcaacggcgcgcccggcaccgcttgggcggatcagcgcgtggccaacggcatcgaggagccgatggatatcaagatgtggtgcatcggcaacgaaatggacggcccgtggcaggtgggccacatgagcccggaagaatatgccggcgcggtggataaggtggcccacgccatgaagctcgccgagtccggtctcgaactcgtggcctgcggttcctcgggtgcctatatgccgaccttcggcacgtgggagaagaccgtgctcaccaaggcttacgagaatctcgacttcgtctcctgccatgcctactacttcgaccgcggccataaaacccggaccgccgcctccatgcaggacttcctggcctcttccgaagacatgaccaagttcatcgccaccgtctcggacgcggccgatcaggcgcgagaagccaacaacggcaccaaagacatcgccctgtccttcgacgaatggggcgtatggtattcggacaagtggaacgagcaggaagaccagtggaaggcggaggccgcgcagggtttgcaccacgagccatggcctaagtctccgcatttgctggaagacatctacaccgcggccgacgcggtggtcgaaggttccctgatgatcaccctgctcaagcactgcgatcgcgtgcgttccgcctcgcgcgcccagctggtcaacgtcatcgcccccatcatggccgaggaacacggcccggcatggcggcagaccacgttctacccgttcgccgaagccgcccttcacgcgcgcggccaggcctacgctccggccatcagctcccccaccatccataccgaggcatatggcgacgtgccggccatcgacgcggtagtcacgtgggatgaacaggcccgcaccggtctgctgcttgccgtcaaccgtgacgccaacaccccgcacacgctcaccatcgacctttccgggctgcccggcctgcccggtctcggcacgctcgcgctcagcaaggcgcaactgttgcatgaggacgatccgtaccgcaccaacaccgccgaagcgcccgaagccgtcacgccgcaaccgctcgacattgcaatgaacgccaccggcacctgcacggcaacgcttcccgccatctcctggatcagcgtggaattccacggctaa

SEQ ID NO: 96 - DNA, 1140 bp, Bifidobacterium sp.
  source: /note="GH8.0-2"
atgacaaatgcaaccgataccaacaagacattgggcgagtccatgttcgcacagtgcggatatgcccaggacgccatcgataagcgcgtgtcacaggtctggtatgaaattttcgaaggcccgaacaaattctattgggagaacgacgaaggccttgcctatgtgatggacaccggcaacaacgatgtacgtaccgagggtatgagctatgcgatgatgatcgccctgcaatacgaccgtaaggacgtattcgacaagctgtggggctgggtaatgcgtcacatgtacatgaaggacggtcatcatgcgcattatttcgcatggtcggtcgcgccggacggtacgccgaactcgaatggtcctgcacctgacggcgaggaatatttcgcgatggacctgttcctcgcctcccgtcgctggggtgatggcgaggatatctacgaatattccgcatggggacgcgagatcttgagatattgcgtccataagggcgaacgctacgacggcgagcccatgtggaatcccgacaacaagctcatcaagttcattccggaaaccgagtggagcgatccgtcctaccatctgccgcacttctatgaagtattcgccgaagaagccgacgaagaagaccgtccattttggcatgaggcagcagccgcaagccgtcgctatctgcaggcggcctgcgacgagcggaccggcatgaacgctgaatacgcggattatgacggaaagccgcatgtcgacgagtccaatcattggcatttctattccgacgcctaccgtaccgcggcgaatatcggactggacgcagcctggaacggtccgcaggaagtgctgtgcgaccgcgtcgccgcgctgcagcgattcttcctgacccacgaccgtactagcgtctacgccatcgacggcaccgccgtggacgaggtcgtgcttcatccggtcggattcctggccgcgaccgcgcaaggctcacttgcggcggtgcattcggcccagcccgacgcggagcataatgcccgtgaatgggtgcgcatgctgtggaatacgccgatgcgaaccggcacgcgtcgttactatgacaatttcctctatgctttcgccatgctggcgttgagcggaaagtatcggtatgaatga

SEQ ID NO: 97 - DNA, 1701 bp, Bifidobacterium sp.
  source: /note="GH51.0-7"
atgaccactcacaacagccagtattccgccgaaaccacccatcccgacaagcaggaaagcagcccggtgccgaccgccgccggcaccacggccagtaacgtctccacaactggcaacgcaaccacgccggacgccagcatcgccctcaacgccgacgccactccggtagccgacgttcccccgcgtctgttcggctcattcgtagaacatctgggccgctgcgtctacggcggcatctacgagcccagccatcccaccgccgacgaaaacggcttccgccaagacgtgcttgacctggtcaaggagctgggcgtcacctgcgtgcgctaccccggcggcaatttcgtatccaactacaactgggaagacggcatcggtccacgcgagaatcgccccatgcgccgcgacctggcctggcattgcaccgaaaccaacgagatgggcatcgacgacttctaccgctggagccagaaagccggcaccgaaatcatgcttgccgtcaacatgggcacccgggggctgaaagccgcgctcgacgagctcgagtatgtcaacggcgcgcccggcaccgcttgggcggatcagcgcgtggccaacggcatcgaggagccgatggatatcaagatgtggtgcatcggcaacgaaatggacggcccgtggcaggtgggccacatgagcccggaagaatatgccggcgcggtggataaggtggcccacgccatgaagctcgccgagtccggtctcgaactcgtggcctgcggttcctcgggtgcctatatgccgaccttcggcacgtgggagaagaccgtgctcaccaaggcttacgagaatctcgacttcgtctcctgccatgcctactacttcgaccgcggccataaaacccgggccgccgcctccatgcaggacttcctggcctcttccgaagacatgaccaagttcatcgccaccgtctcggacgcggccgatcaggcgcgcgaagccaacaacggcaccaaagacatcgccctgtccttcgacgaatggggcgtatggtattcggacaagtggaacgagcaggaagaccagtggaaggcggaggccgcgcagggtttgcaccacgagccatggcccaagtctccacatttgctggaagacatctacaccgcggccgacgcggtggtcgaaggttccctgatgatcaccctgctcaagcactgcgatcgcgtgcgttccgcctcgcgcgcccagctggtcaacgtcatcgcccccatcatggccgaggaacacggcccggcatggcggcagaccacgttctacccgttcgccgaagccgcccttcacgcgcgcggccaggcctacgctccggccatcagctcccccaccatccataccgaggcatacggcgacgtgccggccatcgacgcggtagtcacgtgggatgaacaggcccgcaccggtctgctgcttgccgtcaaccgcgacgccaacaccccacacacgctcaccatcgacctttccgggctgcccggcctgcccggtctcggcacgctcgcgctcggcaaggcgcaactgttgcatgaggacgatccgtaccgcaccaacaccgccgaagcgcccgaagccgtcacgccgcaaccgctcggcattgcgatgaacgccaccggcacctgcacggcaacgcttcccgccatctcctggatcagcgtggaattccacggctaa

SEQ ID NO: 98 - DNA, 1353 bp, Citrobacter sp.
  source: /note="GH4.0-2"
atgtctgcacccaaaattacctttatcggcgccggttccacgattttcgtcaaaaatattcttggggatgtctttcaccgcgatgcgcttaaatctgcgcatatcgccttgatggatctcgatcctacgcgtctggaagaatcacacgttgttgtgcgcaagttgatggattctgcgggcgcgtctggacgaatcacctgctataccgatcaaaaagcagcattacaggatgctgattttgtagtggtcgctttccagattggcggctatgaaccttgtaccgtcaccgattttacggtgtgtaaacgccatggtctggagcagacgattgccgacacgctggggccgggcggcatcatgcgcgcgctgcgtaccatcccgcatttatggcagatttgtgaggatatgaccgaagtctgtccgcaggccacgatgcttaactacgttaacccgatggcaatgaacacctgggcaatgtatgcacgttatccgcatattaagcaggttgggttgtgtcattcggtgcaggggacggcggaggagttggcccgcgatctgaacatcgaccctgcttctttgcgctatcgcagtgccgggatcaaccatatggcgttttatctggagctggagcgcaaaacggcggacggtgcctatgtgaatctctacccggagctgctgacggcctatgaatccggtcaggcgccgaaaccaaatattcacggaaatacccgttgccagaacattgtgcgctatgaaatgttcaaaaaactggggtatttcgtcaccgaatcgtcggagcacttcgctgaatatacgccgtggtttatcaaaccggggcgtgaagatctgattgagcgctataaggtgccattggatgaatatccgaaacgttgtgtggaacagttggcgaactggaaaaaagagctggaagagtacaaaacggctgagcggatcgacattaaaccgtcgcgcgaatatgccagcactatcatgaacgctatctggaccggtgaaccgagcgtcgtgtatggcaacgttcgcaatgacaatctgatcgataacctgccgcaaggctgctgcgttgaagtcgcttgtctggtcgatgcgaatggtattcagccaacgaaagtcgggactctcccgtcacatttggcggccatgatgcaaaccaatatcaatgttcagaccctgctaacggaagccatcctgacggagaatcgcgatcgcgtttatcacgcggcgatgatggatccgcataccgccgctgtactggggattgaagagatttatgcgctggtggacgacctgatcgcgtctcacggcgactggctgccggcctggctgcaccgttaa

SEQ ID NO: 99 - DNA, 2295 bp, Bacteroides sp.
  source: /note="GH3.0-8"
atgaaacattttgtacgaagaatgcaggcgcttgccgcttctttggtcgtagtggccgccgggttacaggcacagaaggctccccgggatatggaccgctttatcgaccagttaatgaaaaagatgacgctggaggagaagatcggccagctcaacctgcccgtgaccggagagatcactaccggacaggcgaaaagcagcgatgtagccaaacgaatccgtaacggagaggtgggaggactgttcaacctgaaaggagtgaaacgcatccgtgaagtacagcggcaggcggtggaggagagccgcctcggcattcccttgttgttcggtatggacgtaatccacggatacgaaaccattttccctattcctctcggcctgtcgtgtacctgggatatgaaagccatcgaagagtccgcccgtatagctgccgtcgaagccagtgccgacggtatctcgtggacattcagcccgatggtggacgtcagtcgtgatccccgttgggggcgcgtgtcggagggaaacggtgaagacccgttcctcggcgcagccatcgcccgtgccatgatacgcggataccagggaaaggatatgagccggaatgacgagataatggcttgtgtgaagcatttcgccctttatggagcatcagaggcggggcgcgattataatacggtggatatgagccgccagcgtatgttcaatgaatacatgctgccctaccaggccgcagtcgaggcaggtgtcggcagcgtaatggcttcgttcaatgaagtggacggtgtgcctgccaccggaagcaagtggctgatgaccgatgtgctgcgcaagcagtggggcttcgacgggtttgtggtaacggactataccggtatcaacgagatgatagaccacggcatgggtgaccagcagactgttgccgccctcgccctgaatgccggggtggatatggatatggtgagcgatgccttcagcggcactctgaagaagtcggtggaggaaggcaaagtatccgcagctgccatcgacgccgcctgccgccgtattttggaagcgaagtataagttgggactgtttgacaatccttataagtattgcgacgtgaatcgtcccaagaagcagatcttcaccaaggaacaccgtgccattgcccgtaagactgcttcggagagctttgtgctgctgaagaatgaaggtgtgttgccactcagcaagaaaggaaccattgccgtagtcggtccgttggcgaacacccgttccaacatgccgggcacctggagcgtagctgctgtgctggataacgctccctcgctggtcgaaggactcagggaagtagtcggtgaccgggcaaaagtggtaaccgccaagggaagcaatctgattggcgatgccgactatgagaagcgcgccaccatgttcggacgtgaactgcaccgggataaccgtacggatcgcgaacttctggacgaagctctgaaagtagctgccggggccgatgtcattgttgccgcactgggcgagtcgtccgaaatgagtggagaaagcagttcgcgtaccaacctggagatgccggatgtacagagagcgctgttgcaggaattactcaaaaccggaaagcccgttgtgcttgtgctttttaccggtcgcccgctggtgctcacctgggaagaagaacacgtgcctgccatcctcaacgtatggttcggagggagtgaagccgcttatgccatcagcgatgtgcttttcggcgatgtcaatcccagtggaaagctgaccgctacttttccgcaaaatgtaggccagattccattgttctacaatcataaaaacaccgggcgtccgttgcaagagggacgttggtttgagaagttccgcagcaattacctcgacgtgagcaacgagccgctctacccgttcggctacggattgtcttatacgacttttgcctacagtgatattcacctgagcagcacggagatgagtgctgatggcgaactgacggcgactgttaccgtcaccaataccggcagccgtgacggagcggaggtggttcagctttacatccgcgacctggtgggcagcgtcactcgtccggtgaaagaactgaaaggttttgagaagattttcctcaaggccggagagtctcgtaaagtaagcttcagcatcacgccggaattgttgaagttctataattacgatttgcagtttgtctgcgaaccgggtgatttcgatgtaatgattggcggaaacagccgggatgtaaaaaaggcacgatttcttctgaagggagaataa

SEQ ID NO: 100 - DNA, 2154 bp, Bacteroides sp.
  source: /note="GH31.0-12"
atgaaatatatttgtatcaaaactgtagcaatttacttgctcgcaaccttacctttattggcgaacgcctcaacacacaaggtaaaaattacacatagcgtcatggttgggaacggaatcgcaaaattcatcccggaaggcttcgacgctcaaaagataccttcttttgcaatagaaaaagaaccacgcgaacaaggaacacttcctgccgactgggtacttgttcccgagttctcactcacggatggtaaagcaaacgcatcattaacagtgccggaaggtacaagcatctatggcggtggtgaagtgaccggttcacttctgagaaatggaaagaccatcaaattatggaatacagactcaggagcttatggtgtagacaaaggtactcgtctgtatcaatcacatccttggatgatgggagtgcgaaaggacggaacagcttttggaattttattcgatactacttggaaagcagaactaagcagtacagacgaaaaaatcgaattaaaaagtgaaggaataccctttcgggtattcatcattgacagggaatctccacaagcagtcattcgcggactatccgaactgaccggcacaatgccaatgattcctcgctgggcactaggttatcagcaatgccggttctcatattctcccgacagccgtgtcattgaaatagcagatactttcagactaaaaagaataccatgtgatgttatctggatggacattgattatatggacggataccgcatctttacctttaatccgaaaagttttccgaatcctaaagcggtgaaccgtgatttgcacatacgtggattccattctgcatggatgattgacccgggagcaaaagttgaccctaactatttcgtatataaatcgggaacagaaaatgacgtttgggtgaaaacagcagacggtaagaacttccacggtgatgcatggccgggagcagcagcattccctgattttacttctcctaaagtaaacaaatggtggagaaacttatataaagattttctagcacaaggagtagatggcgtatggaatgatgttaacgaaccccagatcaatgatacgcccaacaaaacaatgccggaagacaacctgcatcgtggaggaggaaagcttccggcaggtacacatcttcagtatcataatgtatatggcttcctgatggttaaagcatccagggaaggtatactggatgctcgtccagaaaaacgtcctttcattctgacacgttccaacttccttgggggacaacgttatgccgctacatggactggcgacaacggttcttgctgggatcatctaaaaatgtcagttcccatgtcattaacattgggattatccggtcaaccgtttagtggtgcagatataggcggtttcttattcaatgctgatgctgacttattcggcaactggattggtttcggtgccttttatcctttcgcacgtggtcatgcttgcgccggaacaaacaacaaggaaccatgggtatttggacaaaaagtagaagatgcctcacgcatcgctttggaacgtagatatatactactaccctacttttatacactcttacacgaagcctcaactaatggcatgcctatcatgcgtcctgtcttcttctccgaccctaaagacttgtcactgagagcagaggaagaagctttccttgtcggtgataatttacttatcattccagcatttgctaatcaaccggcacttccgaaagggatctggaaagaactgtcacttgtagaaggagatcagaatgataaatatcaggcaaaaatgaagattcgtgggggagctatcattccgactggaaaaataattcagaacactacagaaaattcattagatcctctgacattactagtgtgtctggacgaacagggcaaagcttccggaaatatgtattgggatgcgggagatggttggtcttacaaaaaaggggactatagcctgctacaatttgtcgcagagcgaaatggtgataaagtgactgtaaagctaacaaagaaaaccggaaaatacaacactgagaataaagacatggcagtgattaaaattataacagatcaaggcatacgtcaagccagtggaaatctagtggaaggcattgaaataagactataa

SEQ ID NO: 101 - DNA, 972 bp, Bacteroides sp.
  source: /note="GH43.19-2"
atgaatatgaaaaagtatactttactcctggcattccttttagtaggagtgctgacaggatacagccagcaatctgcctacctgtttgtctatttcaccggaaacaggatgagtgaggaagccatccggatggctgtcagccccgatggatacaactactatgcattaaacggaaaccaaccggtcatcgattcccgtgaaatcagttctacgggtggagtgcgtgacccgcacattcttcgttgtgaagacggaaagacattttacatggtcgtaaccgacatggtctccggcaacggatggagttccaaccgtgccatggtactgttgaaatcgaaagatctcgtcaactggacctccaacatcgtgaatatccagaagaaatacccgaatcaggaagatttgaagcgggtatgggcaccgcaaactatttatgataaagaagcgaagaaatacatggtctactggtcaatgcagcatggtaatggcccggacattatttattacgcatacgctaacaaagatttcaccgatatagaaggagaacccaaaactttgttcctcccgaagaatggcaaatcctgtattgacggagacatcatttataaagacggactttaccacctgttctataaaacggaaggagacggcaatggaattaaaaaagcaaccaccgcctccctgacttccggacaatggacagaatcggaagattataagcaacagacgaaagaagctgtagaaggtgccggcatcttcccgctgataggtacggacaagtacatcctgatgtacgatgtatatatgaaaggcaagtatcagtttacggaaagcaccgatttggagaatttcaaagtcatagacaatgccattagcatggacttccatccgcgccacggcactgtaatgccaattactgacaaggaactgaaacgcttgtacaaggcctacggcaagcccgacaagatgtaa

SEQ ID NO: 102 - DNA, 1545 bp, Bacteroides sp.
  source: /note="GH43.10-2"
atgaatacaagaatcctttgcgtatggatagcgcttctgacttgtcagatagcgggtgcacaaacaaagaatgtgacatggggagatcagggaaacggcacgtatatcaatccgatattgaatgcggactattccgatccggatgtcatcagggtaggcgataagtattatatggtaaactcggactttcattatatgggcatgccggtgctggaatccgatgatatgattaactggaagattatcagtcaggtgtaccgacgcctggactttccggactgggatacgaacggaaattatggaggaggctcatgggccccctctatccgtcatcatgacgggaagttctggatttacttctgtactccccgtgaagggctgatgatgagtacggctaccgatcctcacggcccttggtcacctttgcattgtgtgaaacggattggcggatgggaagacccttgcccgatatgggatgacaatggtcaggcttatctgggacggagccagttgggagccggacctatcatcttgcataagatgagcgccgacgggaggaccttggaagatgacggacacgtgatctataccggtccggtggcagaaggtaccaagtttcacaagcgggacggatattactatatcagtattcccgaaggcggagtaggtgagggatggcagacaattctgcgttcgaaaaacatctacggtccttacgagaagaaagtggtactggaaaaaggttctaccaatgtcaacggacctcatcaaggtgcactggtagatactcccgaaggtgagtggtggttctatcacttccagttgacggaaccgctgggaagagtcgtgcatctgcaacctgcacattggaaagacggatggcccgtgattggggtggacatcgatatgaacggcataggcgaaccggtaaaagtctggacaaaaccgaataccggaaagaaagtgcctgtaagcttcccgcagggaggcgattcctttgattcgcccgagctgaacttgcagtggcagttcaatcataatccttctgacgccgactggaatctgacggaacgaaaaggatggttactgttgaaagctctgaaagcggatcatcttcgggcatcacgcaatatgctgacacagaagtgtatcggatacgaggggacggttacgacagaaatggatatgagttcttggaccgagggacaacgtgccggactattctgtataggcaatttgttcaatggcattggaatactcaaagagaatggcaagaactatctgtatctggagaataatggtagtgtggagaaagtaaagccggtaagcggtaagaagatttatttcagagcaacgatgaatgcacgtaccaaccagcatcagttgtactatagcacggacaataagaactttactccttgtggagaagcttattcgctgagattcggtgactggaaaggtgcccgtgtcggtctgtactcatacaacacgcttcgtgacggaggaaatgctttcttcaactggttcacttacgactttaactga

SEQ ID NO: 103 - DNA, 1989 bp, Bacteroides sp.
  source: /note="GH97.0"
atgaaaaaacttacatttttattattatgtgtcttgtgtacgctttcgttgcaagctcagaagcaatttacactagcctcacctgatggaaatctgaaaacgacaataaccattggcgaccggctgacttatgacattacatgcaacggcaggcagattctgactccttctcccatatcaatgacgttggataacgggactgtctggggagaaaatgcgaaattatccggaacttccaggaagagtgtggacgagatgataccatctcctttctaccgtgccagcgaattgagaaatcattataatggactgaccttgcgtttcaaaaaagactggaatgtagagtttcgtgcatacaatgacggtatcgcctaccgttttgtgaatcaggggaagaagccttttcgtgtggtgacggaagtatctgattattgttttccatcggatatgactgcctccgtgccttatgtaaaaagcggtaaagacggtgattataactcccagttttttaattctttcgagaatacgtatacaacggacaaactgtcgaagctgaataaacagcgcttgatgttcttgccgttggtagtagatgcgggcgatggagtgaaagtctgtatcacagagtccgatctggaaaattatccgggactttatctttctgcttcggaaggcgcgaatcgtctgagcagtatgcatgctccttatccgaagcgtacggtacagggtggtcacaaccagcttcagatgttggtgaaggagcatgaagactacattgccaaagtggataagccgagaaacttcccctggcgtatagccgtggttactaccaccgataaggaccttgccgctaccaatctcagctacctgttaggtgcgccttcacgtatgtccgatatttcatggattaaaccgggaaaggttgcttgggactggtggaatgactggaatctggatggcgttgattttgtgaccggagtaaataatccgacttataaggcatatatagactttgcttctgcaaacggtatcgagtatgtgatacttgacgagggatgggcagtgaacttacaggcggatttgatgcaggttgtcaaggagattgacctgaaagaactggtagattacgcagcttccaaaaatgtaggtatcatcctttgggccggttatcatgcattcgagcgtgatatggaaaatgtgtgccgtcattatgccgaaatgggagtaaagggtttcaaagtggactttatggaccgtgacgatcaggaaatgactgcattcaactatcgtgccgctgaaatgtgtgctaaatacaagctgattcttgacctgcacggcactcataagcctgccggattgaaccgtacttatccgaatgtgttgaatttcgaaggagtcaatgggttggagcagatgaaatggagttcaccgtcagtagatcaggtgaagtatgatgtgatgattcctttcatccgtcaggtttccggtccgatggattatacgcagggggcgatgaggaatgcttccaagggtaactattatccttgttattcagaaccgatgagtcagggaacccgttgccgccaactagccttgtacgtggtgtttgaatctccttttaatatgttgtgcgatactccgagcaactatatgcgcgaaccggaatcaacggcatttatcgcagaaataccaactgtatgggatgaaagtatcgttcttgacggtaaaatgggagagtatattgtgacagcacgccggaaaggggatgtctggtatgtaggtggaattacagattggagtgcacgtgatattgaagtcgattgttctttcctgggtgataaatcttatcatgctactttgtttaaagatggtgtgaatgctcatcgggcaggtcgtgattataagtgtgagtccttcccgataaagaaggacggtaaactgaaagttcatctggcaccgggaggaggttttgcccttaagataaaataa

SEQ ID NO: 104 - DNA, 1773 bp, Bifidobacterium sp.
  source: /note="GH13.30"
atgaaaggggacaacatgaccgaagtcaacgatccgtcgctgtggtggaagcaggccgtggtctaccaggtgtatccacgttccttcaaggattcccgcggcgagggcctcggccagatcgccggcgtcaccgagaaaatcgggtatctgaaggaactgggcgtcgacgccatctggctgagcccgttctacccgtcccagctggccgacggcggctatgacgtggacgactaccgcaacgtcgatccgaaactcggcaccatggacgatttcgacgcgctcgccaaagccgcgcatgccgacggcatcaaaatcgtcgtggacatcgtgccgaaccacagctccaacctgcacgaatggttcaaggccgcgttggccgcgaaacccggctcgctggaacgcgaccgctacatcttccgcgacggcaagggaccgaacggcgacgagccgccgaccaactggcagaaccacttcggcggccctgcatggacgcgcgtgcccgacggccaatggtatctgcacatgttcaccaaggaacagccggactggaactggaaaaacgaggacgtgcgcgccgatttcatcaaaaccctgcgtttctggcttgaccacggtgccgacggcttccgcgtggacgtggcgcacggcctggccaaggatctcgaccgcgatgatctggacgattatgtggtctggtgcaccaacgatcagcccgaagacggctcccatccggtgatcgaccgcgacgaagtgcacgacatctaccacgagtggcgcaaggtgttcaacgagtacgatccgccggcgttcgccgtggctgaggcgtgggtccgaccaagccgccagcatctgtacgcctccccggacgatctcggccagatcttcaacttcgagttcgccaagaaggattggatccgcgacgacatgcacctcgccatcgaggaaggtctggaaagcgccgaacggtccggttccaccgccacttgggtgatgagcaaccatgacgtggtccgccatgccacccgctacgcgctgccccaggtgccgaccggcgaataccatcgactgccgctcgactggctgctgcgcgacggcaccacataccgggaggaccgcgcgctcggcaccaagcgcgcccgcgccgcgatcatgatggagatggcgctgcccggctccgcctacgtgtatcaaggcgaggaactcggcctgttcgaagtggccgacattccgtgggatgagctggaggatccgtccgcatggcgcacctcccgttccgccagcaccaaaggccgtgacggctgccgtgtgccgctgccgtgggttgcggccgacgctccgcagctggacgatccgaacgatgagttcggccatggcggctccttcggattctcgccggcagacgcgaaggccgagccgcatctgccgcaacccaagtggtacaaggatttcgcggtcgatgtcgaatcggccgacccggattccatgctgaacctgtaccgccgcgtgctggcattgcgacatgagttgcagaccaccgacctgagtctcgaatggcttccggaagaccagcccggcaaggcgcatgacggcgccaacggtttcccgggtggcaccatcgcgtaccgccgtgccaacggctgggcctcgatcaccaacttcggcgaagaaccgatcacgttgccgcaaggcgaagtgctgctgacatcaggaccgcttaccgacgatggcaagctgccgcaagataccagcgcttggctcaaactggccgattga

SEQ ID NO: 105 - DNA, 3072 bp, Bifidobacterium sp.
  source: /note="GH2.0-3"
atgacagacatcacacatgtcgatcgcgcatcgcaggcttggctgaccgacccgacggtgttcgaggtgaaccggactccggcccattccagccacaagtggtacgcccgcgacccccagagcggacaatggtccgatctcaagcagagccttgacggcgagtggcgggtcgaggtcgttcaggccgccgacatcaacctcgaagaggaacccgcgacggccgagtcgttcgacgactcctcgttcgagcgtatccaggttccgggccacctgcagacggccggtctgatgaaccacaagtacgtgaacgtccagtatccgtgggacggccacgagaacccgttggaaccgaacatcccggagaacaatcacgtcgcgctctaccgcaggaagttcaccgtctccgcccccgtggcaaacgccaagcaggccggcggatcggtgtcgatcgtgttccacggcatggccacggcgatctacgtgtgggtcaacggcgcgttcgtcggctatggcgaggacggcttcacgcccaatgagttcgacatcaccgaactgctgcacgacggggagaacgtcgtggccgtcgcctgctacgaatactccagcgcctcctggcttgaggatcaggacttctggcgtctgcacggcctgttccgctccgtcgaactcgccgcccgcccgcatgtgcacatcgagaacacgcagatcgaagccgattgggatcccgaggccggcaccgcctccctcgatgccgcgctgaccgtgctcaacgcggccgacgcggccacggtccgcgcgaccctgaaggacgccgacggcaacacggtgtggcagacgacgggcgacgcggaggcgcagaccgcgatctccagcgggccgctgcagggcatcgccccttggagcgccgaaagcccgacgctgtacgagcttgacgtcgacgtcatcgaccaggcgggcgacgtcatcgaatgcacgtcccagaaggtcggtttccgccgcttccgcatcgaggacggcatcctgaccatcaacggcaagcgcatcgtgttcaagggcgccgaccgccacgagttcgacgccgaacggggccgcgccatcaccgagcaggacatgatcgatgacgtggtcttctgcaagcgccacaacatcaactccatccgcacctcgcactacccgaaccaggaacgctggtacgaactgtgcgacgagtacggcatctacctgatcgacgaagccaacctcgaagcccacggcagctggtccctgcccggagacgtcctcaccgaggacaccatcgtgccgggtagcaagcgcgaatgggaaggcgcctgcgtcgaccgcgtcaacagcatgatgcgtcgcgactacaaccacccgagcgtgctgatctggtcactgggcaacgaatcctacgtgggcgacgtgttccgcgccatgtacaagcacgtgcacgacatcgacccgaaccgtccggtgcactacgagggcgtgacccacaaccgtgactacgatgacgtcaccgacatcgagacccgtatgtactcgcatgccgacgagatcgagaagtacctgaaggacgacccgcagaagccgtacctctcctgcgaatacatgcacgccatgggcaactccgtgggcaacatggacgaatacacggcgctcgaacgctacccgaagtatcagggcggcttcatctgggacttcatcgaccaggccatctacgccacccagcccgacggcaccaggagcctgcgctacggcggagacttcggcgaccgtccgtccgactacgagttctccggcgacggcctgctgttcgccgaccgcaagccttcccccaaggcccaggaagtcaagcagctgtactcgaacgtccacatcgacgtgacgaaggactcggtgtccgtcaagaacgacaacctgttcaccgccaccggcgactacgtgttcgtcctgagcgttctcgccgacggcaagccggtctggcagtccacccggcgtttcgacgtgcccgccggtgagacccgcacgttcgatgtcgcatggccggtggcggcgtaccgcgccgacgcccgcgaactggtgctgcaggtttcgcagcgtctcgccaaggcgaccgattgggccgagagcggctacgagctcgccttcggacagaccgtggtgcccgcggacgccaccgcgacgcccgacacgaagccggccgatgggaccatcaccgtgggccgttggaacgccggcgtgcgaggcgccggacgcgaggtcctgctgtcgcgcacccagggcggcatggtctcctacaccttcgccggcaacgagttcgtgctgcgccgtcccgcaatcaccaccttccgtccgctgactgacaacgatcgcggcgccggtcatggcttcgagcgcgtccagtggctgggcgccggacgctacgcccgctgcgtggacaacgtgctcgagcagatcgacgacagcacgctcaagggcacgtacacgtatgagctcgccaccgcgcagcgcaccaaggtgaccgtctcctacacggcccacaccgatggccgcgtgaacctgcacgtcgaataccctggagagcagggtgacctgcccaccatcccggcgttcggcatcgaatggacgctgcctgtgcagtacacgaacctgaggttcttcggcaccggcccggcggagacgtacctggaccgcaaacacgccaagctcggcgtgtggagcaccaacgctttcgcggatcatgcgccgtacctcatgccgcaggagacgggcaaccatgaggatgtgcgttgggccgagattaccgacgatcacggccacggcatgcgcgtcagccgcgccgatggtgccgcgccgttcgcggtaagcctgttgccgtactccagcttcatgcttgaggaggctcagcaccaggacgagctgccgaagccgaagcacatgttcctgcgcgtccttgccgcacagatgggcgttggcggcgatgattcctggatgtcgccggtgcacccccagtaccatatcccggcggacaagccgatcagcctcgatgtcgacctcgagctgatctga

SEQ ID NO: 106 - DNA, 1701 bp, Bifidobacterium sp.
  source: /note="GH51.0-6"
atgaccactcacaacagccagtattccgccgaaaccacccatcccgacaagcaggaaagcagcccggcgccgaccgccgccggcaccacggccagtaacgtctccacaactggcaacgcaaccacgccggacgccagcatcgccctcaacgccgacgccactccggtagccgacgttcccccgcgtctgttcggctcattcgtagaacatctgggccgctgcgtctacggcggcatctacgagcccagccatcccaccgccgacgaaaacggcttccgccaagacgtgcttgacctggtcaaggagctgggcgtcacctgcgtgcgctaccccggcggcaatttcgtatccaactacaactgggaagacggcatcggtccacgcgagaatcgccccgtgcgccgcgacctggcctggcattgcaccgaaaccaacgagatgggcatcgacgacttctaccgctggagccagaaagccggcaccgaaatcatgcttgccgtcaacatgggcacccgggggctgaaagccgcgctcgacgagctcgagtatgtcaacggcgcgcccggcaccgcttgggcggatcagcgcgtggccaacggcatcgaggagccgatggatatcaagatgtggtgcatcggcaacgaaatggacggcccgtggcaggtgggccacatgagcccggaagaatatgccggcgcggtggataaggtggcccacgccatgaagctcgccgagtccggtctcgaactcgtggcctgcggttcctcgggtgcctatatgccgaccttcggcacgtgggagaagaccgtgctcaccaaggcttacgagaatctcgacttcgtctcctgccatgcctactacttcgaccgcggccataaaacccgggccgccgcctccatgcaggacttcctggcctcttccgaagacatgaccaagttcatcgccaccgtctcggacgcggccgatcaggcgcgcgaagccaataacggcaccaaagacatcgccctgtccttcgacgaatggggcgtatggtattcggacaagtggaacgagcaggaagaccagtggaaggcggaggccgcgcagggtttgcaccacgagccatggcctaagtctccgcatttgctggaagacatctacaccgcggccgacgcggtggtcgaaggttccctgatgatcaccctgctcaagcactgcgatcgcgtgcgttccgcctcgcgcgcccagctggtcaacgtcatcgcccccatcatggccgaggaacacggcccggcatggcggcagaccacgttctacccgttcgccgaagccgcccttcacgcgcgcggccaggcctacgctccggccatcagctcccccaccatccataccgaggcatatggcgacgtgccggccatcgacgcggtagtcacgtgggatgaacaggcccgcaccggtctgctgcttgccgtcaaccgcgacgccaacaccccacacacgctcaccatcgacctttccgggctgcccggcctgcccggtctcggcacgctcgcgctcggcaaggcgcaactgttgcatgaggacgatccgtaccgcaccaacaccgccgaagcgcccgaagccgtcacgccgcaaccgctcgacattgcgatgaacgccaccggcacctgcacggcaacgcttcccgccatctcctggatcagcgtggaattccacggctaa

SEQ ID NO: 107 - DNA, 1548 bp, Bifidobacterium sp.
  source: /note="GH51.0-9"
atgccccagcaggaccatctgaccgcacgtctcgtcgtcgatgacgattttgaggtcgctccggtcaacaatcgtctgttcggttcgttcgtcgagcaccttggccgttgcgtgtacaccggcatctacgagcccgaccacccgaccgccgacgagcacggcttccgcaaggacgtcatcgacctggtcaaggaactcggcgccaccaccatccgctacccgggcggcaacttcgtgtccggctaccgctgggaggacggcatcggccccaagcaggaacgtccccgtcgactcgatctggcctggcattccaccgaaaccaacgaattcggcctgcacgagatggccgaatggcttgaggccaccggcggcaacgagctgatggaggccgtcaacctgggcacgcgcggcctgcaggaggccctggacctgctggagtacgcgaacgtgcccggcggcaccgagctgtcggaacgtcgccgcgccaacggcgccgacaagccgttcgatatccgcatgtggtgcctgggcaacgagatggacggcccgtggcagctcggccacaagtccgccgaggactacggcatgctcgccgcctccgtggccgccggcatgcgccagatcgatccggacgtggaactggtggtgtgcggctcctccgcccatggcatgccgaccttcggcaagtgggagcagaccgttcttgagaagacctacgagaacgtgaacttcgtctcctgccacgcctactaccagccgttcttcaaggaggacggcacgcgcgacatggccagcttcctggcctccggcgtggatatggacggcttcatcaaggacgtggccgccaccatcgacgccaccaaggcccatctgaagagcgcgcacgacgtgtacatctcgttcgatgaatggaatgtctggtaccagggtgaggagccgagcaagacccccgagggcatcggcaactggccggtggccccgcgtctgctggaggacatctacaccgccgccgacgccgtggtgttcggcgatctgatgatcacgctgctcaagaacgccgaccgcgtgcgcgccgccagcctggcgcagctggtcaatgtcatcgccccgatcatgacggagccgggcggcccggcctggcgccagaccacgttccacccgttctccgtgaccgcgcgcctggccaagggcggcaccgtgctggagccgaagctgtccgccggcaccgtggatacgccgcgctatggcgaggtcgacggcgtgaacgccgtggccgtgcgctgcgccgacggctcgctcgccgtgtttgcggtgaaccgttcgctcgaggcgaccgccgagttcgagatcaggctgcaggacggcgcgcagccggcatccgtcgaggcgcagacgctgcacgacgacgatctgttcgccgcgaatacgctctacgaccagaaccgtgtgaccccgcgcgccaacgggtcggccatgtacgatgccgagtccggcgtggtccgcgtctccctgccgccggtgagttggaccgccctgcacatcaagtga

SEQ ID NO: 108 - DNA, 1548 bp, Bifidobacterium sp.
  source: /note="GH51.0-11"
atgccccagcaggaccatctgaccgcacgtctcgtcgtcgatgacgattttgaggtcgctccggtcaacaatcgtctgttcggttcgttcgtcgagcaccttggccgttgcgtgtacaccggcatctacgagcccgaccacccgaccgccgacgagcacggcttccgcaaggacgtcatcgacctggtcaaggaactcggcgccaccaccatccgctacccgggcggcaacttcgtgtccggctaccgctgggaggacggcatcggccccaagcaggaacgtccccgtcgactcgatctggcctggcattccaccgaaaccaacgaattcggcctgcacgagatggccgaatggcttgaggccaccggcggcaacgagctgatggaggccgtcaacctgggcacgcgcggcctgcaggaggccctggacctgctggagtacgcgaacgtgcccggcggcaccgagctgtcggaacgtcgccgcgccaacggcgccgacaagccgttcgatatccgcatgtggtgcctgggcaacgagatggacggcccgtggcagctcggccacaagtccgccgaggactacggcatgctcgccgcctccgtggccgccggcatgcgccagatcgatccggacgtggaactggtggtgtgcggctcctccgcccatggcatgccgaccttcggcaagtgggagcagaccgttcttgagaagacctacgagaacgtgaacttcgtctcctgccacgcctactaccagccgttcttcaaggaggacggcacgcgcgacatggccagcttcctggcctccggcgtggatatggacggcttcatcaaggacgtggccgccaccatcgacgccaccaaggcccatctgaagagcgcgcacgacgtgtacatctcgttcgatgaatggaatgtctggtaccagggtgaggagccgagcaagacccccgagggcatcggcaactggccggtggccccgcgtctgctggaggacatctacaccgccgccgacgccgtggtgttcggcgatctgatgatcacgctgctcaagaacgccgaccgcgtgcgcgccgccagcctggcgcagctggtcaatgtcatcgccccgatcatgacggagccgggcggcccggcctggcgccagaccacgttccacccgttctccgtgaccgcgcgcctggccaagggcggcaccgtgctggagccgaagctgtccgccggcaccgtggatacgccgcgctatggcgaggtcgacggcgtgaacgccgtggccgtgcgctgcgccgacggctcgctcgccgtgtttgcggtgaaccgttcgctcgaggcgaccgccgagttcgagatcaggctgcaggacggcgcgcagccggtatccgtcgaggcgcagacgctgcacgacgacgatctgttcgccgcgaatacgctctacgaccagaaccgtgtgaccccgcacgccaacgggtcggccatgtacgatgccgagtccggcgtggtccgcgtctccctgccgccggtgagttggaccgccctgcacatcaagtga

SEQ ID NO: 109 - DNA, 1353 bp, Citrobacter sp.
  source: /note="GH4.0-1"
atgtctgcacccaaaattacctttatcggcgccggttccacaattttcgtcaaaaatattcttggggacgtctttcaccgcgatgcgcttaaatctgcgcatatcgccttgatggatctcgatcctacgcgtctggaagaatcacacgttgttgtgcgcaagttgatggattctgcgggcgcgtctggacgaatcacctgctataccgatcaaaaagcggcattacaggatgccgattttgtggtggtcgctttccagatcggcggctatgaaccctgtaccgttaccgattttacggtgtgtaaacgccatggtctggagcagacgattgccgacacgctggggccgggcggcattatgcgcgcgctgcgcaccatcccgcatttatggcagatttgtgaggatatgaccgaagtctgtccgcaggccacaatgcttaactacgttaacccgatggcaatgaatacctgggcaatgtatgcgcgctatccgcatattaagcaggttgggttgtgtcattcggtgcaggggacggcggaggagttggcccgcgatctgaacatcgaccctgcttctttgcgctatcgcagtgccgggatcaaccatatggcgttttatctggagctggagcgcaaaacggcggacggtgcctatgtgaatctctacccggagctgctggcggcctatgaatctggtcaggcgccgaaaccaaatattcacggaaatacccgttgccagaacattgtgcgctatgaaatgttcaaaaaattggggtatttcgtcaccgaatcgtcggagcacttcgctgaatatacgccgtggtttatcaaaccggggcgtgaagatctgattgagcgctataaggtgccattggatgaatatccgaaacgttgtgtggaacagttggcgaactggaaaaaagagctggaagagtacaaaacggctgagcggatcgacattaaaccgtcgcgcgaatatgccagcactatcatgaacgctatctggaccggtgaaccgagcgtcgtgtatggcaacgttcgcaatgacaatctgatcgataacctgccgcaaggctgctgcgttgaagtcgcttgtctggtcgatgcaaatggtattcagccaacgaaagtcgggactctcccgtcacatttggcggccatgatgcaaaccaatatcaatgttcagaccctgctaacggaagccatcctgacggagaatcgcgatcgcgtttatcacgcggcgatgatggatccgcataccgccgcggtactggggattgaagagatttatgcgctggtggacgacctgatcgcgtctcacggcgactggctgccggcctggctgcaccgttaa

SEQ ID NO: 110 - DNA, 2325 bp, Bacteroides sp.
  source: /note="GH3.0-7"
atgaagaagaatatcatatccatggcagcagcaatggctgttttgtcagcttgcggaccgggtgtgccgcagcttggaaagtcctctctggatgaggtgattggcgccatgaccttggaagaaaaggcgcatctggtagtgggtaccggtatggcaggtttctcgggtgacagtgccgtaatcggtgcaacgagaaagctagtgccgggtgcggcaggaaccacatacccgattgaacgcctcggcattcccgctgtggtgctggctgatggtcccgccggactgcgtatcgaccccaagcgtgagggggattcggctacgtactattgtactcatttccctatcggaactttgctcgcctctacctgggaccaggaactggtggaaagtgtaggtcagtccatcggtaacgaagtgctggaatacggtgcggacgtgctgttggctccggcgctgaacattcaccgtaacccgctttgcggacgtaacttcgagtattattctgaagacccgttggtgtcgggtaagattgccgccgcctacgtacgtggtgtgcagagcaacggtgtgggtaccagtatcaagcactttgctgtgaacaaccaggaaaccaaccgtatggctacggatgcgcatgtatctccacgcgccttgcgcgaaatctacttgaaagggttcgagattgccgtgaaggaatccgctccttggactgtgatgtcctcatacaactacctgaacggtgtctacacttcggaaaacaaggagttgcagacaaccatgttgcgcgacgaatggggcttcaaaggcatagtgatgaccgactggtttggcggcaaggatgccgtggcacagatggtggcaggcaacgacatgttgcagcccggtctgcccaagcagtacgaagccatcgtgaagggtgtgcaggacggagcgttagatgaagccatcctcaatcagaatgtgaagcgtattctggagatgattctccagactccccacttcaagggatataaatactccaacaagcctgatttgaaggcgcatgctgccgttactcgccagtcggcaacggaaggtatggtattgctgaagaacgataacggtgctctgccgctggctgccgacgtgaagaacgtggcactcttcggttgcacttcctacgatttcattgcaggcggtacaggttcgggcaacgtgaaccgcgcttataccgtttcgctattggacggcttgaagaatgccggctatgtggtggatgaagcgctgaagaatagctatgaagcttacctgaaaaccgagaaagaacgtctgtccaaagataagaaagagtggttcatgcccgatacccgtccggctgagatggctgtttccgcacaagtcatccgcgagcaggctgccaaggccgatgtggcactggtgacgctgggacgtacctccggtgagttccttgaccgtatggtagccgacttcaacctcaccaaagaggaacagaacatgttgaaagctgtgtccgatgctttccacgctgccggaaagaaggtagtggtagtgctcaatatcggtggtgtgattgaaactgcttcttggaaatctgctcccgatgccattctttgtgcatggcaggcaggccaggagggaggaaacagtgtggctgacgtgctgagtggcaaggcttctccttcgggcaagctgacaatgactttcccggtgaagtttgaagatgccgcttcttccgacaacttcccgatagacatgcgtgtgagcaccgacctcatgaacaaaggcgggaagaagaacgacgtgaagaacgtggactataccaattacgaagaggacatttacgtgggttaccgttacttcgacacctttggcaagcaggtttcctatcctttcggttacggtctttcctataccacttttgcttacgacaaggctgctgtcaaggcagacaacggtgtctataccgtgtctgtagaagtgaagaacaccggtaaggtagcaggcaaggaagtggttcagctttatgtatccgctcccgatgttgctgccaacaagcccgaaaaggaactgaaggcttttgccaagaccaaggagctgaaaccgggcgaagcggttgtggtgacgctgaaagtgaatgctgatgacctggcttcctacgatgaggctgcatcggcatgggtggtaactcccggaaactacaagttcctcgtcggggcttcctcacgcgacatcaaggctacgctggaggctgaagtagctgccgcaacgcagaagacgaacaacatcctgaaacttcaggaaccgatgagcctcttgaagagatga

SEQ ID NO: 111 - DNA, 2247 bp, Bacteroides sp.
  source: /note="GH31.0-10"
atgaaacctactaattaccatttgttcgatttccttgatttcgatacagagttattaagggatgagtcactttggaaagcctgtaaaccgacagccgtttacgaaaaggatggggatatctgtgtcacggtcccctttcaaaaacagctgttagctaatgatatggttgcggatacggctgtcccccgagaagaatatacgttgatcatacgccagtataatatcggcattacccgtctgtttcttggatttggtgaatatgaactgacagatcagtcggaaatgctgcaattcagcgaacggattcgcagagtacctttgtctgtagagaagcagggaggcaaatggattcttttcacccaagacgggacgaagcgtgccgttatcaatgtagaagagccggctttggaccgatggagcgagttactgcccgatcctcaggaaacactggacatcactctgtatcctgacggcaaacgggaaatccgcctggcagcatacgatcatttctcgcctccccgctatgacggactgcccattgccttctgcaaatggacgggcaaaaaggaacgtgccaccctttctttcgagagccggccggatgaatgctttgcaggaaccggagagcgtttcttcaaaatggacttgagcggacagacgcttttcctcaagaatcaggatgggcagggagtaaataaccggcgtacctataagaatatacctttctatctctccagccggatgtacgggactttttaccatacctgcgcccacagcaaactttcgctggcgggacattccacccgctccgtacagttcctgagcgatcaggctatgctggatgcatttgtcattgccggcgatacgatggaagagatacttcgcggctaccgtgacctgaccggatatccttcgatgcctcctctctggagcttcggagtgtggatgagccggatgacttatttcagtgccgacgaagtaaatgagatctgcgatcgtatgcgtgccgaacattatccctgcgatgtcatccatctggataccggatggttcagaaccgactggctgtgtgaatggaagtttaacgaggaacgttttcccgacccgaaaggattcattcagagattgaagaagaacggttatcgtgtgtccttatggcagttaccttatgttgctgaagatgcggaacagatcgaggaggcaaaggcgaatgagtatatagctcctctgacgaagcagcaggacacggacggttccaacttctcggctctggattatgcgggtactatcgactttacttatccgaaggcaaccgaatggtacaaggggctattaaagcaacttctggatatgggagtcacctgtattaaaaccgatttcggagaaaatatccacatggatgctgtctacaagggcatgaaaccggaactgttgaataacctgtatgccttgctctatcagaaagcagcttacgaaataacaaaggaggtaacaggggacggcattgtctgggcacgtgccgcttgggcgggttgccaacgttatccgttgcactggggaggtgactcctgcagttcatgggatggcatggccggttcactcaaaggaggcctgcacttcggtttatcgggctttgccttctggagccatgatgtccccggattccataccttgcccaattttatgaactcaatcgtagcggaggacgtctatatgcgctggacccagtttggagtgttcacctcacacatccgttatcatggaaccaataagcgggaaccctggcattatccggctatcgccccgctggtgaagaagtggtggaaactgcgctactcgttgattccctacatcatagagcaaagtaaactggcagtagaaagtggctggccattgttacaggcactcatcctgcatcatccggaagataaactctgctggcatatcgatgacgaatattacttcggcaatgatttcctggtagctccggtgatgaatagcgaaaaccgtcgcgacatttatctccccgaaggacagtgggtgaatttctttaccggcgaacggttgcaaggcggacgctggctgaaagaggtgtatgtgcccttggaagagatgcctgtttatgtgcgtgagaatgccgttatcccgatttatccggaggaagtgaattgtacggacgagatggatttaggcaaaagtattgccttgcgcatagatcataattacaaaggattttggactaaataa

SEQ ID NO: 112 - DNA, 2247 bp, Bacteroides sp.
  source: /note="GH31.0-11"
atgaaacctactaattaccatttgtttgatttccttgatttcgatacagagttattaagggatgagtcactttggaaagcctgtaaaccgacagccgtttacgaaaaggatggggatatctgtgtcacggtcccctttcaaaaacagctgttagctaatgatatggttgcggatacggctgtcccccgagaagaatatacgttgatcatacgccagtataatatcggcattacccgtctgtttcttggatttggtgaatatgaactgacagatcagtcggaaatgctgcaattcagcgaacggattcgcagagtacctttgtctgtagagaagcagggaggcaaatggattcttttcacccaagacgggacgaagcgtgccgttatcaatgtagaagagccggctttggaccgatggagcgagttactgcccgatcctcaggaaacactggacatcactctgtatcctgacggcaaacgggaaatccgcctggcagcatacgatcatttctcgcctccccgctatgacggactgcccattgccttctgcaaacggacgggcaaaaaggaacgtgccaccctttctttcgagagccggccggatgaatgctttgcaggaaccggagagcgtttcttcaaaatggacttgagcggacaaacgcttttcctcaagaatcaggacgggcagggagtaaataaccggcgtacctataagaatatacctttctatctctccagccggatgtacgggactttttaccatacctgcgcccacagcaaactttcgctggcgggacattccacccgctccgtacagttcctgagcgatcaggctatgctggatgcatttgtcattgccggcgatacgatggaagagatactccgcggctaccgtgacctgaccggatatccttcgatgcctcctctctggagtttcggagtgtggatgagccggatgacttatttcagtgccgacgaagtaaatgagatctgcgaccgtatgcgtgccgaacattatccctgcgatgtcatccatctggataccggatggttcagaaccgactggctgtgtgaatggaagtttaacgaggaacgttttcccgacccgaaaggattcattcagagattgaagaagaacggttatcgtgtgtccttatggcagttaccttatgttgctgaagatgcggaacagatcgaagaggcaaaggcgaatgagtatatagctcctctgacgaagcagcaggacacggacggttccaacttctcggctctggattatgcgggtactatcgactttacttatccgaaggcaaccgaatggtacaaggggctattaaagcaacttctggatatgggagtcacctgtattaaaaccgatttcggagaaaatatccacatggatgctgtctacaagggcatgaaaccggaactgttgaataacctgtatgccttgctctatcagaaagcagcttacgaaataacaaaggaggtaacaggggacggcattgtctgggcacgtgccgcttgggcgggttgccagcgttatccattgcactggggaggtgactcctgcagttcatgggatggcatggccggttcactcaaaggaggcctgcacttcggtttatcgggctttgccttctggagccatgatgtccccggattccataccttgcccaattttatgaactcaatcgtagcggaggacgtctatatgcgctggacccagtttggagtgttcacctcacacatccgttatcatggaaccaataagcgggaaccctggcattatccggctatcgccccgctggtgaagaagtggtggaaactgcgctactcgttgattccctacatcatagagcaaagtaaactggcagtagaaagtggctggccattgttacaggcactcatcctgcatcatccggaagataaactctgctggcatatcgatgacgaatattacttcggcaatgatttcctggtagctccggtgatgaatagcgaaaaccgtcgcgacatttatctccccgaaggacagtgggtgaatttctttaccggcgaacggttgcaaggcggacgctggctgaaagaggtgtatgtgcccttggaagagatgcctgtttatgtgcgtgagaatgccgttatcccgatttatcctgaggaagtgaattgtacagacgagatggatttaagcaaaagtattgccttgcgcatagatcataattacaaaggattttggactaaataa

SEQ ID NO: 113 - DNA, 2340 bp, Bacteroides sp.
  source: /note="GH92.0-3"
atgaataagatgaaaaagaaagtattgatgatgactatggcggcggtaaccttgtccgccgtagctcagcaaccggtagattacgttaatccgattatcggaaccaatggtatggggcatacttttcccggtgcttgcacccctttcggatgggtacagctgagtccggacacagacacaattccacataatgtgaatggagcttatcagaagaatgcgtatgaatattgtgccggttaccagtatcgggataaaaccatcgtaggtttcagtcacacccacctcagcggcacgggacattccgacctgggagatatattgctgatgcctgctgtcggcgatgtaaaattgaatcccggacgggcggaccatccggaagagggttaccgttcgcgcttcgatcatgccacagagaaagcgacacccggatactacgaagtgatgctggacgactatggcattaaagcgcaactgacagctactcaacggacgggtgtacataaatataccttcccgaaaggaaaagacggtcatctgatcctggacctggtgcatggtatctataattatgacggcaaagtattgtgggcaaacctgcgggtggaaaacgatacattgctgacaggataccgcatcaccaacggatgggcacgtacgaattatacctattttgccatttccttgtcacagccgatcaaggattacggatataaggataaggaaaaggtattgtacaatggcttttggcgtcgtttcaagctggagaagaatttcccggaaatcactggtcgaaagatcgtggcttactttaacttcgaaacggccaaagatcccgaactggttgtaaaggtagccttgtcggcagtcagcacggaaggcgctgtaaagaacctgcgtgccgaggcttccggaaagagcttcgaacagttggcggaagctgcacggacagactggaacaatgaactggatcatttcgaaatagaaggtacaccggatcagaaggcgatgttctacacttcgctttatcataccatgattaatccgtccgtgtatatggacgtagacggttcctatcgcggtctggatcataacatacatcaggcgaaaggattcactaactatactatattctcactttgggatacatatcgcgcggaacatccgttccttaacctggtgaaaccggaacgcaatgcggatatggtggaatcaatgatcaaacatgaacagcagagcgtgcatggcatgttgccgatatggagcctgatgggaaatgagaactggtgtatgagcggttatcatgctgtgtctgtgctggcggatgcaataaccaaaggagttttttcaaatgtggatgaggcattatcggcgatggttagcacatctacggtaccttactatgaaggtgtagccgattatatgaagctgggatatatcccgctggacaagagtggtacggcagcttcctctacgttggaatatgcatacgacgactggactatttatcagacagccttgaaagccggtaataaagagatagcggatacttaccgcaaacgtgctctcaactatcgtaacatctatgatacaagcatcggttttgcccgtccccgctacagtgacggcacattcaaaaaagagttcgatgtgttgcaaacttacggcgaaggctttatcgaaggtaattcatggaacttctcctttcatgtaccgcatgatgtgtttggtatgatcgacctgatgggaggagaaaagacattcgtacagaaactggacgaactcttctccatgcatctgccggagaagtactatgaacataatgaggatattacggaagaatgcctggtaggtggatacgtacatggcaatgaaccgagccatcatgtaccttatttgtacgcatggacctcccaaccgtggaaaacacagtactggctgcgtgaaatcctgaacaagatgtataagaatgacatcaacggactgggtggaaatgatgattgcggacagatgtcggcatggtatcttttctctgtgatgggcttctatccggtttgtccgggtacagaccagtatgtccttggtgctccctatctgccctatctgaagctgacacttcccaacggaaagacactggaaatcaaagcgccgggcgtcagcgacaagaagcgttatgtacagtcactgaaactgaacggcgagtcttatgataaaatgtacatcacacacgaggatatcctgaaaggaggcgtattggaatttaaaatgtcggcatcgcccaacaaacgtcgtggagtatcggcgcaggacaaaccttattcattaactaatggaatcaattaa

SEQ ID NO: 114 - DNA, 3072 bp, Bifidobacterium sp.
  source: /note="GH2.0-4"
atgacagacgtcacacatgtcgatcgcgcatcgcaggcttggctgaccgacccgacggtgttcgaggtgaaccggactccggcccattccagccacaagtgctacgcccgcgacccccagagcggacaatggtccgatctcaagcagagccttgacggcgagtggcgggtcgaggtcgttcaggccgccgacatcaacctcgaagaggaacccgcgacggccgagtcgttcgacgactcctcgttcgagcgtatccaggttccgggccacctgcagacggccggtctgatgaaccacaagtacgtgaacgtccagtatccgtgggacggccacgagaacccgttggaaccgaacatcccggagaacaatcacgtcgcgctctaccgcaggaagttcaccgtctccgcccccgtggcaaacgccaagcaggccggcggatcggtgtcgatcgtgttccacggcatggccacggcgatctacgtgtgggtcaacggcgcgttcgtcggctatggcgaggacggcttcacgcccaatgagttcgacatcaccgaactgctgcacgacggggagaacgtcgtggccgtcgcctgctacgaatactccagcgcctcctggcttgaggatcaggacttctggcgtctgcacggcctgttccgctccgtcgaactcgccgcccgcccgcatgtgcacatcgagaacacgcagatcgaagccgattgggatcccgaggccggcaccgcctccctcgatgccgcgctgaccgtgctcaacgcggccgacgcggccacggtccgcgcgaccctgaaggacgccgacggcaacacggtgtggcagacgacgggcgacgcggaggcgcagaccgcgatctccagcgggccgctgcagggcatcgccccttggagcgccgaaagcccgacgctgtacgagcttgacgtcgacgtcatcgaccaggcgggcgacgtcatcgaatgcacgtcccagaaggtcggtttccgccgcttccgcatcgaggacggcatcctgaccatcaacggcaagcgcatcgtgttcaagggcgccgaccgccacgagttcgacgccgaacgcggccgcgccatcaccgagcaggacatgatcgatgacgtggtcttctgcaagcgccacaacatcaactccatccgcacctcgcactacccgaaccaggaacgctggtacgaactgtgcgacgagtacggcatctacctgatcgacgaagccaacctcgaagcccacggcagctggtccctgcccggagacgtcctcaccgaggacaccatcgtgccgggtagcaagcgcgaatgggaaggcgcctgcgtcgaccgcgtcaacagcatgatgcgtcgcgactacaaccacccgagcgtgctgatctggtcactgggcaacgaatcctacgtgggcgacgtgttccgcgccatgtacaagcacgtgcacgacatcgacccgaaccgtccggtgcactacgagggcgtgacccacaaccgtgactacgatgacgtcaccgacatcgagacccgtatgtactcgcatgccgacgagatcgagaagtacctgaaggacgacccgaagaagccgtacctctcctgcgaatacatgcacgccatgggcaactccgtgggcaacatggacgaatacacggcgctcgaacgctacccgaagtatcagggcggcttcatctgggacttcatcgaccaggccatctacgccacccagcccgacggcaccaggagcctgcgctacggcggagacttcggcgaccgtccgtccgactacgagttctccggcgacggcctgctgttcgccgaccgcaagccttcccccaaggcccaggaagtcaagcagctgtactcgaacgtccacatcgacgtgacgaaggactcggtgtccgtcaagaacgacaacctgttcaccgccaccggcgactacgtgttcgtcctgagcgttctcgccgacggcaagccggtctggcagtccacccggcgtttcgacgtgcccgccggtgagacccgcacgttcgatgtcgcatggccggtggcggcgtaccgcgccgacgcccgcgaactggtgctgcaggtttcgcagcgtctcgccaaggcgaccgattgggccgaaagcggctacgagctcgccttcggacagaccgtggtgcccgcggacgccaccgcgacgcccgacacgaagccggccgatgggaccatcaccgtgggccgttggaacgccggcgtgcgaggcgccggacgcgaggtcctgctgtcgcgcacccagggcggcatggtctcctacaccttcgccggcaacgagttcgtgctgcgccgtcccgcaatcaccaccttccgtccgctgaccgacaacgatcgcggcgccggtcacggtttcgagcgcgtccagtggctgggcgccggccgctacgcccgctgcgtggacaacgtgctcgagcagatcgacgacagcacgctcaagggcacgtacacgtatgagctcgccaccgcgcagcgcaccaaggtgaccgtctcctacacggcccacaccgatggccgcgtgaacctgcacgtcgaataccctggagagcagggtgacctgcccaccatcccggcgttcggcatcgaatggacgctgcctgtgcagtacacgaacctgaggttcttcggcaccggcccggcggagacgtacctggaccgcaaacacgccaagctcggcgtgtggagcaccaacgctttcgcggatcatgcgccgtacctcatgccgcaggagacgggcaaccatgaggatgtgcgttgggccgagattaccgacgatcacggccacggcatgcgcgtcagccgcgccgatggtgccgcgccgttcgcggtaagcctgttgccgtactccagcttcatgcttgaggaggctcagcaccaggacgagctgccgaagccgaagcacatgttcctgcgcgtccttgccgcacagatgggcgttggcggcgatgattcctggatgtcgccggtgcacccccagtaccatatcccggcggacaagccgatcagcctcgatgtcgacctcgagctgatctga

SEQ ID NO: 115 - DNA, 3072 bp, Bifidobacterium sp.
  source: /note="GH2.0-6"
atgacagacgtcacacatgtcgatcgcgcatcgcaggcttggctgaccgacccgacggtgttcgaggtgaaccggactccggcccattccagccacaagtggtacgcccgcgacccccagagcggacaatggtccgatctcaagcagagccttgacggcgagtggcgggtcgaggtcgttcaggccgccgacatcaacctcgaagaggaacccgcgacggccgagtcgttcgacgactcctcgttcgagcgtatccaggttccgggccacctgcagacggccggtctgatgaaccacaagtacgtgaacgtccagtatccgtgggacggccacgagaacccgttggaaccgaacatcccggagaacaatcacgtcgcgctctaccgcaggaagttcaccgtctccgcccccgtggcaaacgccaagcaggccggcggatcggtgtcgatcgtgttccacggcatggccacggcgatctacgtgtgggtcaacggcgcgttcgtcggctatggcgaggacggcttcacgcccaatgagttcgacatcaccgaactgctgcacgacggggagaacgtcgtggccgtcgcctgctacgaatactccagcgcctcctggcttgaggatcaggacttctggcgtctgcacggcctgttccgctccgtcgaactcgccgcccgcccgcatgtgcacatcgagaacacgcagatcgaagccgattgggatcccgaggccggcaccgcctccctcgatgccgcgctgaccgtgctcaacgcggccgacgcggccacggtccgcgcgaccctgaaggacgccgacggcaacacggtgtggcagacgacgggcgacacggaggcgcagaccgcgatctccagcgggccgctgcagggcatcgccccttggagcgccgaaagcccgacgctgtacgagcttgacgtcgacgtcatcgaccaggcgggcgacgtcatcgaatgcacgtcccagaaggtcggtttccgccgcttccgcatcgaggacggcatcctgaccatcaacggcaagcgcatcgtgttcaagggcgccgaccgccacgagttcgacgccgaacgcggccgcgccatcaccgagcaggacatgatcgatgacgtggtcttctgcaagcgccacaacatcaactccatccgcacctcgcactacccgaaccaggaacgctggtacgaactgtgcgacgagtacggcatctacctgatcgacgaagccaacctcgaagcccacggcagctggtccctgcccggagacgtcctcaccgaggacaccatcgtgccgggtagcaagcgcgaatgggaaggcgcctgcgtcgaccgcgtcaacagcatgatgcgtcgcgactacaaccacccgagcgtgctgatctggtcactgggcaacgaatcctacgtgggcgacgtgttccgcgccatgtacaagcacgtgcacgacatcgacccgaaccgtccggtgcactacgagggcgtgacccacaaccgtgactacgatgacgtcaccgacatcgagacccgtatgtactcgcatgccgacgagatcgagaagtacctgaaggacgacccgaagaagccgtacctctcctgcgaatacatgcacgccatgggcaactccgtgggcaacatggacgaatacacggcgctcgaacgctacccgaagtatcagggcggcttcatctgggacttcatcgaccaggccatctacgccacccagcccgacggcaccaggagcctgcgctacggcggagacttcggcgaccgtccgtccgactacgagttctccggcgacggcctgctgttcgccgaccgcaagccttcccccaaggcccaggaagtcaagcagctgtactcgaacgtccacatcgacgtgacgaaggactcggtgtccgtcaagaacgacaacctgttcaccgccaccggcgactacgtgttcgtcctgagcgttctcgccgacggcaagccggtctggcagtccacccggcgtttcgacgtgcccgccggtgagacccgcacgttcgatgtcgcatggccggtggcggcgtaccgcgccgacgcccgcgaactggtgctgcaggtttcgcagcgtctcgccaaggcgaccgattgggccgaaagcggctacgagctcgccttcggacagaccgtggtgcccgcggacgccaccgcgacgcccgacacgaagccggccgatgggaccatcaccgtgggccgttggaacgccggcgtgcgaggcgccggacgcgaggtcctgctgtcgcgcacccagggcggcatggtctcctacaccttcgccggcaacgagttcgtgctgcgccgtcccgcaatcaccaccttccgtccgctgaccgacaacgatcgcggcgccggtcacggtttcgagcgcgtccagtggctgggcgccggccgctacgcccgctgcgtggacaacgtgctcgagcagatcgacgacagcacgctcaagggcacgtacacgtatgagctcgccaccgcgcagcgcaccaaggtgaccgtctcctacacggcccacaccgatggccgcgtgaacctgcacgtcgaataccctggagagcagggtgacctgcccaccatcccggcgttcggcatcgaatggacgctgcctgtgcagtacacgaacctgaggttcttcggcaccggcccggcggagacgtacctggaccgcaaacacgccaagctcggcgtgtggagcaccaacgctttcgcggatcatgcgccgtacctcatgccgcaggagacgggcaaccatgaggatgtgcgttgggccgagattaccgacgatcacggccacggcatgcgcgtcagccgcgccgatggtgccgcgccgttcgcggtaagcctgttgccgtactccagcttcatgcttgaggaggctcagcaccaggacgagctgccgaagccgaagcacatgttcctgcgcgtccttgccgcacagatgggcgttggcggcgatgattcctggatgtcgccggtgcacccccagtaccatatcccggcggacaagccgatcagcctcgatgtcgacctcgagctgatctga

SEQ ID NO: 116 - DNA, 1707 bp, Bacteroides sp.
  source: /note="GH110.0"
atgatgagcgtttggttcatccagttggctatttttgcccagtctagaataatagaggtttttccggagcagggaaaagatattgaaaatatagcgttagctttaaaaaaagctgctgactgtaaaggaaggccggttactgtaaagttttcaccgggaatttatcagttagaccgtgcgaaatcatcacaagtgttatattatatatcaaatacgacttctgagttggatgatcctgatccgactaaacatatcggattgtatcttaatacattaaagaatatcactattgatggttgtgggtcaactttattgatgaatggtgaaatgacaagtttcgtacttgataaatgtgaaggtattgttttgaaaaattttaatatagattataaacatcctactcaaacagaggttgaagtattggaagaggggaatgattatttgattgttcaggtacatcccacatcccaatatcggattgtagacgcacagttggagtggtatggtgatggttggtcttttaagaacggaatagcgcagtcgtatgaccgtataagtgaaatgacttggcgttcttggagtccgatggagaatttgcttcgtacagtagaacttcgtccaaatgtgttatatctgcaatataaagaaaaaccacaagtaggactacatactatttttcagatgcgcgattctttccgtgacgaagtgagtggatttgtaaacagaagtaagggaatactgttggagaatatcaacttctattatttaggaaatttcggggtagtctgtcaatacagtgagaatattactgttgatcgttgtaactttgctcctcgtccaggttcaggacgtactaatgcgggatttgctgattttattcaggtttctggttgccgtggtatgattgatattaagaattcccgttttataggtgcacacgatgatcctataaatatacatggtacacatttgcgagtaatagaatttttgtcggacaatcgtttaaaacttcgttttatgcatgaccagacttttggatttgaagccttttttaaaggagacgatatagaacttgttgattcacgttctctgttggtagtagggaagtgtaaagtaaaagaggcaaaattagtaacgccaagagaaatggaactcactctgtcaagtccactctcttcggaggtaatgcaacagaaagacctggttattgagaacgtgacgtggacaccggaagtgcggattacaaacaattactttgcaagagtaccaaccagagggattcttatcacaacacgacgtaagtctctgatagaaggaaatacattctacggcatgcagatgagtggaatatttgtagccgatgatggattaagctggtatgagtcaggaccggtacatgacttgactattcgtcaaaatacgtttttaaactgtggagaaccgattattagcattgatccggagaatagagaatataaaggggcggttcataaaaatattactattgaagaaaattatttttatatgagaaaaaatagctcatgtgccattcgagcgaaggctgttgatggcctgatgatacgtcataatttgatttattctctagatactgaaaaaaataaagagtctgattttattcagatgtataattgtaatgaagttacaataaaagaaaatcgggtacagttgcaccacctatttaaatga

SEQ ID NO: 117 - DNA, 2325 bp, Bacteroides sp.
  source: /note="GH3.0-6"
atgaagaagaatatcatatccatggcagcagcaatggctgttttgtcagcttgcggaccgggtgtgccgcagcttggaaagtcctctctggatgaggtgattggcgccatgaccttggaagaaaaggcgcatctggtagtgggtaccggtatggcaggtttctcgggtgacagtgccgtaatcggtgcaacgagaaagctagtgccgggtgcggcaggaaccacatacccgattgaacgcctcggcattcccgctgtggtgctggctgatggtcccgccggactgcgtatcgaccccaagcgtgagggggattcggctacgtactattgtactcatttccctatcggaactttgctcgcctctacctgggaccaggaactggtggaaagtgtaggtcagtccatcggtaacgaagtgctggaatacggtgcggacgtgctgttggctccggcgctgaacattcaccgtaacccgctttgcggacgtaacttcgagtattattctgaagacccgttggtgtcgggtaagattgccgccgcctacgtacgtggtgtgcagagcaacggtgtgggtaccagtatcaagcactttgctgtgaacaaccaggaaaccaaccgtatggctacggatgcgcatgtatctccacgcgccttgcgcgaaatctacttgaaagggttcgagattgccgtgaaggaatccgctccttggactgtgatgtcctcatacaactacctgaacggtgtctacacttcggaaaacaaggagttgcagacaaccatgttgcgcgacgaatggggcttcaaaggcatggtgatgaccgactggtttggcggcaaggatgccgtggcacagatggtggcaggcaacgacatgttgcagcccggtctgcccaagcagtacgaagccatcgtgaagggtgtgcaggacggagcgttagatgaagccatcctcaatcagaatgtgaagcgtattctggagatgattctccagactccccacttcaagggatataaatactccaacaagcctgatttgaaggcgcatgctgccgttactcgccagtcggcaacggaaggtatggtattgctgaagaacgataacggtgctctgccgctggctgccgacgtgaagaacgtggcactcttcggttgcacttcctacgatttcattgcaggcggtacaggttcgggcaacgtgaaccgcgcttataccgtttcgctattggacggcttgaagaatgccggctatgtggtggatgaagcgctgaagaatagctatgaagcttacctgaaaaccgagaaagaacgtctgtccaaagataagaaagagtggttcatgcccgatacccgtccggctgagatggctgtttccgcacaagtcatccgcgagcaggctgccaaggccgatgtggcactggtgacgctgggacgtacctccggtgagttccttgaccgtatggtagccgacttcaacctcaccaaagaggaacagaacatgttgaaagctgtgtccgatgctttccacgctgccggaaagaaggtagtggtagtgctcaatatcggtggtgtgattgaaactgcttcttggaaatctgctcccgatgccattctttgtgcatggcaggcaggccaggagggaggaaacagtgtggctgacgtgctgagtggcaaggcttctccttcgggcaagctgacaatgactttcccggtgaagtttgaagatgccgcttcttccgacaacttcccgatagacatgcgtgtgagcaccgacctcatgaacaaaggcgggaagaagaacgacgtgaagaacgtggactataccaattacgaagaggacatttacgtgggttaccgttacttcgacacctttggcaagcaggtttcctatcctttcggttacggtctttcctataccacttttgcttacgacaaggctgctgtcaaggcagacaacggtgtctataccgtgtctgtagaagtgaagaacaccggtaaggtagcaggcaaggaagtggttcagctttatgtatccgctcccgatgttgctgccaacaagcccgaaaaggaactgaaggcttttgccaagaccaaggagctgaaaccgggcgaagcggttgtggtgacgctgaaagtgaatgctgatgacctggcttcctacgatgaggctgcatcggcatgggtggtaactcccggaaactacaagttcctcgtcggggcttcctcacgcgacatcaaggctacgctggaggctgaagtagctgccgcaacgcagaagacgaacaacatcctgaaacttcaggaaccgatgagcctcttgaagagatga

SEQ ID NO: 118 - DNA, 2154 bp, Bacteroides sp.
  source: /note="GH31.0-13"
atgaaatatacttgtatcaaaactgtagcaatttacttgctcgcaaccttacctttattggcgaacgcctcaacacacaaggtaaaaattacacatagcgtcatggttggggacggaatcgcaaaattcatcccggaaggcttcgacgctcaaaagataccttcttttgcaatagaaaaagaaccacgcgaacaaggagcacttcctgccgactgggtacttgttcccgagttctcactcacggatggtaaagcaaacgcatcattaacagtgccggaaggtacaagcatctatggcggtggtgaagtgaccggttcacttctgagaaatggaaagaccatcaaattatggaatacagactcaggagcttatggtgtagacaaaggtactcgtctgtatcaatcacatccttggatgatgggagtgcgaaaggacggaacagcttttggaattttattcgatactacttggaaagcagaactaagcagtacagacgaaaaaatcgaattaaaaagtgaaggaataccctttcgggtattcatcattgacagggaatctccacaagcagtcattcgcggactatccgaactgaccggcacaatgccaatgattcctcgctgggcactaggttatcagcaatgccggttctcatattctcccgacagccgtgtcattgaaatagcagatactttcagactaaaaagaataccatgtgatgttatctggatggacattgattatatggacggataccgcatctttacctttaatccgaaaagttttccgaatcctaaagcggtgaaccgtgatttgcacatacgtggattccattctgcatggatgattgacccgggagcaaaagttgaccctaactatttcgtatataaatcgggaacagaaaatgacgtttgggtgaaaacagcagacggtaagaacttccacggtgatgcatggccgggagcagcagcattccctgattttacttctcctaaagtaaacaaatggtggagaaacttatataaagattttctagcacaaggagtagatggcgtatggaatgatgttaacgaaccccagatcaatgatacgcccaacaaaacaatgccggaagacaacctgcatcgtggaggaggaaagcttccggcaggtacacatcttcagtatcataatgtatatggcttcctgatggttaaagcatccagggaaggtatactggatgctcgtccagaaaaacgtcctttcattctgacacgttccaacttccttgggggacaacgttatgccgctacatggactggcgacaacggttcttgctgggatcatctaaaaatgtcagttcccatgtcattaacattgggattatccggtcaaccgtttagtggtgcagatataggcggtttcttattcaatgctgatgctgacttattcggcaactggattggtttcggtgccttttatcctttcgcacgtggtcatgcttgcgccggaacaaacaacaaggaaccatgggtatttggacaaaaagtagaagatgcctcacgcatcgctttggaacgtagatatatactactaccctacttttatacactcttacacgaagcctcaactaatggcatgcctatcatgcgtcctgtcttcttctccgaccctaaagacttgtcactgagagcagaggaagaagctttccttgtcggtgataatttacttatcattccagcatttgctaatcaaccggcacttccgaaagggatctggaaagaactgtcacttgtagaaggagatcagaatgataaatatcaggcaaaaatgaagattcgtgggggagctatcattccgactggaaaaataattcagaacactacagaaaattcattagatcctctgacattactagtgtgtctggacgaacagggcaaagcttccggaaatatgtattgggatgcgggagatggttggtcttacaaaaaaggggactatagcctgctacaatttgtcgcagagcgaaatggtgataaagtgactgtaaagctaacaaagaaaaccggaaaatacaacactgagaataaagacatggcagtgattaaaattataacagatcaaggcatacgtcaagccagtggaaatctagtggaaggcattgaaataagactataa

SEQ ID NO: 119 - DNA, 1131 bp, Bacteroides sp.
  source: /note="GH43.0"
atgaaatttatattgcgattaggacttgctttactgacaggatttgtctcagtcagcacagcatcggcacaagcatatggaactgctgatacaaacgctccggagctgcgtgtcccaaaatctgttcaaccggcatttgactactggatgcgtgacacatgggcaacactaggccccgacggttactactatatcactggaaccacttctacccccgaccgtcactttccgggacagagacattgctgggattggaatgacggtttgtatctttggcgctccaaagacctgaagatatgggaagccatgggacgaatctggtcaatggaaaaagacggtacctggcagaaagatcccaaagtatataaagagggagagaaatatgcgaagaagtctatcaataatgatccgatggataaccgtttccacgctgtatgggcaccggaaatgcactatataaagagtgcgaaaaattggtttattgtagcctgcatgaatcaatcggcaggcggaagaggctcttttattctgcggagtactaccgggaagccggagggaccttatgaaaatatcgaaggtaacgaggataaagccatttttccaaacattgacggaagcctgtttgaagatacggatggtaccgtatattttgtcggtcacaaccactatatagcacgcatgaaaccagatatgagtggtttggcagaagagataaagacattaaaagaaagtaaatactctccggagccgtatgttgaaggagcattcatctttaaatatgatggaaaatatcatttggtacaagctatctgggcacaccgcacggtgaagggggacacttatgtcgagaaggaagggttaactaataagaaaactcgttatagctatgattgtatcattgccactgccgacaatgtatatggtccttatggtaaacggtataacgcaattaccggcggcggacacaacaatctgtttcaggataaggatggcaactggtgggcaaccatgttttttaaccctcgtggcgcacaggcggccgaatataaagtgacatgtcggccgggattgattccgatgctttatgaaaacggaaaatttaaacctaatcacaattatcaggcaaaatga

SEQ ID NO: 120 - DNA, 972 bp, Bacteroides sp.
  source: /note="GH43.19-1"
atgaatatgaaaaaatatactttactcctggcactccttttagtaggagtgctgacaggatacagccagcaatctgcctacctgtttgtctatttcaccggaaacaggatgagtgaggaagccatccggatggctgtcagccccgatggatacaactactatgcattaaacggaaaccaaccggtcatcgattcccgtgaaatcagttctacgggtggagtgcgtgacccgcacattcttcgttgtgaagacggaaagacattttacatggtcgtaactgacatggtctccggcaatggatggagttccaaccgtgccatggtactgttgaaatcgaaagatctcgtcaactggacctccaacatcgtgaatatccagaagaaatacccgaatcaggaagatttgaagcgggtatgggcaccgcaaactatttatgataaagaagcgaagaaatacatggtctactggtcaatgcagcatggtaatggtccggacattatttattacgcatacgctaacaaagatttcaccgatatagaaggagaacccaaaactttgttcctcccgaagaatggcaaatcctgtattgacggagacatcatttataaagacggactttaccacctgttctataaaacggaaggagacggcaatggaattaaaaaagcaaccaccgcctccctgacttccggacaatggacagaatcggaagattataagcaacagacgaaagaagctgtagaaggtgccggcatcttcccgctgataggtacggacaagtacatcctgatgtacgatgtatatatgaaaggcaagtatcagtttacggaaagcaccgatttggagaatttcaaagtcatagacaatgccattagcatggacttccatccgcgccacggcaccgtaatgccgattactgacaaggaactgaaacgcttgtacaaggcctacggaaagcccgacaagatgtaa

SEQ ID NO: 121 - DNA, 2694 bp, Bacteroides sp.
  source: /note="GH92.0-1"
atgaaaatgaaattattgatactggccgttcttccattcctgacgccgattaacatgaactcacaagaggaaaaagcctcatgggtacagtatgtcaacccattgattggaacagaagtatggcaatccggagtagcggttgccgggcatgaagatccttcgggatatacttttcccggagtgacagagcctttcgggatgacagaatggactgcccatactttagagagcaagcacgctggaacgctgcaccatcgggtaccctactggtataaacataactatatttcgggatttatgggaacacactatccaagtggggccgtcatgttcgattatggtgctgttgaactaatgccggttgtcggacaactgaaatgcaggcccgaagagcgtagttcttcttttacccatataaccgaaaagtcaaaacctcacttctacgaagtcatgttggacgactatcaggtaaaagctcaattatcggctacaaaaacttcagctatcctgcaatttacctatccccagtcggatagtgcttacgtagtggtagatgctatgccttccatgtttacagccggagcaccgggctacattcacatagacccggtacgaaaagaaatttccggtaaaagcatacaatctgccagaggatatcgggaaaccggatattttgtagtccgtttcgataaggatttcgactctttcggcacgtttaatcttaataatgattatcccgaagtaatcgaagagaaatatctgttcactcaaaaagaaggcaagtgggtcaatggcttaaaagggatttatacacaggactcaaagggggtcggacatctgcggagtgaaaaaatcgatccggttatcgattttgactgggactggtataaacctgcggatgatttcagttttaatgattaccaggtgacctggagcggtaaactcaaagctccctctaccggtgaatatacattagggatacaagctgacgacggagcacgattatatatcaacggagaattgctcatcgatgactggaaatctcatagtttcagctatcaacctacccaaaagaagatttctctggaagccggtaaaatgtatgatataaaattggaatattatcagcatgaatggagctcacggataaaactgagttggatcaggcctgataaaaagtcatcaacatcccttctgactggcaatcgacatttggaatcgtctaccaaaatagggggatatatccgttttaaaaccggaaaaaatgaagtaattaaagccatcgttggcacatcctttattagtgtggaacaggcacggataaatctggaaagagaaatcggagccaaaagtatggaaacaatcagtgcacaaacagaagcattatggaataaagaattatcagtcatcgatttgcccggagctacagaacaagataaaattgttttttatacagcgctatatcactctttcctgttgcccagaagtctatctgaagatggaaaatacagaagtccgtttgatggaaaagtacataagggtattagctttacagactattctatatgggacacattcagagcgacccatcctctgttcgtattactgaaacccgattttgcgggagatctcataaccggactcctccatgcctacgatgagggaggctggcttcccaaatggcctaatccgggatataccaactgcatgatgggaactcatagtgatgccataatagcggatgcttatgtaaaaggagtgcgtaactttgatgtagagaaagctaaaaaagcagtgctgaaaaatgcgtatgaaaagggtaaccacattgcttggggacgcttgggcattatggactacgaacgattgggatatgtacctgttgataaatatggagaatcagtagccagaacgatggagtttgcctatgatgattattgtctctcccgtttctttgccgaaaaaggtgaaccggacttatcggataaactaggtaaacgaagcaaaaatttcaggaacgtactggataaggaaaccaaaatggttcgtgcgcgtaaagcagatggttcatggagtaatccggaagattacgatatcagcgtatggagtggttttaaccccaaaggagtgtacaactataaaaagaattatacgttgttcgttccccatgatgttcccgaactaattcgctttttgggaggtaccgattctttagccgtttttatggatgaactattcgataaagatatttactatgtgggtgacgaatttgtgatgcatgctccctatatgtataatctctgtaaaagaccgtggatgactcaaaaaagaatatatgatatagtcaataaatactatctgcccacacctagcggactgccgggaaatgacgactgtggacaattaagttcatggtatatcttcagtgcgatgggattctatcccatgtgtccggcttctattgaatatcagttaggagttccctgtctgccgggctttgtattgcatttgcctcaaaatagaacattcacaattaaaacaaagaatttcggcaaaggcaattgttatgtacgcgctgtatatctcaatggcaagcctcaccgtagttctgtcataactcattcagatattattaacggtggggagattttattcgaattaacagataagcctgcatataattggtttcaatag

SEQ ID NO: 122 - DNA, 2340 bp, Bacteroides sp.
  source: /note="GH92.0-2"
atgaataagatgaaaaagaaagtattgatgatgactatggcggcggtaaccttgtccgccgtagctcagcaaccggtagattacgttaatccgattatcggaaccaatggtatggggcatacttttcccggtgcttgcacccctttcggatgggtacagctgagtccggacacagacacaattccacataatgtgaatggagcttatcagaagaatgcgtatgaatattgtgccggttaccagtatcgggataaaaccatcgtaggtttcagtcacacccacctcagcggcacgggacattccgacctgggagatatattgctgatgcctgctgtcggcgatgtaaaattgaatcccggacgggcggaccatccggaagagggttaccgttcgcgcttcgatcatgccacagagaaagcgacacccggatactacgaagtgatgctggacgactatggcattaaagcgcaactgacagctactcaacggacgggtgtacataaatataccttcccgaaaggaaaagacggtcatctgatcctggacctggtgcatggtatctataattatgacggcaaagtattgtgggcaaacctgcgggtggaaaacgatacattgctgacaggataccgcatcaccaacggatgggcacgtacgaattatacctattttgccatttccttgtcacagccgatcaaggattacggatataaggataaggaaaaggtattgtacaatggcttttggcgtcgtttcaagctggagaagaatttcccggaaatcactggtcgaaagatcgtggcttactttaacttcgaaacggccaaagatcccgaactggttgtaaaggtagccttgtcggcagtcagcacggaaggcgctgtaaagaacctgcgtgccgaggcttccggaaagagcttcgaacagttggcggaagctgcacggacagactggaacaatgaactggatcatttcgaaatagaaggtacaccggatcagaaggcgatgttctacacttcgctttatcataccatgattaatccgtccgtgtatatggacgtagacggttcctatcgcggtctggatcataacatacatcaggcgaaaggattcactaactatactatattctcactttgggatacatatcgcgcggaacatccgttccttaacctggtgaaaccggaacgcaatgcggatatggtggaatcaatgatcaaacatgaacagcagagcgtgcatggcatgttgccgatatggagcctgatgggaaatgagaactggtgtatgagcggttatcatgctgtgtctgtgctggcggatgcaataaccaaaggagttttttcaaatgtggatgaggcattatcggcgatggttagcacatctacggtaccttactatgaaggtgtagccgattatatgaagctgggatatatcccgctggacaagagtggtacggcagcttcctctacgttggaatatgcatacgacgactggactatttatcagacagccttgaaagccggtaataaagagatagcggatacttaccgcaaacgtgctctcaactatcgtaacatctatgatacaagcatcggttttgcccgtccccgctacagtgacggcacattcaaaaaagagttcgatgtgttgcaaacttacggcgaaggctttatcgaaggtaattcatggaacttctcctttcatgtaccgcatgatgtgtttggtatgatcgacctgatgggaggagaaaagacattcgtacagaaactggacgaactcttctccatgcatctgccggagaagtactatgaacataatgaggatattacggaagaatgcctggtaggtggatacgtacatggcaatgaaccgagccatcatgtaccttatttgtacgcatggacctcccaaccgtggaaaacacagtactggctgcgtgaaatcctgaacaagatgtataagaatgacatcaacggactgggtggaaatgatgattgcggacagatgtcggcatggtatcttttctctgtgatgggcttctatccggtttgtccgggtacagaccagtatgtccttggtgctccctatctgccctatctgaagctgacacttcccaacggaaagacactggaaatcaaagcgccgggcgtcagcgacaagaagcgttatgtacagtcactgaaactgaacggtgagtcttatgataaaatgtacatcacacacgaggatatcctgaaaggaggcgtattggaatttaaaatgtcggcatcgcccaacaaacgtcgtggagtatcggtgcaggacaaaccttattcattaactaatggaatcaattaa

SEQ ID NO: 123 - DNA, 1701 bp, Bifidobacterium sp.
  source: /note="GH51.0-3"
atgaccactcacaacagccagtattccgccgaaaccacccatcccgacaagcaggaaagcagcccggcgccgaccgccgccggcaccacggccagtaacgtctccacaactggcaacgcaaccacgccggacgccagcatcgccctcaacgccgacgccactccggtagccgacgttcccccgcgtctgttcggctcattcgtagaacatctgggccgctgcgtctacggcggcatctacgagcccagccatcccaccgccgacgaaaacggcttccgccaagacgtgcttgacctggtcaaggagctgggcgtcacctgcgtgcgctaccccggcggcaatttcgtatccaactacaactgggaagacggcatcggtccacgcgagaatcgccccatgcgccgcgacctggcctggcattgcaccgaaaccaacgagatgggcatcgacgacttctaccgctggagccagaaagccggcaccgaaatcatgcttgccgtcaacatgggcacccgggggctgaaagccgcgctcgacgagctcgagtatgtcaacggcgcgcccggcaccgcttgggcggatcagcgcgtggccaacggcatcgaggagccgatggatatcaagatgtggtgcatcggcaacgaaatggacggcccgtggcaggtgggccacatgagcccggaagaatatgccggcgcggtggataaggtggcccacgccatgaagctcgccgagtccggtctcgaactcgtggcctgcggttcctcgggtgcctatatgccgaccttcggcacgtgggagaagaccgtgctcaccaaggcttacgagaatctcgacttcgtctcctgccatgcctactacttcgaccgcggccataaaacccgggccgccgcctccatgcaggacttcctggcctcttccgaagacatgaccaagttcatcgccaccgtctcggacgcggccgatcaggcgcgcgaagccaataacggcaccaaagacatcgccctgtccttcgacgaatggggcgtatggtattcggacaagtggaacgagcaggaagaccagtggaaggcggaggccgcgcagggtttgcaccacgagccatggcccaagtctccacatttgctggaagacatctacaccgcggccgacgcggtggtcgaaggttccctgatgatcaccctgctcaagcactgcgatcgcgtgcgttccgcctcgcgcgcccagctggtcaacgtcatcgcccccatcatggccgaggaacacggcccggcatggcggcagaccacgttctacccgttcgccgaagccgcccttcacgcgcgcggccaggcctacgctccggccatcagctcccccaccatccataccgaggcatacggcgacgtgccggccatcgacgcggtagtcacgtgggatgaacaggcccgcaccggtctgctgcttgccgtcaaccgcgacgccaacaccccgcacacgctcaccatcgacctttccgggctgcccggcctgcccggtctcggcacgctcgcgctcggcaaggcgcaactgttgcatgaggacgatccgtaccgcaccaacaccgccgaagcgcccgaagccgtcacgccgcaaccgctcgacattgcgatgaacgccaccggcacctgcacggcaacgcttcccgccatctcctggatcagcgtggaattccacggctaa

SEQ ID NO: 124 - DNA, 4002 bp, Butyrivibrio sp.
  source: /note="GH13.28"
atgataaaaatgggaaaaatggcgaagagattcgtcgcagttgccatgtcacttgctatggtagctggaattcctggtgcaaatcttaaagcatttgctacaccggggattgattcagttcaggcagcatcagctgttagcagatcatcaattcatgatggttcaatcctacatgcattttgttggaattttaatactataaaggagaagatgccagagatagcagcagctggatacacagcagttcagacatctccaatcaatgaatgtctttctattcataatggaatggctctttacggagacacagaagatgaaggtcgctggtactatcattatcagcctactgattggaagattggaaactatcagcttggttctcgtgatgaatttaaggctatgtgtgatgaggcagataagtatggcatcggcgtaatcgttgatatcgatccaaatcatactacgcctgtatttgaccaggtatcagatgatttgaaggctgcagcaggtggcgaagacagtctttatcacatcggcgctaaggacggtggtatggcatatgataatcgtatttccgttacttatgatgccatgggtggtcttccagatgtagatacagaaaatccaggattccagaattacttctacgaatttcttcaggactgtattgcttgtggtgcagatggatttagaatcgatactgctaagcacatcgcacttccagatgatggtgttgcagaggagtacgctggacaggaaggcagaaataatttctatccaaatatgaaagcctctattaatgagaaggctgcaaagtcatatgatgatttatttgtctatggtgaggtccttgatggtgatgcagctagacttgctgcatatcaggatatgcttggtggaacctgtgccagcaactacggcggagcaatcagaaacgctgcaagctccggtaatgtttcagtaaagaagctcttaaactacaaaatcagtgacgatacatcaacaggaactacttacacagctgattcaaacaaacttgttacctgggtagagtctcacgataactacattaatgacaagagctacaatgaggttgatgacagagaggtaatccttggctgggcaatcattacagcaagagcagatggaacaccacttttctttagccgtccagaaggaagcagtgcagaaaatccttggggtgcaaaccgcataggcgacgcagggtctgatatttacaaagcaccagaggtagttgctgttaacaagtttagaacagcaatggaaggactttctgagaatcttagaaacccaggaaataattcttcaatccttatgattgaaagaggaaacaagggtgttgtaattgtaaatgccagcgaaaatgattttgctcttgattctgagactaatctttcagatggtacatatgtagattctgttgaaggaagaactggactttacacagtatcagatggaaatatctatggcacagtacctgccaagtcagttgttgtacttgatacattagctgacggagactattccacgatcttcttccacaataccgacggttggaatagcgttagcgctattgcttgcgataatacttttgcttgtgattatacacaggacaattggtggaaggttacaattccagcgaaggaattcaaagtaacatttacagatggtgaaaaacagtctgctgaatttagcattggcgcagataccggcagatttatgacagcaaaatcagataagatatatggaagcaaggctgaggccgaggaggctcttggcattgttacaaagacagtgtatttccttaactcagaggaatggaaatccgtatatgcgtatgcttggacagatgctacacagcatttaggtggttggccaggtgcaccaattgttaatgaagaaggctactggtggaaggctgatgttaagatgattggcgaccagaacttctcaatcattttcaacaacaatgagggctctcagaccgttgatattccaatggatgatatgagcaaaaacgtaattaccatatctgctgaacagcctggtggaaatcttgtagtagatagatattcatcaaaggctgaggcagaagaagctacaggtattaacggaacttccacaacagttcacttctatgatgcagctggttggggaaaagttggtgtttatacctggggagatgtggatttaggcggctggccaggagcagaatgtgaatatgaaggtgatggctggtggaaaaagacaattaattgcggaccaagctcaaatttcaacatcatcttcaataatatgccaacaggagatgatgacaagcgccagacagatgatatgaagtgtgacagcctaaagaaggtttacttcatcggtgctaattataagtatggttcaaaggcagctgctcttgatgcacttgcaaatgacaatcttaagttagagaagaatcttcatccagagctgaatcctgtggaagagcctacagacagacctgttgaggaagagccagtattaggtgaagatgaagtaaaaatctactactacaatactgctaactgggataatgtaaatatgtatgcctggacagatggtgccaacactgaatattttggtggctggccaggaaaagctatgcagcatatcggtggtaactggtattcagtaagtgtaaataaagctgcattaacacacgaaggtttacatctcattgcaaacaatggagatggagagcagattaatgatgtggctcttatttctgagagaccaaatattgaagagaagccttctgagccagataagccagcaccatctgagccagaggaacctactgagcctgagaagaagcttaagccaattcaggaggaagaggctgataaggaaggatatacaaagatttatattcagcttgatgtagataagttcccagaggcagcaaatctctatgcttgggcagagggagttggtgatatcgatggaatcggtggctggccaggactttcaatgactcatattggaaatggatggcacagcatcaacttcccagataagtatttaaataaggctgaggaagtttcagaagaagcatctgaggaaaaagtagaggatgagaaatctgaagttgtaacagatgatactacaaaagaagttgttgaaaataacgaggttgaagagacagaaaaagcttctgatgaagtgatttctgaggaagagtcacaggagccagaagaggattcgcttgttgaagaggttagggagattttaacatcacttgttaatctcatcacttctgcattcaatcctttagaggtaaaggctgctgagcatcagacatttgctgatggaatccatctcatcgtaaacaacggcaatggatatcaggaagatgatgtaaatgcaagatttacaacagttcgtccaagtgcagaggaattaaagcaggaagaggaacttgttgtagagcctacaccagcccctgcaccagcaccacagcctggcggagcttctggaaatggcggttcatcttctggaagtagctcatcctcaggcagtagtgcttcttctggaagtgcttcggctactccagcacagcagattgcatcaatcgctgaaagccaggtcccacttggcgtatcacctgttaaggttgtagaggacagcagtgttgtaaagaaggtggcatctaaggttagaaagagcacttctaaatcgaaagaggtgtctgctgaggaagaagcagtggatactacatcagaggttgagactgaagaatctgtagagcttccagatgcagaaatcccagaggttgatgaagctgagactacagaacctgaaaaagaagaagtaagaattgttgacgagggtgtgcctgaggcagcagtagatacaggcagctcaaatcttgcagtaattatcttaattattgtagctgcagttgttattattggcggcgcaggatttgtggttgtgcgcaagagaaaataa